European Patent Specification EP 3 368 677 B1, published June 7, 2023. Title: INHIBITION OF BOLTING AND FLOWERING OF A BETA VULGARIS PLANT. Applicant: KWS SAAT SE Stichting Dienst Landbouwkundig Onderzoek. The sequence listing filed with the application follows.

SEQUENCE LISTING (42 sequences)

SEQ ID NO: 1 - DNA, 21668 bp, Beta vulgaris
  misc_feature (9833)..(11385): n is a, c, g, or t
  misc_feature (12467)..(12605): n is a, c, g, or t
  misc_feature (13741)..(14088): n is a, c, g, or t
  misc_feature (16396)..(17194): n is a, c, g, or t
atggggagaggaagagtgcagctgaagaggatagagaataagatcaacagacaagtaactttttcaaagagaagaagtggacttgtgaagaaagctcatgaaatttctgttctttgtgatgctgaggttgctctgatcattttttctcaccgaggaaaactctttgagtattcttctgattcttcgtaagtatatatatatatatattaatagtaactacttgttttctgctttctatttttaggtctgatgcatatttaatttaggtaatattaattccttatatctgatccttaatttttttttcttttaccatttcatttttgtttgttttgaataaaagaaaatttccccttcacgtgtgtcgaataggtcaaaatttttacttgaaggatgttctctttgattactaaaataggatccaacaatcacctgaaataaaggaagaagatggtgcaaagtttttactgtcatacttagtatttgataaatattctatgatgaacttgtataaattaggaaatagacctaactttcatgcacgaaaacattattccttcattcaatttttttattacttaaggatttacttttttattgatcatatgaagtagtagtacttgtaatcattcaatttttttgttggttaaataggactacattttaaaacaacccaattttaaaattttttgtgtgaatttcttccctttttaaaaataaagtctattatcatagcttagagtagctgtggcaaagctagacgaaataatacagaaatctggaaaggaaattgtactacttacatgaacacacttatttattacttgcatgatatctgcgaaaaagtttatagcaaatttggttaatatatagcgtagtactttggatattaatattactagtgtacaaatacttgatccaatgggtaatgaaacttatggaagatttgaccatacatgatgatgctaaatattaattgttattgtccagctttgttttccctccatccattggcatcttcatctttacattgctactccactcacttgtcaattgtttcgtcctttatgttctttattcacatgtgcaccatacttcaatactttccccttctttatcctcagtttttttttcttgtcattttagggttaatatccaatgaaatctagtttgctcgttttagatctaattttaattcgatcacaaccatccatatttttgtttcttagcttgacatctattctatggatctgggatcttcggtgtatagatgttctcggttttcagatcaagatcctattcatagacccatttattgtaaacacttaaatgtgttcttaaaaagttagtggctcgccaagtcaactcaataacataacccccacgacttcattacattacacaatgaaagattagatgtatgagtttgtgaagcttataattctatttcaagtaggactaggatgttttgtgcaatcagcagctagtagtctttttaatttaagtcagtcttcattgtgcatcatatatttttagaaatatatgcaagtttgaaaccatttagaacctcatgacccgcctgactcactataaaccggcaagagcttaatttttcacagctttgtatctttatgagtagcgctagctaggggtatgggcatagaaaaaaagggtttgggttagggtcttacaagatcttatccgctatttttatttcataatctttcaaaatacatgtttaataattcaaaatacatgtttaatactatctccatttcacaacatatgcaccaattgcctagctatggtccaacctagttggtttgtagcttgcattggatggttaggatgtattggagttgtttatgtgcaatcaaattttaattacgtatcaaaaaaaaaaaaaaaaaaacatatgcaccaatttccatttggacacacttattgaccaatttttgacaatatttttctcaccattttgtaagaaaaatcaaaatcaagtggaattttgttaagtttatctcagtcaaaagattccatacatcgacattttataatttttaatcatacgcaattagaaatatcaatgtctaaagaagcgtgttggaatacgtgaaaaagcaaatgatacatgaaacagatgtagtatatagaaaacttaattttgtgtcactcggatgtatgtgggcggagccttcctagaaggcgtacccaccttagtggctctgaatctttgacgacccgttcggttggtggtgataatagatggtaatagtaatgtaatttagtctaaatttataaataaatattaatatcattacccatggtaatacaagttcttcacaaaacatgtttcatttaaaaattatcattactaccttttcaagtggtattggatgataataaaattttaggcagggaaatgggtattgggatgaacattaccatgggtaatgacatgcaatttttgttacaagaatacagtataatacattactattgccaccatgtataaccattaatcaaatggaccgtgaggatatgatgttgaagaagaagtcttaacctctacgctattatttactagggtctgtaaattttccttttttaattataattcttgtgaaatcttcttcactgatggtactagcttattaggatgggtttctttagtatattgaaggctcttgttgacagagtataaaaatatttttggggtcgcaaccatcaatttaaacttttgtttgattataaaattattttttgaacatcaacaatctacttaaatttttggttgagttagttctttgacatggtatcacaaccatcatgacataaaggtctcatattcaaatctcattcacctctcatttccaagtagaatatttacctcaggtatgggtatgagggaggcttgtgttgcatgagtcaataacggatcttgaccaataatttaacaggggcgagttgataaattaagttttaatgtaaaattttaaatgatggataaaaacactaatacacaccaaaatataaatatacttttattaatggttacaaagagcttgtagctaatgtaataaatcaaaatcccaaaggtgcaatttttaagaaattatttccatttatttatttgaccattatgaaatcttcaagaaattgagtaagtttttaagaaatttaaggtatagttcattaactaaataaactactccagtaaaaaaaaattaccaaactgctttcttaagtaaaaaaataaataaatttatattttatgattgttaggaatgagtgtgaggaaataaaaagtactattatagttaaataaaaatgaaagttcttcagagaagaagaatagaagatagtacaatcaatgttaaatatttttctaaattagacaaattgatataaaccaaaaataaaggggaagaagaaagaaataagtaaaaaaagaaagaaggaaaagaaaaaaagaaaaaagagaagcaagtgaagaaaaacaaagaagtccaaatgtgtgttgatgcaaggttcgagcttgcaacattaagggctcaaactttcttttacactttggttcactgccaccgtgcccacagcttgttatgtgacatgaagtgtagtttgcttaatttatcttatacagttatgggggaccaagcctccacccgccccttctataatctgtcagtggttgcatccacactttaagtccaatagactcttgtctgagaggaggtgatagagtatataaatatttttggggcctcaaccattagctcaatcttttgattaagttggttctgtgacacttgtactatatactagttatatatatactgtaaaactagtaccacgagaacagtccttaatacaaacaacatgcccttaatagaattttcttagtatacacttaatataggttgactagctttttgcccttcagtatgcacacaccttttataatctgtatcgttgtctggtagatgataataaacctcagtattggcaatatatgaaatgacataatggccatgtttggtgattagagtttagagtttagaggttacagttcagagtttgtggttagatgattacttttttgttcagaggatttgactgctgatttaaataattgttgtgtaaaggtgtttggtaacacttagcttattgtttagagttttgtactttttagagcatgtaaaatgacatttatggacatatgtatttttttaaaacaaattttagtagtaattatatggacaaaatagtcatttgttttttctctctccaaaactctcatgaaaaagctcctctacccagctttttcaaaagagagttttgatcagagttttcggtacaaaactctctttagtcctctctctcaccaaacacccaaattagagtttttattggtcaaaactctaaactctctccaaacctctaaactctctctaaaactctctcccccaaacacccccaatttcttagaaaaatttgttgctcctttttattgcactatatttctatctccaaacataaagtttcttttacaaattttcatttctactccataccacctttatatggcaatataatttctatgaattaaaatgttcacaagttttgaggtggatttcaagagcatggacaatatgatcatgagactctccatacaaaaattacccttaaattttataatcatacaccaagcggtcgttaaagtattggaagtgcttgagtagtttgtgaaaattaacatataataaagtgcagatctcccctctagtaagtagtaagaagtagtaagacgatgtccctcatttgagaaagagaaaaacccttatcagtttctcttgtttctttgactgaacgcaagtcaaatagaagtatgtaactaggaaatccttggagaaatagattttctttaaaactataaaagtatacctatatatatggtaacccacaaaaatgtatataatctgatcaatatctaaacaaagtattcttatgttttctttcatcttgcttatttcctccctttccttttcttactttaatttgtttactctctttaacttatttctttgcgtatctcatttcactttacaaggatatatagttgattatgacagcttaataaatatattttggaactaggatttattggttgtcgttgttattttaatttctacactgatcggctagagtttctagaacatagggctttattgaaaccattagttaacaaaattgaatgacaatgattcaatatgatagaatatgtatgtattagttaatgtttgattattgtttgtatgtatataatcaaagattatttagtaatacttctatatacatattctattagaatcacttagaaagacccattgaacaataataaggataggcagacaagcaaacaaaagaaaaataaacctgttactccttccatttcttaatgttctactcggaattatagatacacactttgacacaaattagaaagagagtgtaaaaagtggatccatattaatatttttatttttttaaatgaggagagaagtgtgggtttattatgtttcaagggagatagagagcattgaatagtgagagaatatgtgccaaagataattaaatcattgtaaatcttttgccaaataaagaataaagcatgtgagtaaaactttaaaaaatgggcgaaaaaggaaagttgagtagaactttaagagacggaaggaatatagaagaggacgtgacagatgggaggaagatcagacatcttagaaggggaatagttaaatttgagatagtcttttaattaaggttctcactaaagaagatataacagtaggggaaagctaaaggttattcaaaactttccttcccatcttcatcacttcatgtctttactttagagctcttaacacttagcctatgaaattctgaactctttgtaagattagtgatagataaaagaatcttatcaatttaatttataaatacaacaggattcaataaaaagatatagagatctataaataaagagccatactgttgtgaacttttatatctatcaaaacctttgcacattagacgtggtataactaaatcaggcttatcgaaattttttaaaattgttttcattatagcccctttatatttagaagttctaagatgattgcatagatagttgatgcaccgttctggtcgacttttttaaacacttctttttgataaatttttttttttgtattcgaatcattattttaggtgtataaagagctgcaaatgatctagatgagattgatctcggtttcatttatatgctaatagtgtgttagatacacactattaaaaaagtcatatgacttagagattattatggaaaagggatagtgcaccgatattaatataatggaaaatgacacacgagttgtccataataacatgtgaaaagtgaactatttaaaaggtttttctgacctagtacatacaaggtgcgtaggtttagctattttagttttttagttttattttttaaagtgaagttagttattgatctgaaatcatataacatgtacgtaccgtagatataaaaaactaccaagtatatatcaatttgaaataaacattattttaatatggcaaaatcacaattgttgactagacctaacactgaagaaaactatgtcatgtttatcaattatgttgcatacagttaaaaacaaatatgttagagaaatcgttatttgaaatagaaaagttgcgcaaaatagtgattaacatcaaaatatgttcagaaagtttttataaatatgtgatcttgcattgtctgttgactgtcgaggtttatgataatttcccctttttccaatgcaaaacttgttgtgctattttctaatgatatattttttcaaagtatggagaagatcctagaaaggtatgagaggtattcttacgcagaaagacggctagcttcaaatgatccagactcacaggtagtgcatttatgtaaatatagatatactcttcatgcccaagaagcctgaattttttatcccactacgtactgcaaagccaagtttaattgaataattgtcctgtttaaattatttagttttcagtacaataatgtaatcattagtttgcatgtttaaaaaagaaaagcacaagttctgatcaagtgaaatataaattgtaacgaaagagccaagctagacaattacctagctaggagttatttgttatcgtttttgtttttaatttctagtttttttttttaaactagaaaatatagtttcaatcttttgttatcagttttcaaaatgacatatttaacataaatatgattgattttaaattcatttattatatcatatttcatttcaaaataagtgaaacacttgtctcaaaaagctcactctcacataaatgataaaagtgtttcacttattttaaaacggaagaattatgacttttacttttcataaaacgaaaaactgaaatatgacaataatctcaaatagcttggagaaaccagatttctatatatttccgtgatgaaatcacttttcattatacgtaggtaaactggacctttgacttcgcaaaactgaaggcgaagcttgaacttctacaaaggaatcataggtatgatggcaatatgtcataatttttctattattatttttgcttccaaaaccagaccatatgtttgtatatttatatagtgatatactccatccgtttcattttaatctatacatttacacttatcaggtatgtcaatgcaaaattttgaggatatatatctttagttttgtatttataaaaattataaaaagtacatattaataaaatacatattatgatgaatctaacaagatcccacatgacgatatttccgtccgcgtatgaataacaaataatggccaaagtgaaatttgtgaatagtgtaaaatatcaaagtgtaacaattaaaataaaacggagggagtagtacttgtttgtcacatacttacttatttttgttctctccacaatgaaactgttctttctaataattaaaaaaagtgcatatgttgatgatttctctgtcactttaagtggatattgaatagtgataatggattactttgtgtataattgcatttcacatttgggtctaattttatacccttttcgcatatcatgctttgtgaatagtacatatgatgttcaagaatgtgagaagacatatcatacttttgatatacctcaaacatgggtgtatactgtatagtgaacgaaagtgttagtgtaattttatttaggaggtttagtggtttgtcctatatataatgctagtagttatacaccatagttgttgatgagcatcaactggctttcctaacatttttttctccataactttacccttaccttacattagattactctaggattacattctacctaaaatattattactcccatcattttaggtaaatatttttactttgatttttcgattattttcaagagtttaaaataatgattaaaatttaccatgatcaggcactacttaggacaagagcttgactcacttaacatgaaggaacttcagagtttagagcaacaacttgatactgctctcaaaaatgttcgatctaggaaggtaagaaattttacttgtctaccgtagtttcataataaattagtatttgggctcgggctttgccccagattggtattgtcttttcaaatttgatatgcatttttttccatttccactaaaatatattaagaaaattcaacatttaaaggatacaaatataataatgtggatacttaaagtatgattaaaatttggttgagatggtaattgtgtcatgtataatagcaagaagtcacaagttcaaagctcgttgcaagctaaatttatttttgttgattgacatgacttatcaacacactggacaattctaatcatctagtggagtagcatatactagcaatttatgcacgtgatgtgtgccttacttttttagaatataatttataacttttttgagcataaacaaaggtaaaatttgaacattagacatatttttttgggctagctaaatttgttgtttaaacctatatcacttaaccaaactcctcttttattatttattgatttatattttatttaaaatttttaaaattaaaatgatgagcaataaaagaatgttaagtagatttattaagtatttcttatatttttatcaacaaagtattttgtgttaattaaattatttcactttgttaattgattgtattttcctttttaatttattacttgattgtgtattgattgatcaaacataatttttttgttaatttttttatgctatatttgaatttatttttctttcatctgtttttggtagagtagttgatttactaaagggtaattaaataaatttattgggggacaccatagctcccccctcccttatataatagagatttgtatagatttattgtcttcctcaattattgattaactagtcttctatgcacgcgatgcgtgtgttgattgtttgggtctattcttaatataaatttcatcaaaatataattatagtagtgtgatttacaattattgctatacaaactactgtaatttataaagttgttagaaattgagataaaaatttagatgtgaaattttgtggtcaaattatatttgtaattttttaaactgagtaaccgtttttctcatcatgtcaagttactttgttaatgcttatttaatttattattggaatttttgacccatctttaaattagaaaaggatataatnnnnnnnnnnnnnnnnnnnnnnnnnnnnnnnnnnnnnnnnnnnnnnnnnnnnnnnnnnnnnnnnnnnnnnnnnnnnnnnnnnnnnnnnnnnnnnnnnnnnnnnnnnnnnnnnnnnnnnnnnnnnnnnnnnnnnnnnnnnnnnnnnnnnnnnnnnnnnnnnnnnnnnnnnnnnnnnnnnnnnnnnnnnnnnnnnnnnnnnnnnnnnnnnnnnnnnnnnnnnnnnnnnnnnnnnnnnnnnnnnnnnnnnnnnnnnnnnnnnnnnnnnnnnnnnnnnnnnnnnnnnnnnnnnnnnnnnnnnnnnnnnnnnnnnnnnnnnnnnnnnnnnnnnnnnnnnnnnnnnnnnnnnnnnnnnnnnnnnnnnnnnnnnnnnnnnnnnnnnnnnnnnnnnnnnnnnnnnnnnnnnnnnnnnnnnnnnnnnnnnnnnnnnnnnnnnnnnnnnnnnnnnnnnnnnnnnnnnnnnnnnnnnnnnnnnnnnnnnnnnnnnnnnnnnnnnnnnnnnnnnnnnnnnnnnnnnnnnnnnnnnnnnnnnnnnnnnnnnnnnnnnnnnnnnnnnnnnnnnnnnnnnnnnnnnnnnnnnnnnnnnnnnnnnnnnnnnnnnnnnnnnnnnnnnnnnnnnnnnnnnnnnnnnnnnnnnnnnnnnnnnnnnnnnnnnnnnnnnnnnnnnnnnnnnnnnnnnnnnnnnnnnnnnnnnnnnnnnnnnnnnnnnnnnnnnnnnnnnnnnnnnnnnnnnnnnnnnnnnnnnnnnnnnnnnnnnnnnnnnnnnnnnnnnnnnnnnnnnnnnnnnnnnnnnnnnnnnnnnnnnnnnnnnnnnnnnnnnnnnnnnnnnnnnnnnnnnnnnnnnnnnnnnnnnnnnnnnnnnnnnnnnnnnnnnnnnnnnnnnnnnnnnnnnnnnnnnnnnnnnnnnnnnnnnnnnnnnnnnnnnnnnnnnnnnnnnnnnnnnnnnnnnnnnnnnnnnnnnnnnnnnnnnnnnnnnnnnnnnnnnnnnnnnnnnnnnnnnnnnnnnnnnnnnnnnnnnnnnnnnnnnnnnnnnnnnnnnnnnnnnnnnnnnnnnnnnnnnnnnnnnnnnnnnnnnnnnnnnnnnnnnnnnnnnnnnnnnnnnnnnnnnnnnnnnnnnnnnnnnnnnnnnnnnnnnnnnnnnnnnnnnnnnnnnnnnnnnnnnnnnnnnnnnnnnnnnnnnnnnnnnnnnnnnnnnnnnnnnnnnnnnnnnnnnnnnnnnnnnnnnnnnnnnnnnnnnnnnnnnnnnnnnnnnnnnnnnnnnnnnnnnnnnnnnnnnnnnnnnnnnnnnnnnnnnnnnnnnnnnnnnnnnnnnnnnnnnnnnnnnnnnnnnnnnnnnnnnnnnnnnnnnnnnnnnnnnnnnnnnnnnnnnnnnnnnnnnnnnnnnnnnnnnnnnnnnnnnnnnnnnnnnnnnnnnnnnnnnnnnnnnnnnnnnnnnnnnnnnnnnnnnnnnnnnnnnnnnnnnnnnnnnnnnnnnnnnnnnnnnnnnnnnnnnnnnnnnnnnnnnnnnnnnnnnnnnnnnnnnnnnnnnnnnnnnnnnnnnnnnnnnnnnnnnnnnntatatatatatttagctaagaaaaaaaagacatttcattgggggataccataactcccccttagcttatataatagagatactatacttcttttctgatagtgtcaaatttaattataaatctttaacattggccaattaataattggacaagaaaaaaatgagacaataataaataaggcgatcttcacagacgtattaacatgatggtaattaaaaatgttaatcatagatctttgtgttatcttaataatataaatttactaattagaatgtatcacataaagtaagtattaatagcagcataggataattcttataatggagattttatatttttttatataattatatgatttattgttgaaaatattagttgattttaactggttgtttattcaatgacagaaccaactgatgcacgagtccatttctgaactccagaagaaggtaataactccattttttactctcaaaggtttattgtttttaacttatttcttctaaccttttatatatgagaaggtattgggttagacgcgtctgaccataatattaggtcggatgactttcagttggtttcaattttatttcagttggtttcaatttttgtccagttggtttcaatttttgttcagttggtttcaattttttttagctggtttcaatttttgttcagttggtttcaatattttttagttgatcttttttatttcagttggatgtcttttaagttcagttacttatcttattgtttcatttacgtgttttattgtaactgaaaacaaaacttaagtaaatgaaataaaataagttctaaataaaagcaacttagggcctgttctccccagcttattttcagttcagttcaattcagttcagttcaattcaattcatttcagttcagttcagatcagatcagttcagttcagatcagatcagttcttgacaatacttttactctcacatatcactattcatttcagttcagttcaattcaattcagttcagttcaattcagtttagttcagttcagttcagttcaattcagttgttttatgccgaagagaacaggcccttagnnnnnnnnnnnnnnnnnnnnnnnnnnnnnnnnnnnnnnnnnnnnnnnnnnnnnnnnnnnnnnnnnnnnnnnnnnnnnnnnnnnnnnnnnnnnnnnnnnnnnnnnnnnnnnnnnnnnnnnnnnnnnnnnnnnnnnnnnnnattcatttcagttcagttcaattcaattcagttcagttcaattcagtttagttcagttcagttcagttcaattcagttgttttatgccgaagagaacaggcccttagttttcagttacttatattatcgtttcagttagttttcttattctttcatttaacaactaactaaaataaaaaaaaaaaaactaactgaaagcaaaacttaattaaatgcaaaaaattaagttctaaatgaaaccacatacgatcgaaatttcaatcatttcaaacattatggtgttttcgattctttcaaagaaggcaagctgctcccgctattctaccctctttagatcacaataaagctcaggcctcacattcaaagtttcctcaaagatggacgttccaagtatcacatagacacatagtcctcttctccaaacgctctccttcctatcttgatgtcattagcaaacttcttgatccagacggcgccaacaaccgcaccatgatctccctctaaagtactgacggcccgtttggttgttggtcataaatgatggtaatgggaatgaagttgtgtgtaaatttgtgaaaaatatcattgtccattcccatggtaatgctaatttatcttaatgtgtccactttccttctagaattttcattctcatccaataccaccttgtaaggtggtaatgagtggtaatgaaaattgcttccccttggagacaaaaatacaagtttaggagtgagattgattgctcatggagaaaaaaagtctccccatggagatattaagggtgattccctaataaaattacacttaaaatttattcccattaccgcaatttattaacatctaccaaacgggccgtgaaagtcttgaaacacatagtcgagtgagtagctttgaggaaccatctgtaaaagaacctgagggagccaatgtgtgcgtaagtaccaacggcgtgttgtcagtggaaaaggtggtgccgtggtggcactcagtagtgatggagccgccgtggtgtttgagtgttgccaaatacaaaggcggaatttcgtaatctctaatttcttctgtgaaatttttgggatcagcctgtccgaccaaacacattggatcaaacggtctgacccaatagtttcaannnnnnnnnnnnnnnnnnnnnnnnnnnnnnnnnnnnnnnnnnnnnnnnnnnnnnnnnnnnnnnnnnnnnnnnnnnnnnnnnnnnnnnnnnnnnnnnnnnnnnnnnnnnnnnnnnnnnnnnnnnnnnnnnnnnnnnnnnnnnnnnnnnnnnnnnnnnnnnnnnnnnnnnnnnnnnnnnnnnnnnnnnnnnnnnnnnnnnnnnnnnnnnnnnnnnnnnnnnnnnnnnnnnnnnnnnnnnnnnnnnnnnnnnnnnnnnnnnnnnnnnnnnnnnnnnnnnnnnnnnnnnnnnnnnnnnnnnnnnnnnnnnnnnnnnnnnnnnnnnnnnnnnnnnnnnnnnnnnnnnnnnnnngatataaatagagatggaggacaagggtcttggttttgtcatgttgtcaaagagttgaacaatggttttttcgtattgttaaaaaattaaaaaaccagaggccttcaatctcttgatagatatagatagaaaaggaggacaaggccgttcttggttttgttatattgtcaaagagttgaacaatgattttttcgtgttgtcaaaaaattaaacaatgaaaaaagatggcgggtgcttgatctaatagatcggaccatggattgaaggtcttttaacttattttatatatatattgaacttatctgaagattatttaactctttgaaattgtattaacttccgaactttatgaacttttttaattcttcaaaacttatctacattttatttgaaaaaatattgaagacaaaaaaaccctcagttggtttaaagctgcggtaagatagagtgtaaatgttatttttttttattaaatcaagaaataaaaagaaatattaaataaaaagaattaaaaatggaaatgatgacagaaacttatggcttggaggagcaatacttttaagatagacctaaaccttaaataagttaaaatggaagtaatttttcagtagaatcttattccaatctatactccgtgtttactccatgtaatgcacatataataaaaaaattagaaattacatagtataaggtttgatcctgtgactgtaagtttatatactaacttcttaaccactagagcaagtgatatttagtgttatcattttaaagtataattttaacaaatgaaatttttttcttacccggaacatagctcggacctaataactagttgaacaattataatctgtaacttaaaatgatcctaattactgtactttcattacctataataatagaatcttactatcattggttcagaaaaaaaaaatcttattaaatgttaaccatttatttgtaattgaaacatacatgcacataaatgtaacttttagtttatcttaacttaaaaactgagaaaatgttagttggaaacttttgtatatatgtttggataaacgacgctcaaaagtaggggctaaaattttagtagataatataagattatactccatctgttctagatagacttctcatttttaattttggcagtattcataaataaaggaaatctttcaaaaaaatttccaatatataagaaaaaaaataatcatgtgcggttttgtttgattcgtctcattgtgtacattaggaaaattaaacttatataatttttactactatgtaattaaagatattaacgatacaaaatgtgtattgacaaacttatattggagtaataggaagtctattaagggaccgaagaaatattacgtaaataaatctaatacaaactaatataaattctactccagacaataaagattctgtcttatattgccaagatatagtagctatttattttatcttaacaaacataaatgtttctaatgcttaaacatggacatgtattattttgtaaaatattatgtattatccaaagttacatatttaaaggaagttctattgcttgctctcttttagcactgcccaaaaaggttaaagtaattttttttctctgtttaaaaaaaaaatgcattatatacagataatttttgctagtcaataaagctatccttatgacttatgagtgctacttgactagggatgtgttgtactcaattggaggtatacatacaccaagattatagagcttttattttgcctataaaaaatggaagccggataggataccaaaaaagctttgacttaaatttgtaatgcataaaaatgatgatacctaacttattagccatacttatctaagcgtacgtcaatttaaatattgtgttattgattaataatgatccttatatatccatattttgacaattaaacggtaaattagagagaaaagtttgagaaaataattatagcttacgtaatgctataatccaaagtgtctccgcacaagcgtgggacaaaatagtactttcggagaagttacaatcaacagctagggagtcttcattgttcttgaatagaaggatggaaacaaagttcaccttcttttattaaagtattaaggtttgttattagctcaatatccaatactttctctgctttttattacttcgtctgtttcaaattaaatgattttttttttattttacactatttttaaatttcacttttaccatcatttatgatttatatgtgaatgaaaacatagttacgtgtgatcttgttttttttttttttttttgtnnnnnnnnnnnnnnnnnnnnnnnnnnnnnnnnnnnnnnnnnnnnnnnnnnnnnnnnnnnnnnnnnnnnnnnnnnnnnnnnnnnnnnnnnnnnnnnnnnnnnnnnnnnnnnnnnnnnnnnnnnnnnnnnnnnnnnnnnnnnnnnnnnnnnnnnnnnnnnnnnnnnnnnnnnnnnnnnnnnnnnnnnnnnnnnnnnnnnnnnnnnnnnnnnnnnnnnnnnnnnnnnnnnnnnnnnnnnnnnnnnnnnnnnnnnnnnnnnnnnnnnnnnnnnnnnnnnnnnnnnnnnnnnnnnnnnnnnnnnnnnnnnnnnnnnnnnnnnnnnnnnnnnnnnnnnnnnnnnnnnnnnnnnnnnnnnnnnnnnnnnnnnnnnnnnnnnnnnnnnnnnnnnnnnnnnnnnnnnnnnnnnnnnnnnnnnnnnnnnnnnnnnnnnnnnnnnnnnnnnnnnnnnnnnnnnnnnnnnnnnnnnnnnnnnnnnnnnnnnnnnnnnnnnnnnnnnnnnnnnnnnnnnnnnnnnnnnnnnnnnnnnnnnnnnnnnnnnnnnnnnnnnnnnnnnnnnnnnnnnnnnnnnnnnnnnnnnnnnnnnnnnnnnnnnnnnnnnnnnnnnnnnnnnnnnnnnnnnnnnnnnnnnnnnnnnnnnnnnnnnnnnnnnnnnnnnnnnnnnnnnnnnnnnnnnnnnnnnnnnnnnnnnnnnnnnnnnnnnnnnnnnnnnnnnnnnnnnnnnnnnnnnnnnnnnnnnnnnnnnnnnnnnnnnnnnnnnnnnnnnnnnnnnnnnnnnnnnnnnnnnnnnnnnnnnnnnnnnnngtacatcaaggaaatttgcattaatgaaaaacgggagtacaacctaatggtaatacaaccaaactaaacagaaagaagaaacaacagacagtaagaaaacctctataacgcgtaaaaacaatttaacataaacactaactagaaaaagtccaggccgaataacatttgtcttgtgcgatggggagggaagatgaaggagagtgaaaatctgttgaaagacacaactctgacgatcttcatagagagattgtcgtacaactgctagtagatcctgtccactaggcacgaaatcccaaggtccttgatgagcctcctgggattctcctgattcgttgaacaaagaagtcactttcgagagtaacttcggaccctgctgcgagggtcttcgaaaatcagtcacattagactgaaacccgaaaaacaaggtggaggtcttgacgtgccccaaaacaagttgggggcgtcccacaagatgcgttttttaggtgtgatgacacatgatgtcatcacgagaaattggggcgagttagtttgatgaactacgccccactgacggatcctaagatccaaagtgacaatctcgaaaccagaagaccgacaaacaacagatctgaaacatacaaacatgaaaataatgaaagcataaactgccacccgacatatagagctccggcaaacaacaccatcaagaacttgcaccaaagacttccttggcatactaaagacactgattccaactaacactagcgggggacggggaagggacactcgactacacctaaacctaaccaggggacggggaaggggaacttagactaaaccttcgtaaaaagggggggatcggggaggggaaaaccttgaccaaggaagctggttttaaaaaccacttagccgagccaaaaaccgtgggtgggaagaagaaacagaccacaaacagggggaaccgggggatgggaactcaccgaacaggggagggggagaaatcgcacagactcggggaacgcctaaggactgggggacgaccaacgaacgaaaggttggggtggtgcgaaaacaagggagggggacgcaccgacgaacaaaaaaaccgacgaagaggccgaaaaagcgaaaggccgacggagataagattgaaaggcgacgaaaaaagaaaaaggaacaaaacgaaagaaaaacgaactcgtcggagacccgccggagacctacgcggcgccggatctccggcgagttctagggttagagggtttgttgtgtttgtttagggagaaggcagaggttttttttttttacgtgtgatcttgttagatttgtcttaacatgtattctttaatatacttttttttttataatttttgcaaatgcaaaattagagatatatgtcctctaaattttacattcacatacgtgataaataagagtgctacaactaatttgaaacggataaagtatttgaattgtttttcatttaaaaaagttcgctatcatttataatgttatatatttgccaatatgttatctctttctctctcttaccagagtttagatccagtagagttagtaaataattctaccacgtagagttgaacaaatcatagccattgattttcaaatcattggtttatatattctttcccaaaactcccccctattttccccaaaaatcctccccctccttatctctttccataaaatctgagtcgttgattttaaaatataaggtttggattcaactccactatgtagagttttcatcaaactccaccgaatccgagcccctcctaccatagtacttcttgatttccccatatttctttcctcatcttggtcctcaagcacattttaatattatgggtattaaacaatagagaaagtatttacttatagagaaagtattttcaatgattccctaaatttttttttgaaagaaagaaaagggatttcattaatatttcgccaaacggcacttacaagtcatttctgaaaaacataaaattctaaaagaaatacatatcaccctagaaatgtaaacatcgcagatttgacttaattttgccttaataaaaatcttcatctgaagcaatgcaatctgtgagttcgctctggttcggcatacgatctgcagatgcggaaattttgggatgaacgtactccaatagtcttccataattttacagaagttgtgaaaccctaattcttcatgttgaatctcgaacttcaaccaatgagaataatttctcatacctaaaaacaaaagaaccatactcacaactcccataggggagaaggagatttccaaaacagaaactaaaaaccccataaaagggtttgagaaaatctcataaagagatactaatttattgaacaaaacaagaaaatgaactaaaaactgaaaataaaagggaaaaaggggcttaccatggatgaaaacatccatggcagccccctaattgatgaagaaggggtaagggaggctagggttttagagagagaaaaggagaggggaggctaggttttaaaaaaaaatataatgattccctaaatttacttatatatatttaccaagatgacgtgatgttttacaaggcccatgatttttacgcgatcatgaaaaacacagccaatttgaatggagcaaatatctacgcgtcattttagatatttttgtatgggaaagttttttttgaccaatgtaattattaagaagcatcggccaccgggtagataagatgtcactatacatccttttccaaacttaagtatgcctgttgaacttttgttgcgtttgcagattcatttgaaattatatttcctcagatcctctacttgtaaaagaatgttccattattttcttagtttacatgatatttacaatagtatttgtctacattttgttcatattacttagtgatcagtgtatacgtcatatattagtttgaactttgaagacatttattttctatatacttcctttgtctgctaaattactttggaaagctttgttttttttattaatataagaccctttggagtttggaaatcactatctaatgaaatatataattcatcattagaacaaaaatacaaatatcgtactatcacctatcatgttccttttggatttcgcttcacaaaaatacattttaaaaaaaaataaaataacaaatggtagctaacaacttattacttttaaaagtttgtgtgcaccctaataagtactcaaagtagtatgtaacagagagagtataatgctaaaatacaaactaaataaacaagaaagtgtttctcaacaataatttgctgcaggaattaggaaacaaagtaaataaattgcatgtttatcatcaatacaatttactggtagttaattacaaacttcactcatgataattgaaagaggccactcaatttcagctaggagttgtttatttatttatttttctttcagttaaattttgactacccacaaaatcttcatctggacctaatctgcaatttgtggattttggatgaaatttctaacctatttaagtagtcttattgtttaaataacccatgcaattaaattaggttatatgggggtgattcatttaccaggcccaagattttatctcattctcaattattatcgcaacacccatgaacctaagccaacatgacttatttaccaggccagctagagaagaacaaggttgctgattttcttgtccgtgattgtagaagaaatgttagaaatctaaatgttgttagggatttacccctcccccctactgagtgtatgaacttattattgacggattgttgtaggcttccaagccaaaactctgattaagttttcttttatgccattttaaccaaaaaaaaaaaaaaagctaggaagctagctcagcgcgctctaattatttcacatgtgacatgttttacacttattcatacttctatatgcaggagagggcaatgcaggagcacaataacatcctgtctaagaaggtacttgcacttgaccagtttgtgtaatattgtaatttaatttcttagattttggttgcatgctttgatgacgaatgacgattgacgaatacatttttatgcagatcaaggagagaggaaaaaatctagagcaagtgcaacagatgcagtggcagaaccagcaccagcaccagcaccagcagcagccgccaccgccgccacaaaatcatcaagttcctcctgatgcatcaaatttcatgctcccacctccaattccttctttgaacacggggtagttacttcttcaacttaatttcctctattcaatattaagttaagaaacagatcacgtgattagttcgttaatattgctaattaataatcatattgttatatatcatgcattagtgggtaccaaggacaatttggtggagaagtaaggaggaatgatcttgacctgacgctagaaccgatatactcatgtcacatgggatgctttacaacatga

SEQ ID NO: 2 - DNA, 780 bp, Artificial Sequence
  BvAP1 cDNA
atgggaaggggtagggttgagctgaagaggatagagaataagatcaacagacaagtaactttttcaaagagaagaagtggacttgtgaagaaagctcatgaaatttctgttctttgtgatgctgaggttgctctgatcattttttctcaccgaggaaaactctttgagtattcttctgattcttctatggagaagatcctagaaaggtatgagaggtattcttacgcagaaagacggctagcttcaaatgatccagactcacaggtaaactggacctttgacttcgcaaaactgaaggcgaagcttgaacttctacaaaggaatcataggcactacttaggacaagagcttgactcgcttaacatgaaggaacttcagagtttagagcaacaacttgatactgctctaaaaaatgttcgatctaggaagaaccaactgatgcacgagtccatttctgaactccagaagaaggagagggcaatgcaggagcacaataacatcctgtctaagaagatcaaggagagaggaaaaaatctagagcaagtgcaacagatgcagtggcagaaccagcaccagcaccagcaccagcagcagccgccaccgccgccacaaaatcatcaagttcctcctgacgcatcaaatttcatgctcccacctccaattccttctttgaacacgggtgggtaccaaggacaatttggtggagaagtaaggaggaatgatcttgacctgacgctagaaccgatatactcatgtcacatgggatgctttacaacatga

SEQ ID NO: 3 - DNA, 29237 bp, Beta vulgaris
  misc_feature (1029)..(1924): n is a, c, g, or t
  misc_feature (20703)..(20722): n is a, c, g, or t
atggggagaggtagggttcagctcaaaagaattgaaaacaagatcaaccgtcaagtgaccttctccaaacgtcggattggattgttgaagaaagcgcacgagatctccattctctgcgatgccgatgtagctctcatcatcttctccactaaaggcaagctcttcgagtatgcttctgatacctggtatgtctaattttataacttcttcttttgtacatcaataattttatcatcgactcaactaaaagcttaagcagatggttagggttctattattattgaattacctcaaatttgtcatcgactcaactaaaagtagagtatatttcatgtagatcaggtgctttttttgaatatattgtcagttttagaactacaaaatgttgaacacaagtatttatacgcacgctgacatgtgaattttttaattgacaactttctaaattaatactctaaattactaatatgaagaacgtaatttattatttatcactttcagacaaaggcatgtttgttttttctattatttttcccatgaaaattctcaccaatatccgattctgtatgttaattttagtaatttctaattttgatgacttaataaattgtaaaaaagtataaaataaacaaatatccaaaacatctttgttttcaagagaaatatcttaaaaacttttgttttttaagagaaatatcttaaaacactttttatcatactactatgatgatgtataaatctattcaaaaaaaaaaaaaaatgatgatgtataaataatttaaagagttaagtttattagaaattatagatatttatagagctgagtaataaaataatactctacagattatatgtagctgatgtagtgtgtctgctcctgtaagatttcctttttatctccaaaaaaattgcattgatattcgagccttgccgacccccttttcctcttcaaccatttgataagatcctatgcactgagtaatctagtattatatgttagatgttatatattaataagctaaaattgtnnnnnnnnnnnnnnnnnnnnnnnnnnnnnnnnnnnnnnnnnnnnnnnnnnnnnnnnnnnnnnnnnnnnnnnnnnnnnnnnnnnnnnnnnnnnnnnnnnnnnnnnnnnnnnnnnnnnnnnnnnnnnnnnnnnnnnnnnnnnnnnnnnnnnnnnnnnnnnnnnnnnnnnnnnnnnnnnnnnnnnnnnnnnnnnnnnnnnnnnnnnnnnnnnnnnnnnnnnnnnnnnnnnnnnnnnnnnnnnnnnnnnnnnnnnnnnnnnnnnnnnnnnnnnnnnnnnnnnnnnnnnnnnnnnnnnnnnnnnnnnnnnnnnnnnnnnnnnnnnnnnnnnnnnnnnnnnnnnnnnnnnnnnnnnnnnnnnnnnnnnnnnnnnnnnnnnnnnnnnnnnnnnnnnnnnnnnnnnnnnnnnnnnnnnnnnnnnnnnnnnnnnnnnnnnnnnnnnnnnnnnnnnnnnnnnnnnnnnnnnnnnnnnnnnnnnnnnnnnnnnnnnnnnnnnnnnnnnnnnnnnnnnnnnnnnnnnnnnnnnnnnnnnnnnnnnnnnnnnnnnnnnnnnnnnnnnnnnnnnnnnnnnnnnnnnnnnnnnnnnnnnnnnnnnnnnnnnnnnnnnnnnnnnnnnnnnnnnnnnnnnnnnnnnnnnnnnnnnnnnnnnnnnnnnnnnnnnnnnnnnnnnnnnnnnnnnnnnnnnnnnnnnnnnnnnnnnnnnnnnnnnnnnnnnnnnnnnnnnnnnnnnnnnnnnnnnnnnnnnnnnnnnnnnnnnnnnnnnnnnnnnnnnnnnnnnnnnnnnnnnnnnnnnnnnnnnnnnnnnnnnnnnnnnnnnnnnnnnnnnnnnnnnnnnnnnnnnnnnnnnnnnnnnnnnnnnnnnnnnnnnnnnnnnnnnnnnnnnnnnnnnnnnnnnnnnnnngatgatattatgtatcattattatcagtcatttattattgatagataatgttattatttccatagatcatatataatcttaccatatttactccctatgattatatatttctatctattaacatagtaatagtgatatactaacaacgagtatctttcaagtaaataaatcatatatatagggttagaaggtaaaaaagacaatattttatgagactttatttacacccttcgtctcataaactcctttctattttttgtgttcactcgttttctaaagttttttctacttcttttactttttattggataaatactttttccgtctgtatgtgatctacttatattagtatttatagatagattatactcttaaagtattacattcacaaaatcatgtgaattattaattaaagtaaaattatgagtatggtattataacttaaacgaagtagttgtattgtttaaaccaataagtataataacttataaaacttaaaagttgattctacacttatcatgcacttgtgttttgatgggttaaaaattagctagtacataagtaacataacataaacttatctctgtatagtatgttgaattattactttatatttgaaaagaacaaagacacaataagtccaaaagatccgatcttttgattatcaactatgtaagtgtctttcctaaatgatcaatcaccttaattagtatactaaacaggacaattatgacatataacacttttctatttgtacaagttaattaacccattgacattcattcagttagcctacatttttcaataggtagtcatcatcattctttttttaaccaatttttttacaataaccattacctaccaacaacattttcaaataatgaactgaatgatggattccgtcaaggaaattgttcgtggacagtttgtttacctcccaaatttcctttaatctcatgctttctccatcatccaaacaatctaataccaatcgttttctctaattgcataaaccctaattgttgaatcctttaatcttgccttttcacattgcccaattcctttagtatgatattttttattcgataatccctgataagtaaattcactaatctaatttcagatggattgttgtagagattggggaattgaagattttttgccttctttgttcttgtttacaatgaaggatgaagtttcatggaatattgaagagaaatttgagaaaagaaagaaagtgtgggctttactgacgacaaaaactgtcattttggtggtttttttcactaaggcatgtttggcactagcgtttaaggtagcggttagcgatttgacaagatcaaaacgctacttaagaaaatgatgagtgtttggtaagatagtggttgttgtagcaggtagcaattagagtagattatgagtagcggttgtggaatgttactacaagtaacgtttgagatttagaggtagcagtccagcaaagaaacattgtataatagcataaggtagaattaattaaccaatgtttttttatttctttttccttttattgtttattaataattttattttatgccaattcaatgtttattttacaatagcaaaaatgtaatttaaatatttattttaaacataataaattttataagtattttagtaaaattggtaatataaatttttcgagggttgaatattttcttagatgtatacatttctttgaatagttaaaaaatcatatctcctttttgtgtaacttctttgaaaaataaatcttgaatttaactattgaacgaacatatgaaattattgtagttcatttcatattataataaatgttaggtattgtcttttacaatttcaactacttttggcaaacaattctgattaaacagctattttaatcgctgatcgttgacagcaaccgctaacagctactagaaccgctacttttgccaaacatgcctaaaccaagtaatatcggggattctttattatataaaaagttaataatgtgattatttgaaaaaaaggttgactttatatgttgtttaaagaaaaaaaaacatttattaatagaaaatatactatataggtctctatatacccagggcgaaatgaatgtgtatcttttcaaatgagtatgcgtacatgttctgtaaatgcatatttcatatgagcataatgtttttactattattatgcacatttgtgttttaatttttcaaatgagtatgtaaggaaaacatgtattcttggcatgtcagtgttagtgatttttgttgttatataaatgttttcgtgatttgtgaatgtggtacaaacattcatgtgccatggcgtttagcaaaacttttctagctcacatgatgcttcaagctaattgcaatgaactaatataagggagaggacattttacgaattagttttacattgatagtagtttgaagaagatagtttaggagatagtttgttggaatagaagctatgtgttagaattagttatagtcatcaatttttgaataagactcattattatttcaatccttctaccttttaattactagtccaactctcactctttggtattaaattacaccattcctacggactatctaacaactctaaccacggcccatactttttcttcttaacataaaataatattacgcttactaactactaactcctatgacatctaccttttcaataaaataacaattgataactatataacaacttataatctaaaagtaagtgtcttgataagtgtagagtattgtgggacgaagggagtaattcatagcaaatactatcatagcaatacaatactaggagactaagatgtgagttttgaacttcaaaaaaaaatatacgcgacatagttcaccggaagaactgcagcacaacaaatgcaaatggggattaaatgaggagttcacctacatcacacacaagagcgattgaggattttcagatctggaagaagagcgaaaaatcaggcgagagcttcaactttcggagtttaatggaagagctaatgatgattgaattattcagttggatttatcttttgtaagatgaggggatgaagttgaagattgccataataacccttgagggcgacacaatggtggtgggaatggaaatatggaccacgaccgatttatgagtggaaagaattgaagtctctgatacaatgacgttttggtatatcatcggtgctttcatggctgtcagatctaccgaaaggaaaagtagtggtgaaaacaaatgtcgttcaaaccaaccacctttgactttcaatattgaagtgacaaggaaaactggcaccttagctagtgacttggtggagtctttgcgtaaaccggtggaaaagaagcttatctttgagttttagtgtggtcttggtgcttgtttaagtggcttgactatttaggaggaaaaaaatcaattgtgaacaattggtgagtaacctaaaaatcaattgtgaacaattggtgagtaacctaaaaatcaattgtgaacaattggtgagtaacctttaaaccagactcaagagtgggaaagaggcggttagacaagtagatttagaggaagaggaggtagaaaatagattagaattttttttgggagttttcaaatgtagtggtatcggctcataacaaggtggtcaaatggatggagagcttggtcgtttgagtagtctcatggtggtgattataactacgttggcgataaacaagttcgctttaccaagaagttgattggtggaagagagattttcataaagaggggctcgtatagcaacagctttgtgtggtctcagtttcattgtcggcaaagccgtgggtggtaaatatggtgattttggagattgttatgatggagggagttatggtggtttcatgagacatggatgctatggtggtgctgtgatcggtggagaagaggagctcgtgaaaggtcactctgatggagcgggtgtaatggtggtctaggttttttcggcatcggaggttgcgtatctcgtgaaggttcacatttgtacaccggtgaatactatggtggtgaactaggatgacagtcaaggtgaccatagtagaaaaaaaaaacataaaccatgtagcttagatgatttgaaaaaaaatcatgtttttggagaagaatcttaaatattatgacagaggcaaacttgtcattgaccaaatagatgacatagcaattgcacgtgtctcgttaaaatttgaaaccataaaaaattcaaattgcacttcatatgcctttcttttggttgaaaacttcatataccctaatgcgtcaatatggttctttttccaaaaaaaaaagtaaattatttcggcgttagtaaaagcaggtccacctccataatccattttattaagccaactcctctaccctacttttgcaacctatcatttcttattttctaaaatcatatcaaaaaaacaagtgtgaacccaaaactaactatattatacctaagtctaatttcttcatccaatgtgttcaaccccatttttcaacccttccactcataaacccatcttctttcactcctaaaactttcagctcacgctcgtatcacctctttactcacatatcagcccaaacgatttcttattgaatccactaaattatgtatatcgattttttcaccaagtactccgagttttcaaaaaatttacctggtacccccaagttttcaaactacacgggatacccctaagtttcaaactaatacactcagatacccttaatgactaacgacattaatcgccgttagtcattaaccttaattttctagatttcaacctaattaaccactaaccctaaccccaaccctaaccctaataataaccctaaacctaaccctaaccacccctccccaaccctcccaccacccctgccccccatcctccactcctgcgcagccagcaggccccccacccatttgattttaaggaagaaacacgtatcagggaagggggagaacttagctctgacagcggcaacggaccaccgacgagtctggactgtaggacggcagcgtcaaggcgcgagccggttgggctactgcagttcaaagcaaacaggggaggggaatcgagccgagaagagagctaaggaaagaggggtgatgggcgttgcggagatggtgcgcatagtggtggtggtgtgggggagctgtggtgggggagaaatcgaatgggtgggggagagagggtggggggctgcggtggggttggggctggagggggtagggtgggtgggtggaggggtggtggttgggtggtagtgggacaactctcaaacatgattctttctcaaacatgattctttctcatatccttttttggatttccttaaaaaaatccatatccaaataacgttgaccggtgagggacaactctttaacactattctttctcaaatcttatgaaatcttcacatttaactcgatctccctttcaatgaacctaaagatatatattaatagagttgcaaattcctaaactctagaaaattcaaatacaacataagagtcctagattcttccacaagatgtattatatctttcaaagtttcccagataaaattagtaattaggaaactccttaacaaggatacttaaagttttatctaaatcttgcataaattgaaatccaaccataattatgaataaataatcataaagaatcctaacataaataactagaaaataagataataaagaagcaacaaaagaatctcataaccaccatttgaatcccgcatgagaacccaaatagttgttgttccttataaaaacccaccacctttcttcgggtattatgacggtattggactatagtatgagacgagatctcttaatcaccaatcaactattgtaaacttgtgagcctgaataatttatttgagatacaattctaaggttgtttatgaacgtgtttggtaaaattgttattgataactcgttcgtggaaaataaatgcaaaagtcaacatgccaaaaaaagtgctaaaatcaactttcggctttgcttgaaatgttaagttttaagctatccaagagccattagtcaaaatctattgaaagcgtactcaaaaaccatttatcaaacacccctacaaatccctttagaaaacaataggagttgtacaatataagtattgagttataaagttgatcaagtgatttaggaggttgttccaaatcaatctacaagagtttgtatacttataccccttcgtttttttaattgttacacttaggccttgtttgacaaatagagtttagcggttagagtttagattttgctgttagagttttaactttttgttaaatagatttgactgctgatttgacaacttcttcttataaatgtgtttggtaattattaacagattgctaaaagcttattaccctttatttatgtgaaatgacatgtatagacattttaatccacatgggtattattattattattattcgaggcatacaagtcattgaatatatttttacctaatcctctaaagaaaaagctcctattaggagctttttcatttcgagagtttttattccagaactctcttcaaaactcttttttaccaaagaataggagctttttcatttcaagagtttttactccagaactctctttaaaactcttttttaccaaacaccccttttagagtttttgactagtcaaaactctaaaagtggtccaaatttctcttttaactccaaaactctaattgccaaacacccccttacacttttcacgcataccaatgcaacactttgacgattaacatctccagttttttatttgtaaaaattataaagagtgcatattaataagtagggctgttcaaagtgcggtctggaccgcaccaaaccgcaacccaaaccgttgtttcgcggtttggtttggtttgcggttttaaaattgcggtttgggttatgatttcaagcaaaccgcggtttgcggtttgggttgggtttttatttttgtaaaccaaaaccgcaccgcaaaccgcaatgttacattttttttaaaaaaataaattaaatacatttatgaaggtgacatacaattataaaattgaaaaaagaagtttgaggtaaaaaactttaacacttatgataaatcattatatatgtttaattatgaattcagcttcatatctatttggactcttattaacaattttcttttaatcttaggaaacaaaagtaatgtcgcggaggaaataatggttaaaccgcaacccaaaccgcaccaaaccgttttgcgcggtttgggttgggttggtttgggaaaaagtgcggtgcggtttgggttggaaaattttcaaaccgtatatttgcggtttgggttgggttacatcccaaaccgcacaaacccaaaccgcgaacacccctattaataagatacatattaattcgaatttgacaagatccacatgactatgtttttattcgcgtataaaccacaaaagaaggttcaagtaaaatttgtgtatggtgtaacatgtcaatcaaagaacggaggtaatatttgtcaagacactttagtcacttctaaattcctataaacaaagaaatatggaagaaaactggtgatgaaaattgaaaaggtgggtataataagagagacacaattctaaaataagaaaatattaataataaaataataagttacgataggcctcatgtttgaaaacggaaaaaataaggagatagttcgtgtaaaaaggagggagtaaagggtaatgcatactttgtattgcaagcttagttttaaaaggcataagacgcaaagcgcatcgaggcacaagacgaaggcgcatgcatctcgtagttgaggcgtgtaatgattttacttcacaaccacctgagcaacccaatacagaacgaccacaagaaaaatagaaagaaaggaaatgattttgattgatcagcagaaaatacagagcattcgagaggctcagtctctcccaaggactacaagatactactaaatttcacacccccttcagtccccttacacccttatttatactacttctgctctcctattttaacggctactgacattctctgagctggcctgctattcctctttttgtgctgacatttctgaatattctgtggtagtggctccattctcacatttggacaggtttacccctccatttctttcgtgcatacgtcagccacggtttggggattgaattcattacattaccctgcccccaaagactcaccttgtcctcaaggtggaaggaagggaaacgttcttgcaccaaatctgcatcttcccacgtggcttcaaaaggtgctaagtccttccatttcagtagcacttcagtctgcgtatgcctccctctctgtgtctgacgtacgtccaataattcttcaggttccacaactagttccaagtctgctgctagttgagttggtacagtggttgctgcctgggcatctccaattgctcgtttgagctgggatacgtgaaatataggatgtattttactggtgcctggtaactggagtttataggcgaccttgcccaccttttgcagaacagggaatgggccatagaagcgggctgccagcttctcaaatggtcgcttggccaaggattgttgacggtatggctggagctttaagtaaaccagatcccccacttcaaaggactcatcgcgccttcttgtgtcagcataggctttcatcttttgctgggagcgtagtagatgaaagcgtaaatcatcgaggatggcatcccgttcttgcaacacttcctctaagttatctactggcgtttgccctctgcctactcgccacaagtgtgtgggtcacgcccgtacaacaccctgaatggagtcagcttagtagacatgtggggagaggtgttgtgtgagtattcagcccaagggagccactttgcccaagtcttcgggtgccccgccacgaaacatctcagatatgtctcaagtcctttgttcacaatctcagtttgtccatcggtttgcgggtgataggcggtgcttctccttagtgttgtcccttggagtcgaaacaactctttccaaaaagtactcagaaaaattcgatccctatccgaaacgattgatgccggaaacccatgaagttttacaacctccctgatgaaagcttcagccacttgtgagagcactaaaaggatgacgaagcccaatgaaatgcgcatatttcgataaacggtccaccactactaagatcgtgtccacccccttggacaagggcaatccttctatgaaatcaagagtgatatcctcccaaacctgagctggaatggctaagggctgcagtaggcctgctggcttttgttgagagctcttatgctgttgacaaatgctacatcgctgcacgtacaatgccacgtgcttcctcatacctatccaataccactcagccgccaacctaaggtacgtttttacttcacctgcatgtcctccttctggggaatcatggtaagctatcatcaacttaggaatgatgacggaagtgttgggaattaccattcgccccttataccgcagcttgccatcctccaccgtgaaccccacaagtggtttatctccctgcgccacttcttccctgagccttttaaggaaccaatcctcctctacctctttttggagctctgcccagtccactccttgggttgtgattatggtccctagctccatttcacctacagtttttctagaaagcgcatccgcaaccttgttggttgcccccggtttgtagtgtatttcaaagtcaaacccaattaatttgcttacccatttctgaaaatcagcccccacttcccgttgttgtgtgatgaaacgcaaactttgttgatccgtatggatcacaaatcttctccccaaaaggtaatgtttccatttctggaccgcaaggcatatggcaattaattccttctcataaacggacttgtgttgtgctctcggtccaaggagcttgctgtagaatgcaatgggcctgccctcttgcattaggactgcccccaccccatacccagacgcatccgtctcaactacgaaaggcttatggaaatcgggcatagcaagaaccggtggctgggtcatagcttcctttaagtgagagaaagctgaagtagctttttcggaccagccaaaggagtccttacgcaattgctcggtaaggggctgggcaatttgcgcgtattgcctgataaacttgcgataatacccggtcagccctaaaaatcctcgaagctccctcaaattcttgggaacttcccactccaccatggcccttatcttctccatgtctactgccaccccatgctgcgaaatttacatgccccaagtaggccactgtcttcctccccaagtcacatttcttctggttagcgaacagtttgtgcaatgctaacagctgcaacaccaatcccatgtgtcgtgcgtggtcctctttggtcttactgtagaccagaatgtcgtcgaagaagaccagcacaaacttcctcagatatggacggaaaacgttattcatgagtgactgaaaagttgctggggcattggtgagcccaaagggcattacgagaaattcgtaatgtccttcatgggtgcgaaaagcagtcttatgggtatcctccgggcgaactaaaatttgatggtatccggccttaaggtcgagtttagagaagatggtagcgccatgtaactcgtctagtagctcatcaatgaccggtatcggatacttatccggaaccgtctccttgttcaaagcccgataatcgacacaaaacctccaagaaccatcttttttcttcaccaataatacggggcttgaaaatggactagttgagggcttgatgatgcctgcctccagcatctctcggatgagtctctcgatttcgtctttttgaaattgagggtaacggtatggcctaacccccaccggattactgccttccttcaacgtgattgcatgctcatgccccctctttggtggcaggcccaccggagtatcaaaaacttccgcaaactgactaattaccttctgtaaaaattcgggtacttcttgtgcctccttcaactccgcttctccccttttcccatcatcctcaatctggttgagctccaagagaaaaccccctttttcttttcggattgcctttatcatggctctaagtgagattttagatcttgctaaggaagggtcccctctcaatgtcaccactctgccctccacttcaaactgcataacctgagttttccagttggtaatcactgaccccaatttctcgagccactgcactcctaatattaaatctgagttacccaggccgagaggtaaaaaatcctctgttacttcgatttcccccagctttaaagtcaccccttgacacaccccagtaccatggacagcttcaccattccctaaagacactccaaatccccctgcatctgagatgaccaactcaagttcctcaacagttaacaaggaaataaaattgtgagtggcacccgggtcaatcatgaccaccacctctcttcctttaatttttctagtgattttcatcgttttaggactcatcaaaccaatcacagagttgagagatacctcagtaggaagttccggtggtggttcggacggtggtgcacgagctgcgtcgctcacctcttcggtttcttcctcctcgtcatgcatcagaatcacgctgatctcttttctccggcagatgtggccggcggtccacttatcgtcacatttatagcacaacccttttgctctcttctcttgatattctttctcggaaagtcgcttgaactctacagatttttttccttgccccccagcaattggatacgtgttcaaggtgttggaatttccccctgggttttgggcccacattttgctggcaggtgggttgaggctggtcgttggattgaaggaagcccctacactccttgtcattccccctctgttataaatcgagtaaggcccattcttagttggcccacttcttttataacccacaatcctattcctttcctcaattcggcctgctagttccattgcttgctctaggtccataggattgagtaacctgacctccactttgatatcctcttccagcccattaatgaactgacccatgagtatttcttctggtactctactcaacggtgccgccttctcaataaaagtgcgtcgatactcatccaccgtggtggtttgctttgtggccaaccaccgttcccacaatgaaccatagtgggttggtcgaaactgacggaggaggtactccttcagatctgcccaccaccttatcggccgccttttattctcccactggtaccacctgagggcatccccctctatagacacaaccgccgcctccagggcttcactgctactcaggccataaaacgaaaaatatcgctcggctctaaggatccacccatccggatcggacccatggaaaatgggcatctctaactttcgatatttccagttccccccggaagtcgaacctcctggccctccacctgagccgccatccccatacgatcggcccccgagctggaaacctccatattcgtccccttctcggccccccagatttatcaggtcaggagccctccgttccggcggtcgggggtgtccagtgacggtttcgggtgtctcccgcgagggttgtggcaaggttgctcggatttcaacctgaaatttcctctgttcagcacgcaacccttgaatcgtcccatcctgtgtctcccttgaccggttaatccggtcctccagcctaacggccaagacctccatctcctcgcgactcttcctcgccgcctcattctggccttccaagatttgagcggtcaacgattcccccatggcattaatggcagattccaccgccctggacaccatggtggccactgacccttcgagggctgccattctttcttctaatgaatccaccctctgcacttcgtttcttggtgccatggatcgatgctctgataccaagtgtaatgattttacttacttcacaaccacctgagcaacccaatacagaacgaccacaagaaaaatagaaagaaaggaaatgattttgattgatcagcagaaaatacagagcattcgagaggctcagtctctcccaaggactacaagatactactaaatttcacacccccttcagtccccttacacccttatttatactacttctgctctcctattttaacggctactgacattctctgagctggcctgctattcctctttttgtgctgacatttctgaatattctgtggtagtggctccattctcacatttggacaggtttacccctccatttctttcgtgcatacgtcagccacggtttggggattgaattcattacaaggcgcacctttggtaccaagagacttagacatcaaataaagaagcattgtaatacttagaataaacattgtttttatattctaaaacacatattttctctaagacacctagtaatctcatagtggatgtcatctagtttaggtggtaaggttttattgagttggtactcaagacctcagacttagaggtggcaaacggatcatacgggtcgggtgaaaatgagtcgggtcataatcgggtcacctttgtgtccaggttacggtcaggtcgagttcgttcgggtacgagttcatattgagtccatgaggtttcatgtcatatcgggtcgggttagattggatttacaatttcgcaaataaataaaacgcatataatactaaagagagtaaattaaataattaacggacactagctaaatcatatattagtattttatgatgtattttccttaaatttatttaaaaaataactaatatgacaatttttcgggccgggttcgggttgtggtcatcattatcgggtcaatttagtatcgggtaggctcgggttcatgtcatattcgggtctattttaattcgagtcgggttatttcggatttaagctctatttcgggtcagtattttcgatgaagaacgggtttcggatcgggtcaccggatacggatctattttgccgagtcagactgcttttcaaacctaataatctcagtttttccacctattcagatttgcctatgatctctatttagataaatgagtacaatattgtgtctatccatgaaaatgaatatctcacaatgtaaaaggatatctctaaatttcactaatcactctatctgttttgaataataatattctattttattgcatgtagtaaagatcgagtatttagtgagatttggagaaaagaggaggctagagagaaactaggatttagagaggagaagggggctctgtaacacatacaagatagatactcttttacactaacttttcaagatactcaacatataaaatcagcatcatcttccaaacaacaactttaagccacccatgaatcttaattagataataaaacataatcgtgaatcatctatcctttgtttggggggatcctaaagcaattgaggaaaagctttgatgcaaatatcaattgtgtaaaaaagcaagtattcgttcgtgatgttgctatactaggttattttttggatccaaaagtcattcctactagaatcatttaggaaaattgtcagtatgaattttaaattcaggttataaccaaagataattgaaaattgtcaaacttttcaaataattccgaaataaacatgtttgtaacatggataaacttttcattgcttttcaaataattccaaaataaacatgttataacatagataaccttttcagataattccaaaataaacatgttgtatcatggataaacttttcattgtttctagtcacttaaaattctaaaaaaatctttcctccctactgttactctctctagcaccaaatctatcacatgagaaggcagaggttttcaaaataaaccgttacttaatttggtacttatttcttgatcggtgttcatatcatatgagttcctactctatatctctctactcttctaaatccttgtgtcacttcctgtgtttcataaataaaaaggaggaagtattagttttgaaacgaaaggagtatggtgcatacattgatagaaaaaagaagttatttgtccttatttcactcatataacaacaccaaattctgtattgttatcacaaaataaaacttggattatctttgtttcatagcccaaatttagaattagtttgtcagatttccaatcatctaattacaatattagagctagacctaggacaaaaggtgggtttggctacttggtaatagctatgtctagtgctaggatatgtcattgtcgtagaaccatgttatggacatcttaagaaacaaggttaacctaattggttggagatcctactttcacttttataataaagtttcgattcttgcctatttgtaaagtagaattcctaaatttcccttcactgatatttatcttaacataaaaaaatgttataaacattgggattgtatataagtcaaaataaattgacaatcttggtaacaactaagttaacattaattttataagtaaatgattaatcccaatataatctcttatttagtaaatgagacaaacttgtacaccttcgtgttagactcgttaatgttcgctaacaattcattcagtagtcaacagcattttaaatttgaaataagtgttcttgtggtttttgagagatcaagcaagaaaacatgtctctcccctttgaccaactaattgggattaagaatactagttttaagattttaagaatgagttatagtctttcttagaccgctacaatccccttgttgatatgaaccagatatattttgtgttcaaatagtagatcaatgcattgttgataatcctttgttaatgtacttgttgatcttattttgtacttttggtagatgcgctatactttctttcgattgctcattttgaactcttaactacatatgttagtttaagtagatgatttagaattgctatttcaatcttcaataagcaatttaagttgtcaaaccttgtttcacatcattagggtgaaagttatttggataaagacctatatctaattcaatccaaagcaaattagtaatgcggattggactcaaactatgtttagattggattcgaattgagtttcttttctttttcttaaaaaaattggattttccgatcgaattgagggtgattagatccaaaataaccgaatagtagataggatttgtgttgtatattagaattgggcttaaggatttccattttaacaaaaaaaccaaatggtccgactatcaaaaactataatttgatagtcatgcctatcgaaaactttattttcattctcgcacctaattatgggcttgtataaattagttctactatcgaaaactaattttgatgctcgtgcctaatttaaattttcgaaaaaatgaagttaagaaaattggatatttcggattggatccaatatatcttgtgaattattaatttggattagtttggactcaaattcttattggattggattcaaattaaaagattaaaattcaaattttgttcgaatcaaattggagtaggcttaagtttaaatcatacaccgaactttcaccactacccatcatgcttaagcttctaatgtaagagagtgtttgggagttgagctcgaacaactaaatttctaaaagaaccaagttcaaacaagaaatctaaaagctcgattaaacttgagtcaagctcaaacacctatattccttattggagcttgactgaagattgaacacttattccttattaagctttacgctaaaacattgctcgactcaactcttctacatccctatagttcaaaagaaatagttgtgggctgtggtgctcttgtagaccaacgcactagtttaacaaagctaagtgcctgactgcaattccatacacattacgatcaccatgacctagtttcagctcacactttggaagtctaatttgaacttgttctctacctccaattcattgtggggtaggaggcgatagttaagggatcaaaatcttatgatataacttgcataggctatgccactatataatgcgtcttgtgtcccatattagtttaatcaaattgaaatgttttaccatttatatcttcaattatgtatggatactaatatttgatttgacgtttgatatgatattaaatgtggactgttattcttgatgtgcttgagaagcttttttggggccagttagaaactatattccttttatggtcctaactaggttgttgttggtgtgttcccaaataacagcatggaaaggatactcgagcgctatgaaagacactcatatgcagagagacaactgactgctccagatcctggatcccatgtaatccagctaggcaactatcttttctaagcatttaaatcgttgagatttcaattttaaatgtgttttaactgataattcatgcattatatgcttaggtaagtttgactctggaacacgcaaaacttaaggctaggctggacattcttcagaaaaatcaaaggtaataagatccagaccaaatataatttgtataataaccaccttatgaggaaaatttaagatccttgataatttcaggcattacatgggagaagaacttgataccttgagtctcaaggagcttcagaatttagagcatcaaattgacagtgctcttaaacacatcaggtcaaagaaggtagtttcacagttgcattagatcatcttatggatcaattggatcacttgtttgtattttagcgttgctcaacacggtcgtctaatatagtgtgcaaaacgacctacagggcaacaccttttatagggctcgaaaatacgaaaaattaaatgtttgttttagtcatattgttcaaacccaagctttatcttgtcaaaaatattttataatgattattttttagaatacattatttacatttttgcaatttatgcataatacttctaaggtccaactttataattgaaatagaagtccttaaattttaaagacgaccttgaggaaacctaatttcttctcatatataattaaatcaattattctacaagttagtagaacaaatactacaataacaacaatattgaagccctaatctcagtaggattggattgattgtatgaagtcttattagtggccgttaaatgtttcttgtaggtcaagatgacatggctcatatagtaaggttacttgactaaaagacgaggatttgtttcgacttagattttaacaagtttccctcatttgttaacacctaagcgtactaaatcaaattctaggttttactcactcaaatttccgatttaggaagggcttgaggatagttgtattatcgtaactgactaatcaaaggagcctctcttagatcaggtttcacttgccaattctaacaacttgtttggtaaaaggaatttggaatgaaaagaaaggaattgaaaagaaacattctacttttcaatgtttcattcaaaaataacattttaagtgataggaaatggaaagaagtgaaacgaaagcctctttacaaaattatcatttttctacccccccccccccccaaaaaaaaaaaaaaaaataagtagtaagtagtagaagaagaaataaataactaacaagagtagtaagtttttacgttttctttctnnnnnnnnnnnnnnnnnnnnattcaaatcagaactgaatagtcataaccggaagattagtttctctctagcgtgactagggtttgagtaaaaagagaaaacttaaatcaaacatgggatattaaggttttttttcctttcttcagttcttttctcttcccaatcctttcctaaaaatgaaccaaacaggctgcaaggttttcacttgcttaacacaagatttatttttaaaaataattacactccaaacttttaagcttaaaaccaattttaattcaaatcagaactgaatagtcataactggaagattagtttctctctagcgtgactagggtttgagtgaaaaagtctagggtttcatgtcattcttcttgcttcgagtcccttcttgggattgttgttagccattatggctaccgaaatcgttattaaatgtctaaatcttagaattactgctgaagaaaacaacttggtgtttctcgaagatgttgatgataactcgcagcaccatacgctcgcactggcgattgttggaaaggttctttcgtcaagaccatacaatttcgaggcacttaaatgaaccttaaactagatatgggtgatatccaaaggagccctacttcaccctattgaaaacggactttttgtggtacaatttgcgacaattaaggaccgatctaaggttctagtcagcagaccatggaccttcgatataaaccttgttctcttagatgctattgaagggggtactcaatcttgacccattgcccgttttggactcgcttgtataaccttcctatggactgccgatatgagaagttcatcaaaaactattgttggtgtattgggggaggtattggaagttgattttgacaggattgtttgggataaatctgcaagagtaaaggtgaagattgacattacaaaatcgttttgtcgtgtgcagatgatcaagactaacaggggtgaggctgtgatgatcaatgttaagtatgaaagacttcctacaatttgttatgtgtggaattctggccatattgaaagagattgtgtgaagacccaggaagaagagaaacaagtggagagacaatagggggtcttggaggcctctccgcgtaggggacgattaaagatggtgaaagagtcgaaagccttccttcagtgtgctcgtacactccactttaataacaaggaagaagtaaggggtgaggaaccacgggattatgtggagccgaggggttattgtcggctatcttagggggtaaaactttggtggtccaggagatagtggacggctctaaggatgccatcgaggaagttcgtgctgaaggtgcaccactctagcccccttgtaccctttgggtaatgccatgctaccttttacttttgctgttgggagtgctaatcctactccctcccaccgaaaagttaaaattaaaaacaaggcaagggttcagggtgttttgaaccaagttaatgttgtgggtgttggggggttggctaataatgggggttgtgagaaaaggatattccccaacccgatggtgttagaaaaagaaaaggggttcaatgaagagggtttaagatagcaaaacgagaggattgtatgtaacctatcagtagggaggtaactattgaggtggaggtgggcgagacccaaccccgcccgacattatgaatatcctatgttgcaactgttggggattgggcaacccccgggaagttcggatgcttcgtaggtggagcaatagtgctacactgagttcggtttttatttctaaaactatgattagtggtcgtgatgtggaaagggtgcaaagcgggtagggttttgattgggcaattggggtggatagcgttggaacttcaagagtttggtgcatttattggaaagctggggaagtggactttactctagtctctctatcaagtcatcatatttgtgggaatgtgaagcttgttgatgggaaggtatgatgcttagtgagtatttatggttgggcggatacaattcaaaagtataaaacatgggagcttatgcaatcctttcactcatatcatgggccgatattgtttggttgggacttcaatgagattttgacaatcggagaaattgaaggagggtccgaaactcaatgaagtaacatgcataattttctagaaactttagatgacatgaagcttagggaccttggctattcgggaacttggtatacataagagagaggctttaagccacggaagagaatgagggagaaacttgatcattttgttgcatcttcatcatggtgtgacttctttccgaaagctacagttgagcacttgatgcgctacaaatcggaccacactcctattttggttcgccttgtaggccatcagtgaagacataagaagaaaaagacgtagttttgttttgagactgcttgggtgcttgaggaaggttgtgaggcccaatgggtgagtcatgggccgggtttactcgcgaggtatttatcgagcgctttaaagccgtggaaggtgggttcaaagcaaggagtgatgggtctcttagtaatctgggcccgcgtgtgagggagattgaggaggccattatagatgggaggcagcgaagcagataaggactatgaggctctatgagactcctctcccacgaaagttagacgaggtgttggacaagcaggagacgttttggtttttgaggtctcgtgtgagttagataaaggatggtgatcgtaatacacaatatttccaccacaaagcttcccaacacaaacgtcgcaactacatagcggggatgtatgataataaaggggtgtggcaagataacgaagaggatattgaagggaatatttcagagtattaccaaacctcgttcggttcgtgctccccctctaggaagaacgtcgcggttgtccttgaggttgtgagcccggtgataactgatgatatgaatatggcggttatgaaatcttacactaaagatgaggtgtgggaagcactaaaccacatgaagcctaacggaatgcatgccatcctttatagaggttctggaataccttggagatgatattacatctgtcattttaggtattattcatggcacccgaccccagatgtttttaacaagactaatattgtgctcattcctaaagtcaaatccccaaatcttgtttctgagtttcgcccgattagcctctgtgatgttatctataaacttgcctcaaaagtacttgctaacagattaaaacaggtttgcctgacattgtttatgataaccagagtgcatttgtgtccggaagctatattacgaacaatgctttgatttctcttgaattatttgactctatgaaaaaatgatacagagctaggaaaggttttgtgtcgatgaaattggatatgagtaaagcctataaaagagttgagtggtgttttttcagtagtgtgttggagaagttggattttgctgaatcatgagtgaatgttgttatgagatgtgtgtcttttgtgcagtactcttttgtggttaatgataatatatgtggagctctgacaccctcaagggggctttgacagggagaccctatatccccgtatttgtttatacttgttgcagataccgttttagctcttcttagcaaggcattcaacaatgcgtggctatacttgatattctcaacaaatatgaggcagcatcaggctagaaaataaatattgacaagtcaggaatctctttcaataaaagatttgacgtattttatggccatgaaacaagttgagaagcatcagaaagacttggtatcccaactttggctaggagttcgaaaaaagtcatatttgctgacattcaagagcgaatttggaagaagctgcacggatggagagaaaaacttctcgcgggcttgaaaagaaactctcttaaaagttgtggttcaagcaattctaacctatttggtgggcgtttacagattcctaaccagtattatccaggccattcatttggccatggtaaagttttggtgggggtcgaaaagggcccacaattcgatgcatctggggggatatgtgctcaccaaaatgtttaaggagccttagctttaaagacttaggggtgttcaatgaacctaaactaaggaggaatgcgtggcatttgattcctgctggtgagtccctttcgggtcgagtgttctcggccaagtactattcgaagtcaacctttttggactcatttctaggtccggtaggtagcttctcttggaagagtatttggggggccaaggcattagttaagggtgttttatggtgcgtaggcaatggcagacaaatcaacatatggcgtgactcgcgggtgttgaatggtgatagtaggttcatccccggagagcgcgtttcaggccttgaggatgtttgtgatctaatagattttgcacaatggagtgcgatgtggaccttgtcacgattgcttcaatgaagatgatgctcaagccattttagtcatacctctaagtaagcgccttctgaaggacatggtctcttgggctttcactaaggatgaattttttttgtaaaaacaacctatatggccggttggtcgaggaatttgaatttgtttcacaaagcatggctgcaaatctggggccttaacgtgtctccgaaggtctgccacttcctttggcgtttatgctcggtacccttcctgttcgagctcttttaaaacgacgccacataactgatgatgattcatgtcctttgtctaaaggagcccggaaagcatatcacacgcgttgttctattgcccatatgtagccgaagcatgggagagtgcgggcctcacaaattgtttgcctttgtttgatggggctggtatgcttgatgcgtggggggagtgggaaacaatcgatgactagtcccttgtaagacttagcttcttggcttatcacttgtggtttaggcgaaataaatgtgtttttgaaggggtggtgagagcgaatgagagtgttgtggaatatgccactaaagctactgttgatcatggtttgtatagtgcccgcatttatggtgggtcgaaggctaccgcatccaaaagctcgaaggtatgggttccccctccagcttgtcgtacgatctaaaggttgatgcatcagtggggaatggtggatgggtggggctaggagtaatcgcctgaaactagaaaggggaggtgctcgtggctgcaactaggagggtcagagcttgtggcccgtggaaatggctgaagggaaggctctttgtcttgctcttaggcttgcctcgctcatacaacttgcaagaagtgatcgtggagtttgactgtcaatcttggtgaaccatctctccaagggtgctatttactttgcatttttaagtcaaagcttgaaccttgataaaaaaatcccgttcgacatgaaaagtgccttgattttgcgggtttgggagtgccttattgattctggggtttgatttgtaacacctttagtaaaaacatgtaagctaactgtaaaacgaacattaatcaaactaggatatgtaaaattcctaaatcaagaagaatttccacttgtgctgaatttgtccaccttgcatgacacccaataaaagcccatgtctcctagaaccccttatgccgccttattcatcttttctcaagttgagttggagtcctctatggtccactcgacttctttagcacactctcggtaaaaacttttaatattattttattttagactccaccatcttgacatttattccttcttaaacttgcttcacacaaacatctaacactagaattctatatagaatagcttgaatctctcttaggataaccttatagtaaatgcaactacgcctatccttaaacctttctaagaggagctttatcgtatttacattcgcttcactttgaaacgtcgctaagtgtatgttgcactttccaaaccatgtgttagctaagaccaagttatatgactgcataacctaaatagtcttcctcgagaaaattcactagttggatcggaagagtttgtgtaaatctatggcggcgcgggactgggccttcacgatttcaagtgttttaatgcagctcttctaggtaaacaagtttcctaatagcgtggtgactcaaatattgaggacttgttgttatactaatgctattcctggcggcacttaaggggtgaaataggtggtacaaaggagtgcttgatggcgtgtgggtagtagttgaatatatcagtatgatcaagtccatggatccctcgtacttattcgtgcaagattatttttccacgaggcaaagcgagcgagaatcttaaggtttatgatcatattcatcttgtacgtgctaagggtaatgtccctttcaataatgagctatttctccttttgagcaagagcgtatcttaagcattcctcgtagttctcgtctccccaacgatgttttatgttggaatctgaatttggagaaagacggagacttttcgttcggtctatcgagccattcttttgagttggatggcgagagcgtgatttcatcgtcaatacgctctaatttatggagtataatatggcaggatagtacctttcaacgtgttaagcttttatctgcattgtcgacacaaaggggattgagtaagcctgtgccgagtatggaaccattgtgtaatctttatgcgttggaggatcaatggagctacacttcttacgagactttgttattggaagggcttatatgggatccaactagggtagtcaaaacattggtcggggctgcgctgcaattttggggacttggcaccggcgtttttggagtagctccctcatgtggaacataggcttttgatgacgatatactaggctagatggaatataagagagaggtgtttgtttgaggaggaggtttgtgatccctatcaaaccacatgcataatctcatggcgtagcttcatgtggaacactgacatattgcatgtgtagggttaggtgcttgcctaggacaccacatgggaagagctccgttaagcttaatgtggatggagggtgtgtggaagggttgggtgcgtccactggagtggtgattagggggatggatgaaaaagcgttgtagttgcaacatagaaaggtggaggactgcgaggaaccgttaaaaaggctatattttatggtgttcatttggttgtggaagtcgatttttgaaatatggttgttggaagtgactatcttcacctcgttgaagcaacttcttcaaaagtggaaggcaaaaatagcttccatgttattgttgatgacattgttcatggtagtggtatgttaaatacttcgtcttgtagttttgttcgtagggatgggaatagggtttctcacgaactcccccatggaaatatcataatggctcatgctcataggtaaatgaataagctaacaaaattgttcatctttgcagaaccaactcatgcatgaatcgatttctcagcttcagcgaaaggtagacagctctagagagagcatctagtctcaaaaataccatgagattctgtagtgtcctgacatgttttatatgacaggacaaagcgttaaaggagcacaacaacttgctatccaagaaggtataagttcagcaagattgtttagtaacattgttaatcttgctgattgctttgaaacatgtcttgctatggttaacaatgttgactgaaccaaaataggtgaaggagagggagaaggtgctggctcagcaggcagaattggatcagcaaaatcatgacaataactcatctggctttgtgatgtctcaagctttgccctcactgaatacagggtcagtcctcaataacctctaatcatttttccaagatccaaagtaaacatggtttcataatttaattaagatttttttgaaccatgtctccatacaaccttactaggactaatactactaatttaagaccccaacgataaacaacaataattagccatatctggctagcaccttttggacaacacaccacatgagactcttggccaacttctttgatttccttcagtctgatagatatgaatatcttctgaagagctctttggttcataattattgatttagaaaagaattcagcaaggtgagtcatttggtaaccttaaggtcattatgggggtactaaatcaaagtgaagatatatttaggtggcatcagaagagatgatatagataggttgtatcctgtcgataggttatttggatatgtatcaaaagtttcttttataatatatctatactgattggttgatgtatcaaatatccctacagattgtgaaaaaatcccctacagattgtgaaaatatccctagaacctgtgatgatataagatgtgctccgcatgctttattgaacataatgtattcaattcttgaaatgcagaggaacaagcagcagtgcagtggaagatgaagcaacacaaccaccaaatctaaacagcaactctgcacaaataccgtcctggatgcttcaacacatccaagagcagtaa

SEQ ID NO: 4 - DNA, 735 bp, Artificial Sequence
  BvFUL cDNA
atggggagaggtagggttcagctcaaaagaattgaaaacaagatcaaccgtcaagtgaccttctccaaacgtcggattggattgttgaagaaagcgcacgagatctccattctctgcgatgccgatgtagctctcatcatcttctccactaaaggcaagctcttcgagtatgcttctgatacctgcatggaaaggatactcgagcgctatgaaagacactcatatgcagagagacaactgactgctccagatcctggatcccatgtaagtttgactctggaacacgcaaaacttaaggctaggctggacattcttcagaaaaatcaaaggcattacatgggagaagaacttgataccttgagtctcaaggagcttcagaatttagagcatcaaattgacagtgctcttaaacacatcaggtcaaagaagaaccaactcatgcatgaatcgatttctcagcttcagcgaaaggacaaagcgttaaaggagcacaacaacttgctatccaagaaggtgaaggagagggagaaggtgctggctcagcaggcagaattggatcagcaaaatcatgacaataactcatctggctttgtgatgtctcaagctttgccctcactgaatacaggaggaacaagcagcagtgcagtggaagatgaagcaacacaaccaccaaatctaaacagcaactctgcacaaataccgtcctggatgcttcaacacatccaagagcagtaa

SEQ ID NO: 5 - protein, 259 aa, Beta vulgaris
MGRGRVELKRIENKINRQVTFSKRRSGLVKKAHEISVLCDAEVALIIFSHRGKLFEYSSDSSMEKILERYERYSYAERRLASNDPDSQVNWTFDFAKLKAKLELLQRNHRHYLGQELDSLNMKELQSLEQQLDTALKNVRSRKNQLMHESISELQKKERAMQEHNNILSKKIKERGKNLEQVQQMQWQNQHQHQHQQQPPPPPQNHQVPPDASNFMLPPPIPSLNTGGYQGQFGGEVRRNDLDLTLEPIYSCHMGCFTT

SEQ ID NO: 6 - protein, 244 aa, Beta vulgaris
MGRGRVQLKRIENKINRQVTFSKRRIGLLKKAHEISILCDADVALIIFSTKGKLFEYASDTCMERILERYERHSYAERQLTAPDPGSHVSLTLEHAKLKARLDILQKNQRHYMGEELDTLSLKELQNLEHQIDSALKHIRSKKNQLMHESISQLQRKDKALKEHNNLLSKKVKEREKVLAQQAELDQQNHDNNSSGFVMSQALPSLNTGGTSSSAVEDEATQPPNLNSNSAQIPSWMLQHIQEQ

SEQ ID NO: 7 - DNA, 2366 bp, Beta vulgaris
atgatagaaccgcagctgaaagcatgcaacaaaaatgtgaagaatccggagagcaggaagactgcttccacttcgtacaattctgcttctaggaagcaaagcaggaagggagaaaatcctattcgtgttactccgttaggagagcaatcttctgattttggatgttctagtacttggatatgtaaaaattctgcatgtagagctgttctgtctatagatgatgcgttctgtcggaggtgttcatgctgcatctgtcatcaatttgatgataataaagaccctagtctttggttggtttgtgaatccgagtctgggcagggtgattcttgtggattatcatgccatattgagtgtgcatttcaacaagaaaagctgggagttgtgaaccttgggcaatacatgcatttggatgggagttactgttgttcttcttgcggcaaagtctctgggatacttgggtcagtacttctgttttatgtagtgagatattgacctgaagtcatgcttgttttgatggaagataaataatttaaaaaaaatgttacatgcccaactattacaaggccagtagaaaactatgagatatattaattttgatattactgtggaggctcagttgaatttatatgcttgagttttactcactaatggcaggtgttggaaaaagcaattggctatagctaaggatgctcgacgtgtcgatgtgctttgctatagaatatttttgagttacagactcctcgagggcacagctaagtttaaggacctccacgagattgttgcagaagctaaaacaaagctggaggcagaggtgggtcctatgaacggagactctgtcaagatggccagaggtattgttagcaggcttgctattgctgcagatgtgcaaaagctctgttcgcacgcgattgataaagctaatgaatggctcgccaatgtttctagcattagttcaaattgcaaaggttagaatacatacagcctttattgttctccatttacttggtgagtattctattataataaattattaatttcttttggcataatggtggcagtggatgcacttcctgctgcatgcaggtttctatttgaagaagttacttcttgttcacttgctatagttttgatagatatccccacaccaatgactgattccgtcaaaggctacaagctatggtactgcaaaagtagacatgagacttttgcaagggagcctacatccgtctttccaagggagaaaagaaaaatatctgtaaagaatctcaagccttgcaccgagtacacattcagaatagtttcctacacagaagttggtgatttaggccactctgaggctaagtgtttcaccaagagtttggagatcattagtaagaaatccaccacagtgggctgtaagaaggaagatccttgtgttgagaggagctcctcgaatgcaaaggaacaacataattcaaatttggctgcaatatcttctggattcaaggtgcgggaccttgggaaaatcttgcacctagcatgggcccaagaacagggttgccttgaaggtttctgcagtgctgatgtagaacaatgctgtggagtaactaaatgtgaatctccaaaagatcaccagtcacctccacctgtttctcgtgagcttgacctaaatgtagtttcagttcctgatttaaatgaagaccttacccctcccttagagtcttcaagggatgaagacaacggatgcacgctagagcgtgctactgggcctgatgatgatgctgcttcccatggtgttgagaagaatgggcttgggctagccaggtcaaatggtagtgggccaagtgatgagtctcaagcttgggctctcatccgaaatggagatgtgcctgctgttgattccttggcagagacccgtcggaagaggtcttcaagtgcgaatgaagaaacacatgactgtgacagcactctgataaatggatcgccatttcggatttcaggcgggcctggttctctagacggtaactttgagtattgtgtgaaggtcatccggtggttggagtgtgagggctatctaaaacaggaatttagattgaaattattgacttggtttagcttaagatctactgaacaagagcgtcgggtagtcagcactttcattcaaactctgatggatgatccaaagagcttagcaggacagctagttgattcctttggagatctcatatccagcaagaggcccaggactagtttcactagtaagtttatgtctatagttgttctttgattgagaaattttatgtcttctttcaaacatttctattactcttcttattctgaagttttggactaattttgtcatgctaattacaggcattccttcctaa

SEQ ID NO: 8 - DNA, 2285 bp, Artificial Sequence
  BvVIL1 cDNA
atgatagaaccgcagctgaaagcatgcaacaaaaatgtgaagaatccggagagcaggaagactgcttccacttcgtacaattctgcttctaggaagcaaagcaggaagggagaaaatcctattcgtgttactccgttaggagagcaatcttctgattttggatgttctagtacttggatatgtaaaaattctgcatgtagagctgttctgtctatagatgatgcgttctgtcggaggtgttcatgctgcatctgtcatcaatttgatgataataaagaccctagtctttggttggtttgtgaatccgagtctgggcagggtgattcttgtggattatcatgccatattgagtgtgcatttcaacaagaaaagctgggagttgtgaaccttgggcaatacatgcatttggatgggagttactgttgttcttcttgcggcaaagtctctgggatacttgggtgttggaaaaagcaattggctatagctaaggatgctcgacgtgtcgatgtgctttgctatagaatatttttgagttacagactcctcgagggcacagctaagtttaaggacctccacgagattgttgcagaagctaaaacaaagctggaggcagaggtgggtcctatgaacggagactctgtcaagatggccagaggtattgttagcaggcttgctattgctgcagatgtgcaaaagctctgttcgcacgcgattgataaagctaatgaatggctcgccaatgtttctagcattagttcaaattgcaaagtggatgcacttcctgctgcatgcaggtttctatttgaagaagttacttcttgttcacttgctatagttttgatagatatccccacaccaatgactgattccgtcaaaggctacaagctatggtactgcaaaagtagacatgagacttttgcaagggagcctacatccgtctttccaagggagaaaagaaaaatatctgtaaagaatctcaagccttgcaccgagtacacattcagaatagtttcctacacagaagttggtgatttaggccactctgaggctaagtgtttcaccaagagtttggagatcattagtaagaaatccaccacagtgggctgtaagaaggaagatccttgtgttgagaggagctcctcgaatgcaaaggaacaacataattcaaatttggctgcaatatcttctggattcaaggtgcgggaccttgggaaaatcttgcacctagcatgggcccaagaacagggttgccttgaaggtttctgcagtgctgatgtagaacaatgctgtggagtaactaaatgtgaatctccaaaagatcaccagtcacctccacctgtttctcgtgagcttgacctaaatgtagtttcagttcctgatttaaatgaagaccttacccctcccttagagtcttcaagggatgaagacaacggatgcacgctagagcgtgctactgggcctgatgatgatgctgcttcccatggtgttgagaagaatgggcttgggctagccaggtcaaatggtagtgggccaagtgatgagtctcaagcttgggctctcatccgaaatggagatgtgcctgctgttgattccttggcagagacccgtcggaagaggtcttcaagtgcgaatgaagaaacacatgactgtgacagcactctgataaatggatcgccatttcggatttcaggcgggcctggttctctagacggtaactttgagtattgtgtgaaggtcatccggtggttggagtgtgagggctatctaaaacaggaatttagattgaaattattgacttggtttagcttaagatctactgaacaagagcgtcgggtagtcagcactttcattcaaactctgatggatgatccaaagagcttagcaggacagctagttgattcctttggagatctcatatccagcaagaggcccaggactagtttcactagcattccttcctaaataaatcttaactaaggacggcacacatatcttggatacaattcagatgtttaggacacaatttttaggaggcagtacctgattttcctcgagaaagggattccatcagtggttaactgcacattttagaaggtatttgttagagtttccttgaccacatttgtagaaagattcacattgagacaatcattgttgccttctcgcattgaaggaaggatatatgcttcaatgaatatttaaattctagttcaatttactaattaattagtttgttttctcaaaaaaaaaaaaaaaaaaaaaaaagtactagtcgacgcgtggcc

SEQ ID NO: 9 - protein, 653 aa, Beta vulgaris
MIEPQLKACNKNVKNPESRKTASTSYNSASRKQSRKGENPIRVTPLGEQSSDFGCSSTWICKNSACRAVLSIDDAFCRRCSCCICHQFDDNKDPSLWLVCESESGQGDSCGLSCHIECAFQQEKLGVVNLGQYMHLDGSYCCSSCGKVSGILGCWKKQLAIAKDARRVDVLCYRIFLSYRLLEGTAKFKDLHEIVAEAKTKLEAEVGPMNGDSVKMARGIVSRLAIAADVQKLCSHAIDKANEWLANVSSISSNCKVDALPAACRFLFEEVTSCSLAIVLIDIPTPMTDSVKGYKLWYCKSRHETFAREPTSVFPREKRKISVKNLKPCTEYTFRIVSYTEVGDLGHSEAKCFTKSLEIISKKSTTVGCKKEDPCVERSSSNAKEQHNSNLAAISSGFKVRDLGKILHLAWAQEQGCLEGFCSADVEQCCGVTKCESPKDHQSPPPVSRELDLNVVSVPDLNEDLTPPLESSRDEDNGCTLERATGPDDDAASHGVEKNGLGLARSNGSGPSDESQAWALIRNGDVPAVDSLAETRRKRSSSANEETHDCDSTLINGSPFRISGGPGSLDGNFEYCVKVIRWLECEGYLKQEFRLKLLTWFSLRSTEQERRVVSTFIQTLMDDPKSLAGQLVDSFGDLISSKRPRTSFTSIPS

SEQ ID NO: 10 - DNA, 184 bp, Artificial Sequence
  BvAP1 cDNA
ctagagcaagtgcaacagatgcagtggcagaaccagcaccagcaccagcaccagcagcagccgccaccgccgccacaaaatcatcaagttcctcctgacgcatcaaatttcatgctcccacctccaattccttctttgaacacgggtgggtaccaaggacaatttggtggagaagtaaggagga

SEQ ID NO: 11 - DNA, 150 bp, Artificial Sequence
  BvAP1 fragment
ctagagcaagtgcaacagatgcagtggcagaaccagcaccagcaccagcaccagcagcagccgccaccgccgccacaaaatcatcaagttcctcctgacgcatcaaatttcatgctcccacctccaattccttctttgaacacgggtggg

SEQ ID NO: 12 - DNA, 100 bp, Artificial Sequence
  BvAP1 fragment
ctagagcaagtgcaacagatgcagtggcagaaccagcaccagcaccagcaccagcagcagccgccaccgccgccacaaaatcatcaagttcctcctgacg

SEQ ID NO: 13 - DNA, 50 bp, Artificial Sequence
  BvAP1 fragment
ctagagcaagtgcaacagatgcagtggcagaaccagcaccagcaccagca

SEQ ID NO: 14 - DNA, 212 bp, Artificial Sequence
  BvFUL fragment
agagggagaaggtgctggctcagcaggcagaattggatcagcaaaatcatgacaataactcatctggctttgtgatgtctcaagctttgccctcactgaatacaggaggaacaagcagcagtgcagtggaagatgaagcaacacaaccaccaaatctaaacagcaactctgcacaaataccgtcctggatgcttcaacacatccaagagcag

SEQ ID NO: 15 - DNA, 150 bp, Artificial Sequence
  BvFUL fragment
tctggctttgtgatgtctcaagctttgccctcactgaatacaggaggaacaagcagcagtgcagtggaagatgaagcaacacaaccaccaaatctaaacagcaactctgcacaaataccgtcctggatgcttcaacacatccaagagcag

SEQ ID NO: 16 - DNA, 100 bp, Artificial Sequence
  BvFUL fragment
aagcagcagtgcagtggaagatgaagcaacacaaccaccaaatctaaacagcaactctgcacaaataccgtcctggatgcttcaacacatccaagagcag

SEQ ID NO: 17 - DNA, 50 bp, Artificial Sequence
  BvFUL fragment
gcaactctgcacaaataccgtcctggatgcttcaacacatccaagagcag

SEQ ID NO: 18 - DNA, 399 bp, Artificial Sequence
  BvVIL1 fragment
cacagctaagtttaaggacctccacgagattgttgcagaagctaaaacaaagctggaggcagaggtgggtcctatgaacggagactctgtcaagatggccagaggtattgttagcaggcttgctattgctgcagatgtgcaaaagctctgttcgcacgcgattgataaagctaatgaatggctcgccaatgtttctagcattagttcaaattgcaaagtggatgcacttcctgctgcatgcaggtttctatttgaagaagttacttcttgttcacttgctatagttttgatagatatccccacaccaatgactgattccgtcaaaggctacaagctatggtactgcaaaagtagacatgagacttttgcaagggagcctacatccgtctttccaaggga

SEQ ID NO: 19 - DNA, 396 bp, Artificial Sequence
  construct comprising BvFUL fragment and BvAP1 fragment
agagggagaaggtgctggctcagcaggcagaattggatcagcaaaatcatgacaataactcatctggctttgtgatgtctcaagctttgccctcactgaatacaggaggaacaagcagcagtgcagtggaagatgaagcaacacaaccaccaaatctaaacagcaactctgcacaaataccgtcctggatgcttcaacacatccaagagcagctagagcaagtgcaacagatgcagtggcagaaccagcaccagcaccagcaccagcagcagccgccaccgccgccacaaaatcatcaagttcctcctgacgcatcaaatttcatgctcccacctccaattccttctttgaacacgggtgggtaccaaggacaatttggtggagaagtaaggagga

SEQ ID NO: 20 - DNA, 300 bp, Artificial Sequence
  construct comprising BvFUL fragment and BvAP1 fragment
tctggctttgtgatgtctcaagctttgccctcactgaatacaggaggaacaagcagcagtgcagtggaagatgaagcaacacaaccaccaaatctaaacagcaactctgcacaaataccgtcctggatgcttcaacacatccaagagcagctagagcaagtgcaacagatgcagtggcagaaccagcaccagcaccagcaccagcagcagccgccaccgccgccacaaaatcatcaagttcctcctgacgcatcaaatttcatgctcccacctccaattccttctttgaacacgggtggg

SEQ ID NO: 21 - DNA, 200 bp, Artificial Sequence
  construct comprising BvFUL fragment and BvAP1 fragment
aagcagcagtgcagtggaagatgaagcaacacaaccaccaaatctaaacagcaactctgcacaaataccgtcctggatgcttcaacacatccaagagcagctagagcaagtgcaacagatgcagtggcagaaccagcaccagcaccagcaccagcagcagccgccaccgccgccacaaaatcatcaagttcctcctgacg

SEQ ID NO: 22 - DNA, 100 bp, Artificial Sequence
  construct comprising BvFUL fragment and BvAP1 fragment
gcaactctgcacaaataccgtcctggatgcttcaacacatccaagagcagctagagcaagtgcaacagatgcagtggcagaaccagcaccagcaccagca

SEQ ID NO: 23 - DNA, 795 bp, Artificial Sequence
  construct comprising BvFUL fragment, BvAP1 fragment and BvVIL1 fragment
agagggagaaggtgctggctcagcaggcagaattggatcagcaaaatcatgacaataactcatctggctttgtgatgtctcaagctttgccctcactgaatacaggaggaacaagcagcagtgcagtggaagatgaagcaacacaaccaccaaatctaaacagcaactctgcacaaataccgtcctggatgcttcaacacatccaagagcagctagagcaagtgcaacagatgcagtggcagaaccagcaccagcaccagcaccagcagcagccgccaccgccgccacaaaatcatcaagttcctcctgacgcatcaaatttcatgctcccacctccaattccttctttgaacacgggtgggtaccaaggacaatttggtggagaagtaaggaggacacagctaagtttaaggacctccacgagattgttgcagaagctaaaacaaagctggaggcagaggtgggtcctatgaacggagactctgtcaagatggccagaggtattgttagcaggcttgctattgctgcagatgtgcaaaagctctgttcgcacgcgattgataaagctaatgaatggctcgccaatgtttctagcattagttcaaattgcaaagtggatgcacttcctgctgcatgcaggtttctatttgaagaagttacttcttgttcacttgctatagttttgatagatatccccacaccaatgactgattccgtcaaaggctacaagctatggtactgcaaaagtagacatgagacttttgcaagggagcctacatccgtctttccaaggga

SEQ ID NO: 24 - DNA, 845 bp, Beta vulgaris
ctaggtcagattcgctatctatcttcttcttcttttttgttggtcaatcactctgaagaacctttatgacaagtagtattaagtttcatgaacttctagtttaaactcgctctaaaaatactaaaagattacatttcaatatatattcctgtgttatatatacacatgctgttttgtagtaaatattatgtgaagttggtcttaaaattgacatgatgtaaatatcacgtcagtttttataaccgattcaaattaaacatcagttataacaagcgatgcaaatattatgtgaagttgcatcagttgttaataaatcgatgtaaattatttgcatcaacaagatacgaatcgtttatttaagtgatgtaaaatttctttacatcaattataagtaatacaaatattcaatataagtgatttaaaatgatattttttttgtagtgatcccatgtgaagttataattcattctttcagcatcatagtctcttggagttttctctttgtcctcaccacacttattattctcttcccttttaactatcaaaagataccctccccttaactttaagattttaaattaagaaatcgtagacacgaaaaatctaagaactaacaaatattttgataaagacagcttctaaaattcaatatctgaatagtatctcttggaaaatgtcgtgttgtggtcggtcacatttcaacactcttgtacaaaagcgtcaacttgacttcatgtgacagtttttgtttattagagatgtttagttgtagaattgatgatttatgtatataacaacgatattctatagatatatattgatgttaaaagataaacaggaggaac

SEQ ID NO: 25 - DNA, 29 bp, Artificial Sequence
  forward primer WAG-AP1FUL
ctcgagagagggagaaggtgctggctcag

SEQ ID NO: 26 - DNA, 31 bp, Artificial Sequence
  reverse primer WAG-AP1FUL
cccgggtcctccttacttctccaccaaattg

SEQ ID NO: 27 - DNA, 31 bp, Artificial Sequence
  forward primer vil1RNAi-fwd
gtcgaccacagctaagtttaaggacctccac

SEQ ID NO: 28 - DNA, 29 bp, Artificial Sequence
  reverse primer vil1RNAi-rev
ctcgagtcccttggaaagacggatgtagg

SEQ ID NO: 29 - DNA, 411 bp, Artificial Sequence
  VIL1 cDNA fragment for cloning of VIL1-AP1-FUL RNAi construct
gtcgaccacagctaagtttaaggacctccacgagattgttgcagaagctaaaacaaagctggaggcagaggtgggtcctatgaacggagactctgtcaagatggccagaggtattgttagcaggcttgctattgctgcagatgtgcaaaagctctgttcgcacgcgattgataaagctaatgaatggctcgccaatgtttctagcattagttcaaattgcaaagtggatgcacttcctgctgcatgcaggtttctatttgaagaagttacttcttgttcacttgctatagttttgatagatatccccacaccaatgactgattccgtcaaaggctacaagctatggtactgcaaaagtagacatgagacttttgcaagggagcctacatccgtctttccaagggactcgag

SEQ ID NO: 30 - DNA, 408 bp, Artificial Sequence
  construct comprising BvFUL fragment and BvAP1 fragment for cloning of VIL1-AP1-FUL RNAi construct
ctcgagagagggagaaggtgctggctcagcaggcagaattggatcagcaaaatcatgacaataactcatctggctttgtgatgtctcaagctttgccctcactgaatacaggaggaacaagcagcagtgcagtggaagatgaagcaacacaaccaccaaatctaaacagcaactctgcacaaataccgtcctggatgcttcaacacatccaagagcagctagagcaagtgcaacagatgcagtggcagaaccagcaccagcaccagcaccagcagcagccgccaccgccgccacaaaatcatcaagttcctcctgacgcatcaaatttcatgctcccacctccaattccttctttgaacacgggtgggtaccaaggacaatttggtggagaagtaaggaggacccggg

SEQ ID NO: 31 - DNA, 25 bp, Artificial Sequence
  forward primer for VIL1-AP1-Ful
gtcgaccacagctaagtttaaggac

SEQ ID NO: 32 - DNA, 25 bp, Artificial Sequence
  reverse primer for VIL1-AP1-Ful
cccgggtcctccttacttctccacc

SEQ ID NO: 33 - DNA, 780 bp, Artificial Sequence
  BvAP1 cDNA showing sites for mutagenesis
  mutation (1)..(1): any nucleotide except a
  mutation (2)..(2): any nucleotide except t
  mutation (3)..(3): any nucleotide except g
  mutation (52)..(52): c to t
  mutation (151)..(151): c to t
  mutation (262)..(262): c to t
  mutation (316)..(316): c to t
  mutation (343)..(343): c to t
  mutation (376)..(376): c to t
  mutation (388)..(388): c to t
  mutation (391)..(391): c to t
  mutation (418)..(418): c to t
  mutation (433)..(433): c to t
  mutation (463)..(463): c to t
  mutation (484)..(484): c to t
  mutation (541)..(541): c to t
  mutation (547)..(547): c to t
  mutation (550)..(550): c to t
  mutation (556)..(556): c to t
  mutation (562)..(562): c to t
  mutation (568)..(568): c to t
  mutation (574)..(574): c to t
  mutation (580)..(580): c to t
  mutation (586)..(586): c to t
  mutation (589)..(589): c to t
  mutation (592)..(592): c to t
  mutation (610)..(610): c to t
  mutation (619)..(619): c to t
  mutation (688)..(688): c to t
  mutation (694)..(694): c to t
bvhggaaggggtagggttgagctgaagaggatagagaataagatcaatagacaagtaactttttcaaagagaagaagtggacttgtgaagaaagctcatgaaatttctgttctttgtgatgctgaggttgctctgatcattttttctcactgaggaaaactctttgagtattcttctgattcttctatggagaagatcctagaaaggtatgagaggtattcttacgcagaaagacggctagcttcaaatgatccagactcataggtaaactggacctttgacttcgcaaaactgaaggcgaagcttgaacttctataaaggaatcataggcactacttaggataagagcttgactcgcttaacatgaaggaactttagagtttagagtaataacttgatactgctctaaaaaatgtttgatctaggaagaactaactgatgcacgagtccatttctgaactctagaagaaggagagggcaatgtaggagcacaataacatcctgtctaagaagatcaaggagagaggaaaaaatctagagtaagtgtaatagatgtagtggtagaactagcactagcactagcactagtagtagccgccaccgccgccataaaatcattaagttcctcctgacgcatcaaatttcatgctcccacctccaattccttctttgaacacgggtgggtactaaggataatttggtggagaagtaaggaggaatgatcttgacctgacgctagaaccgatatactcatgtcacatgggatgctttacaacatga

SEQ ID NO: 34 - DNA, 735 bp, Artificial Sequence
  BvAP1 cDNA showing sites for mutagenesis
  mutation (1)..(1): any nucleotide except a
  mutation (2)..(2): any nucleotide except t
  mutation (3)..(3): any nucleotide except g
  mutation (19)..(19): c to t
  mutation (52)..(52): c to t
  mutation (235)..(235): c to t
  mutation (316)..(316): c to t
  mutation (325)..(325): c to t
  mutation (376)..(376): c to t
  mutation (391)..(391): c to t
  mutation (433)..(433): c to t
  mutation (457)..(457): c to t
  mutation (463)..(463): c to t
  mutation (466)..(466): c to t
  mutation (541)..(541): c to t
  mutation (544)..(544): c to t
  mutation (559)..(559): c to t
  mutation (562)..(562): c to t
  mutation (601)..(601): c to t
  mutation (664)..(664): c to t
  mutation (694)..(694): c to t
  mutation (715)..(715): c to t
  mutation (724)..(724): c to t
bvhgggagaggtagggtttagctcaaaagaattgaaaacaagatcaaccgttaagtgaccttctccaaacgtcggattggattgttgaagaaagcgcacgagatctccattctctgcgatgccgatgtagctctcatcatcttctccactaaaggcaagctcttcgagtatgcttctgatacctgcatggaaaggatactcgagcgctatgaaagacactcatatgcagagagataactgactgctccagatcctggatcccatgtaagtttgactctggaacacgcaaaacttaaggctaggctggacattctttagaaaaattaaaggcattacatgggagaagaacttgataccttgagtctcaaggagctttagaatttagagcattaaattgacagtgctcttaaacacatcaggtcaaagaagaactaactcatgcatgaatcgatttcttagctttagtgaaaggacaaagcgttaaaggagcacaacaacttgctatccaagaaggtgaaggagagggagaaggtgctggcttagtaggcagaattggattagtaaaatcatgacaataactcatctggctttgtgatgtcttaagctttgccctcactgaatacaggaggaacaagcagcagtgcagtggaagatgaagcaacataaccaccaaatctaaacagcaactctgcataaataccgtcctggatgctttaacacatctaagagcagtaa

SEQ ID NO: 35 - DNA, 780 bp, Artificial Sequence
  BvAP1 cDNA mutation position 262
  mutation (262)..(262): c to t
atgggaaggggtagggttgagctgaagaggatagagaataagatcaacagacaagtaactttttcaaagagaagaagtggacttgtgaagaaagctcatgaaatttctgttctttgtgatgctgaggttgctctgatcattttttctcaccgaggaaaactctttgagtattcttctgattcttctatggagaagatcctagaaaggtatgagaggtattcttacgcagaaagacggctagcttcaaatgatccagactcataggtaaactggacctttgacttcgcaaaactgaaggcgaagcttgaacttctacaaaggaatcataggcactacttaggacaagagcttgactcgcttaacatgaaggaacttcagagtttagagcaacaacttgatactgctctaaaaaatgttcgatctaggaagaaccaactgatgcacgagtccatttctgaactccagaagaaggagagggcaatgcaggagcacaataacatcctgtctaagaagatcaaggagagaggaaaaaatctagagcaagtgcaacagatgcagtggcagaaccagcaccagcaccagcaccagcagcagccgccaccgccgccacaaaatcatcaagttcctcctgacgcatcaaatttcatgctcccacctccaattccttctttgaacacgggtgggtaccaaggacaatttggtggagaagtaaggaggaatgatcttgacctgacgctagaaccgatatactcatgtcacatgggatgctttacaacatga

SEQ ID NO: 36 - DNA, 735 bp, Artificial Sequence
  BvFUL cDNA mutation position 316
  mutation (316)..(316): c to t
atggggagaggtagggttcagctcaaaagaattgaaaacaagatcaaccgtcaagtgaccttctccaaacgtcggattggattgttgaagaaagcgcacgagatctccattctctgcgatgccgatgtagctctcatcatcttctccactaaaggcaagctcttcgagtatgcttctgatacctgcatggaaaggatactcgagcgctatgaaagacactcatatgcagagagacaactgactgctccagatcctggatcccatgtaagtttgactctggaacacgcaaaacttaaggctaggctggacattctttagaaaaatcaaaggcattacatgggagaagaacttgataccttgagtctcaaggagcttcagaatttagagcatcaaattgacagtgctcttaaacacatcaggtcaaagaagaaccaactcatgcatgaatcgatttctcagcttcagcgaaaggacaaagcgttaaaggagcacaacaacttgctatccaagaaggtgaaggagagggagaaggtgctggctcagcaggcagaattggatcagcaaaatcatgacaataactcatctggctttgtgatgtctcaagctttgccctcactgaatacaggaggaacaagcagcagtgcagtggaagatgaagcaacacaaccaccaaatctaaacagcaactctgcacaaataccgtcctggatgcttcaacacatccaagagcagtaa

SEQ ID NO: 37 - DNA, 21668 bp, Artificial Sequence
  BvAP1 genomic DNA showing sites for mutagenesis
  mutation (1)..(1): any nucleotide exept a
  mutation (2)..(2): any nucleotide exept t
  mutation (3)..(3): any nucleotide exept g
  mutation (52)..(52): c to t
  mutation (151)..(151): c to t
  mutation (6999)..(6999): c to t
  mutation (7640)..(7640): c to t
  mutation (8573)..(8573): c to t
  mutation (8606)..(8606): c to t
  mutation (8618)..(8618): c to t
  mutation (8621)..(8621): c to t
  mutation (8648)..(8648): c to t
  misc_feature (9833)..(11385): n is a, c, g, or t
  mutation (11796)..(11796): c to t
  mutation (11826)..(11826): c to t
  misc_feature (12467)..(12605): n is a, c, g, or t
  misc_feature (13741)..(14088): n is a, c, g, or t
  misc_feature (16396)..(17194): n is a, c, g, or t
  mutation (21152)..(21152): c to t
  mutation (21313)..(21313): c to t
  mutation (21319)..(21319): c to t
  mutation (21322)..(21322): c to t
  mutation (21328)..(21328): c to t
  mutation (21334)..(21334): c to t
  mutation (21340)..(21340): c to t
  mutation (21346)..(21346): c to t
  mutation (21352)..(21352): c to t
  mutation (21358)..(21358): c to t
  mutation (21361)..(21361): c to t
  mutation (21364)..(21364): c to t
  mutation (21382)..(21382): c to t
  mutation (21391)..(21391): c to t
  mutation (21576)..(21576): c to t
  mutation (21582)..(21582): c to t
bvhgggagaggaagagtgcagctgaagaggatagagaataagatcaacagataagtaactttttcaaagagaagaagtggacttgtgaagaaagctcatgaaatttctgttctttgtgatgctgaggttgctctgatcattttttctcactgaggaaaactctttgagtattcttctgattcttcgtaagtatatatatatatatattaatagtaactacttgttttctgctttctatttttaggtctgatgcatatttaatttaggtaatattaattccttatatctgatccttaatttttttttcttttaccatttcatttttgtttgttttgaataaaagaaaatttccccttcacgtgtgtcgaataggtcaaaatttttacttgaaggatgttctctttgattactaaaataggatccaacaatcacctgaaataaaggaagaagatggtgcaaagtttttactgtcatacttagtatttgataaatattctatgatgaacttgtataaattaggaaatagacctaactttcatgcacgaaaacattattccttcattcaatttttttattacttaaggatttacttttttattgatcatatgaagtagtagtacttgtaatcattcaatttttttgttggttaaataggactacattttaaaacaacccaattttaaaattttttgtgtgaatttcttccctttttaaaaataaagtctattatcatagcttagagtagctgtggcaaagctagacgaaataatacagaaatctggaaaggaaattgtactacttacatgaacacacttatttattacttgcatgatatctgcgaaaaagtttatagcaaatttggttaatatatagcgtagtactttggatattaatattactagtgtacaaatacttgatccaatgggtaatgaaacttatggaagatttgaccatacatgatgatgctaaatattaattgttattgtccagctttgttttccctccatccattggcatcttcatctttacattgctactccactcacttgtcaattgtttcgtcctttatgttctttattcacatgtgcaccatacttcaatactttccccttctttatcctcagtttttttttcttgtcattttagggttaatatccaatgaaatctagtttgctcgttttagatctaattttaattcgatcacaaccatccatatttttgtttcttagcttgacatctattctatggatctgggatcttcggtgtatagatgttctcggttttcagatcaagatcctattcatagacccatttattgtaaacacttaaatgtgttcttaaaaagttagtggctcgccaagtcaactcaataacataacccccacgacttcattacattacacaatgaaagattagatgtatgagtttgtgaagcttataattctatttcaagtaggactaggatgttttgtgcaatcagcagctagtagtctttttaatttaagtcagtcttcattgtgcatcatatatttttagaaatatatgcaagtttgaaaccatttagaacctcatgacccgcctgactcactataaaccggcaagagcttaatttttcacagctttgtatctttatgagtagcgctagctaggggtatgggcatagaaaaaaagggtttgggttagggtcttacaagatcttatccgctatttttatttcataatctttcaaaatacatgtttaataattcaaaatacatgtttaatactatctccatttcacaacatatgcaccaattgcctagctatggtccaacctagttggtttgtagcttgcattggatggttaggatgtattggagttgtttatgtgcaatcaaattttaattacgtatcaaaaaaaaaaaaaaaaaaacatatgcaccaatttccatttggacacacttattgaccaatttttgacaatatttttctcaccattttgtaagaaaaatcaaaatcaagtggaattttgttaagtttatctcagtcaaaagattccatacatcgacattttataatttttaatcatacgcaattagaaatatcaatgtctaaagaagcgtgttggaatacgtgaaaaagcaaatgatacatgaaacagatgtagtatatagaaaacttaattttgtgtcactcggatgtatgtgggcggagccttcctagaaggcgtacccaccttagtggctctgaatctttgacgacccgttcggttggtggtgataatagatggtaatagtaatgtaatttagtctaaatttataaataaatattaatatcattacccatggtaatacaagttcttcacaaaacatgtttcatttaaaaattatcattactaccttttcaagtggtattggatgataataaaattttaggcagggaaatgggtattgggatgaacattaccatgggtaatgacatgcaatttttgttacaagaatacagtataatacattactattgccaccatgtataaccattaatcaaatggaccgtgaggatatgatgttgaagaagaagtcttaacctctacgctattatttactagggtctgtaaattttccttttttaattataattcttgtgaaatcttcttcactgatggtactagcttattaggatgggtttctttagtatattgaaggctcttgttgacagagtataaaaatatttttggggtcgcaaccatcaatttaaacttttgtttgattataaaattattttttgaacatcaacaatctacttaaatttttggttgagttagttctttgacatggtatcacaaccatcatgacataaaggtctcatattcaaatctcattcacctctcatttccaagtagaatatttacctcaggtatgggtatgagggaggcttgtgttgcatgagtcaataacggatcttgaccaataatttaacaggggcgagttgataaattaagttttaatgtaaaattttaaatgatggataaaaacactaatacacaccaaaatataaatatacttttattaatggttacaaagagcttgtagctaatgtaataaatcaaaatcccaaaggtgcaatttttaagaaattatttccatttatttatttgaccattatgaaatcttcaagaaattgagtaagtttttaagaaatttaaggtatagttcattaactaaataaactactccagtaaaaaaaaattaccaaactgctttcttaagtaaaaaaataaataaatttatattttatgattgttaggaatgagtgtgaggaaataaaaagtactattatagttaaataaaaatgaaagttcttcagagaagaagaatagaagatagtacaatcaatgttaaatatttttctaaattagacaaattgatataaaccaaaaataaaggggaagaagaaagaaataagtaaaaaaagaaagaaggaaaagaaaaaaagaaaaaagagaagcaagtgaagaaaaacaaagaagtccaaatgtgtgttgatgcaaggttcgagcttgcaacattaagggctcaaactttcttttacactttggttcactgccaccgtgcccacagcttgttatgtgacatgaagtgtagtttgcttaatttatcttatacagttatgggggaccaagcctccacccgccccttctataatctgtcagtggttgcatccacactttaagtccaatagactcttgtctgagaggaggtgatagagtatataaatatttttggggcctcaaccattagctcaatcttttgattaagttggttctgtgacacttgtactatatactagttatatatatactgtaaaactagtaccacgagaacagtccttaatacaaacaacatgcccttaatagaattttcttagtatacacttaatataggttgactagctttttgcccttcagtatgcacacaccttttataatctgtatcgttgtctggtagatgataataaacctcagtattggcaatatatgaaatgacataatggccatgtttggtgattagagtttagagtttagaggttacagttcagagtttgtggttagatgattacttttttgttcagaggatttgactgctgatttaaataattgttgtgtaaaggtgtttggtaacacttagcttattgtttagagttttgtactttttagagcatgtaaaatgacatttatggacatatgtatttttttaaaacaaattttagtagtaattatatggacaaaatagtcatttgttttttctctctccaaaactctcatgaaaaagctcctctacccagctttttcaaaagagagttttgatcagagttttcggtacaaaactctctttagtcctctctctcaccaaacacccaaattagagtttttattggtcaaaactctaaactctctccaaacctctaaactctctctaaaactctctcccccaaacacccccaatttcttagaaaaatttgttgctcctttttattgcactatatttctatctccaaacataaagtttcttttacaaattttcatttctactccataccacctttatatggcaatataatttctatgaattaaaatgttcacaagttttgaggtggatttcaagagcatggacaatatgatcatgagactctccatacaaaaattacccttaaattttataatcatacaccaagcggtcgttaaagtattggaagtgcttgagtagtttgtgaaaattaacatataataaagtgcagatctcccctctagtaagtagtaagaagtagtaagacgatgtccctcatttgagaaagagaaaaacccttatcagtttctcttgtttctttgactgaacgcaagtcaaatagaagtatgtaactaggaaatccttggagaaatagattttctttaaaactataaaagtatacctatatatatggtaacccacaaaaatgtatataatctgatcaatatctaaacaaagtattcttatgttttctttcatcttgcttatttcctccctttccttttcttactttaatttgtttactctctttaacttatttctttgcgtatctcatttcactttacaaggatatatagttgattatgacagcttaataaatatattttggaactaggatttattggttgtcgttgttattttaatttctacactgatcggctagagtttctagaacatagggctttattgaaaccattagttaacaaaattgaatgacaatgattcaatatgatagaatatgtatgtattagttaatgtttgattattgtttgtatgtatataatcaaagattatttagtaatacttctatatacatattctattagaatcacttagaaagacccattgaacaataataaggataggcagacaagcaaacaaaagaaaaataaacctgttactccttccatttcttaatgttctactcggaattatagatacacactttgacacaaattagaaagagagtgtaaaaagtggatccatattaatatttttatttttttaaatgaggagagaagtgtgggtttattatgtttcaagggagatagagagcattgaatagtgagagaatatgtgccaaagataattaaatcattgtaaatcttttgccaaataaagaataaagcatgtgagtaaaactttaaaaaatgggcgaaaaaggaaagttgagtagaactttaagagacggaaggaatatagaagaggacgtgacagatgggaggaagatcagacatcttagaaggggaatagttaaatttgagatagtcttttaattaaggttctcactaaagaagatataacagtaggggaaagctaaaggttattcaaaactttccttcccatcttcatcacttcatgtctttactttagagctcttaacacttagcctatgaaattctgaactctttgtaagattagtgatagataaaagaatcttatcaatttaatttataaatacaacaggattcaataaaaagatatagagatctataaataaagagccatactgttgtgaacttttatatctatcaaaacctttgcacattagacgtggtataactaaatcaggcttatcgaaattttttaaaattgttttcattatagcccctttatatttagaagttctaagatgattgcatagatagttgatgcaccgttctggtcgacttttttaaacacttctttttgataaatttttttttttgtattcgaatcattattttaggtgtataaagagctgcaaatgatctagatgagattgatctcggtttcatttatatgctaatagtgtgttagatacacactattaaaaaagtcatatgacttagagattattatggaaaagggatagtgcaccgatattaatataatggaaaatgacacacgagttgtccataataacatgtgaaaagtgaactatttaaaaggtttttctgacctagtacatacaaggtgcgtaggtttagctattttagttttttagttttattttttaaagtgaagttagttattgatctgaaatcatataacatgtacgtaccgtagatataaaaaactaccaagtatatatcaatttgaaataaacattattttaatatggcaaaatcacaattgttgactagacctaacactgaagaaaactatgtcatgtttatcaattatgttgcatacagttaaaaacaaatatgttagagaaatcgttatttgaaatagaaaagttgcgcaaaatagtgattaacatcaaaatatgttcagaaagtttttataaatatgtgatcttgcattgtctgttgactgtcgaggtttatgataatttcccctttttccaatgcaaaacttgttgtgctattttctaatgatatattttttcaaagtatggagaagatcctagaaaggtatgagaggtattcttacgcagaaagacggctagcttcaaatgatccagactcataggtagtgcatttatgtaaatatagatatactcttcatgcccaagaagcctgaattttttatcccactacgtactgcaaagccaagtttaattgaataattgtcctgtttaaattatttagttttcagtacaataatgtaatcattagtttgcatgtttaaaaaagaaaagcacaagttctgatcaagtgaaatataaattgtaacgaaagagccaagctagacaattacctagctaggagttatttgttatcgtttttgtttttaatttctagtttttttttttaaactagaaaatatagtttcaatcttttgttatcagttttcaaaatgacatatttaacataaatatgattgattttaaattcatttattatatcatatttcatttcaaaataagtgaaacacttgtctcaaaaagctcactctcacataaatgataaaagtgtttcacttattttaaaacggaagaattatgacttttacttttcataaaacgaaaaactgaaatatgacaataatctcaaatagcttggagaaaccagatttctatatatttccgtgatgaaatcacttttcattatacgtaggtaaactggacctttgacttcgcaaaactgaaggcgaagcttgaacttctataaaggaatcataggtatgatggcaatatgtcataatttttctattattatttttgcttccaaaaccagaccatatgtttgtatatttatatagtgatatactccatccgtttcattttaatctatacatttacacttatcaggtatgtcaatgcaaaattttgaggatatatatctttagttttgtatttataaaaattataaaaagtacatattaataaaatacatattatgatgaatctaacaagatcccacatgacgatatttccgtccgcgtatgaataacaaataatggccaaagtgaaatttgtgaatagtgtaaaatatcaaagtgtaacaattaaaataaaacggagggagtagtacttgtttgtcacatacttacttatttttgttctctccacaatgaaactgttctttctaataattaaaaaaagtgcatatgttgatgatttctctgtcactttaagtggatattgaatagtgataatggattactttgtgtataattgcatttcacatttgggtctaattttatacccttttcgcatatcatgctttgtgaatagtacatatgatgttcaagaatgtgagaagacatatcatacttttgatatacctcaaacatgggtgtatactgtatagtgaacgaaagtgttagtgtaattttatttaggaggtttagtggtttgtcctatatataatgctagtagttatacaccatagttgttgatgagcatcaactggctttcctaacatttttttctccataactttacccttaccttacattagattactctaggattacattctacctaaaatattattactcccatcattttaggtaaatatttttactttgatttttcgattattttcaagagtttaaaataatgattaaaatttaccatgatcaggcactacttaggataagagcttgactcacttaacatgaaggaactttagagtttagagtaataacttgatactgctctcaaaaatgtttgatctaggaaggtaagaaattttacttgtctaccgtagtttcataataaattagtatttgggctcgggctttgccccagattggtattgtcttttcaaatttgatatgcatttttttccatttccactaaaatatattaagaaaattcaacatttaaaggatacaaatataataatgtggatacttaaagtatgattaaaatttggttgagatggtaattgtgtcatgtataatagcaagaagtcacaagttcaaagctcgttgcaagctaaatttatttttgttgattgacatgacttatcaacacactggacaattctaatcatctagtggagtagcatatactagcaatttatgcacgtgatgtgtgccttacttttttagaatataatttataacttttttgagcataaacaaaggtaaaatttgaacattagacatatttttttgggctagctaaatttgttgtttaaacctatatcacttaaccaaactcctcttttattatttattgatttatattttatttaaaatttttaaaattaaaatgatgagcaataaaagaatgttaagtagatttattaagtatttcttatatttttatcaacaaagtattttgtgttaattaaattatttcactttgttaattgattgtattttcctttttaatttattacttgattgtgtattgattgatcaaacataatttttttgttaatttttttatgctatatttgaatttatttttctttcatctgtttttggtagagtagttgatttactaaagggtaattaaataaatttattgggggacaccatagctcccccctcccttatataatagagatttgtatagatttattgtcttcctcaattattgattaactagtcttctatgcacgcgatgcgtgtgttgattgtttgggtctattcttaatataaatttcatcaaaatataattatagtagtgtgatttacaattattgctatacaaactactgtaatttataaagttgttagaaattgagataaaaatttagatgtgaaattttgtggtcaaattatatttgtaattttttaaactgagtaaccgtttttctcatcatgtcaagttactttgttaatgcttatttaatttattattggaatttttgacccatctttaaattagaaaaggatataatnnnnnnnnnnnnnnnnnnnnnnnnnnnnnnnnnnnnnnnnnnnnnnnnnnnnnnnnnnnnnnnnnnnnnnnnnnnnnnnnnnnnnnnnnnnnnnnnnnnnnnnnnnnnnnnnnnnnnnnnnnnnnnnnnnnnnnnnnnnnnnnnnnnnnnnnnnnnnnnnnnnnnnnnnnnnnnnnnnnnnnnnnnnnnnnnnnnnnnnnnnnnnnnnnnnnnnnnnnnnnnnnnnnnnnnnnnnnnnnnnnnnnnnnnnnnnnnnnnnnnnnnnnnnnnnnnnnnnnnnnnnnnnnnnnnnnnnnnnnnnnnnnnnnnnnnnnnnnnnnnnnnnnnnnnnnnnnnnnnnnnnnnnnnnnnnnnnnnnnnnnnnnnnnnnnnnnnnnnnnnnnnnnnnnnnnnnnnnnnnnnnnnnnnnnnnnnnnnnnnnnnnnnnnnnnnnnnnnnnnnnnnnnnnnnnnnnnnnnnnnnnnnnnnnnnnnnnnnnnnnnnnnnnnnnnnnnnnnnnnnnnnnnnnnnnnnnnnnnnnnnnnnnnnnnnnnnnnnnnnnnnnnnnnnnnnnnnnnnnnnnnnnnnnnnnnnnnnnnnnnnnnnnnnnnnnnnnnnnnnnnnnnnnnnnnnnnnnnnnnnnnnnnnnnnnnnnnnnnnnnnnnnnnnnnnnnnnnnnnnnnnnnnnnnnnnnnnnnnnnnnnnnnnnnnnnnnnnnnnnnnnnnnnnnnnnnnnnnnnnnnnnnnnnnnnnnnnnnnnnnnnnnnnnnnnnnnnnnnnnnnnnnnnnnnnnnnnnnnnnnnnnnnnnnnnnnnnnnnnnnnnnnnnnnnnnnnnnnnnnnnnnnnnnnnnnnnnnnnnnnnnnnnnnnnnnnnnnnnnnnnnnnnnnnnnnnnnnnnnnnnnnnnnnnnnnnnnnnnnnnnnnnnnnnnnnnnnnnnnnnnnnnnnnnnnnnnnnnnnnnnnnnnnnnnnnnnnnnnnnnnnnnnnnnnnnnnnnnnnnnnnnnnnnnnnnnnnnnnnnnnnnnnnnnnnnnnnnnnnnnnnnnnnnnnnnnnnnnnnnnnnnnnnnnnnnnnnnnnnnnnnnnnnnnnnnnnnnnnnnnnnnnnnnnnnnnnnnnnnnnnnnnnnnnnnnnnnnnnnnnnnnnnnnnnnnnnnnnnnnnnnnnnnnnnnnnnnnnnnnnnnnnnnnnnnnnnnnnnnnnnnnnnnnnnnnnnnnnnnnnnnnnnnnnnnnnnnnnnnnnnnnnnnnnnnnnnnnnnnnnnnnnnnnnnnnnnnnnnnnnnnnnnnnnnnnnnnnnnnnnnnnnnnnnnnnnnnnnnnnnnnnnnnnnnnnnnnnnnnnnnnnnnnnnnnnnnnnnnnnnnnnnnnnnnnnnnnnnnnnnnnnnnnnnnnnnnnnnnnnnnnnnnnnnnnnnnnnnnnnnnnnnnnnnnnnnnnnnnnnnnnnnnnnnnnnnnnnnnnnnnnnnnnnnnnnnnnnnnnnnnnnnnnnnnnnnnnnnnnnnnnnnnnnnnnnnnnnnnnnnnnnnnnnnnnnnnnnnnnnnnnnnnnnnnnnnnnnnnnnnnnnnnnnnnnnntatatatatatttagctaagaaaaaaaagacatttcattgggggataccataactcccccttagcttatataatagagatactatacttcttttctgatagtgtcaaatttaattataaatctttaacattggccaattaataattggacaagaaaaaaatgagacaataataaataaggcgatcttcacagacgtattaacatgatggtaattaaaaatgttaatcatagatctttgtgttatcttaataatataaatttactaattagaatgtatcacataaagtaagtattaatagcagcataggataattcttataatggagattttatatttttttatataattatatgatttattgttgaaaatattagttgattttaactggttgtttattcaatgacagaactaactgatgcacgagtccatttctgaactctagaagaaggtaataactccattttttactctcaaaggtttattgtttttaacttatttcttctaaccttttatatatgagaaggtattgggttagacgcgtctgaccataatattaggtcggatgactttcagttggtttcaattttatttcagttggtttcaatttttgtccagttggtttcaatttttgttcagttggtttcaattttttttagctggtttcaatttttgttcagttggtttcaatattttttagttgatcttttttatttcagttggatgtcttttaagttcagttacttatcttattgtttcatttacgtgttttattgtaactgaaaacaaaacttaagtaaatgaaataaaataagttctaaataaaagcaacttagggcctgttctccccagcttattttcagttcagttcaattcagttcagttcaattcaattcatttcagttcagttcagatcagatcagttcagttcagatcagatcagttcttgacaatacttttactctcacatatcactattcatttcagttcagttcaattcaattcagttcagttcaattcagtttagttcagttcagttcagttcaattcagttgttttatgccgaagagaacaggcccttagnnnnnnnnnnnnnnnnnnnnnnnnnnnnnnnnnnnnnnnnnnnnnnnnnnnnnnnnnnnnnnnnnnnnnnnnnnnnnnnnnnnnnnnnnnnnnnnnnnnnnnnnnnnnnnnnnnnnnnnnnnnnnnnnnnnnnnnnnnnattcatttcagttcagttcaattcaattcagttcagttcaattcagtttagttcagttcagttcagttcaattcagttgttttatgccgaagagaacaggcccttagttttcagttacttatattatcgtttcagttagttttcttattctttcatttaacaactaactaaaataaaaaaaaaaaaactaactgaaagcaaaacttaattaaatgcaaaaaattaagttctaaatgaaaccacatacgatcgaaatttcaatcatttcaaacattatggtgttttcgattctttcaaagaaggcaagctgctcccgctattctaccctctttagatcacaataaagctcaggcctcacattcaaagtttcctcaaagatggacgttccaagtatcacatagacacatagtcctcttctccaaacgctctccttcctatcttgatgtcattagcaaacttcttgatccagacggcgccaacaaccgcaccatgatctccctctaaagtactgacggcccgtttggttgttggtcataaatgatggtaatgggaatgaagttgtgtgtaaatttgtgaaaaatatcattgtccattcccatggtaatgctaatttatcttaatgtgtccactttccttctagaattttcattctcatccaataccaccttgtaaggtggtaatgagtggtaatgaaaattgcttccccttggagacaaaaatacaagtttaggagtgagattgattgctcatggagaaaaaaagtctccccatggagatattaagggtgattccctaataaaattacacttaaaatttattcccattaccgcaatttattaacatctaccaaacgggccgtgaaagtcttgaaacacatagtcgagtgagtagctttgaggaaccatctgtaaaagaacctgagggagccaatgtgtgcgtaagtaccaacggcgtgttgtcagtggaaaaggtggtgccgtggtggcactcagtagtgatggagccgccgtggtgtttgagtgttgccaaatacaaaggcggaatttcgtaatctctaatttcttctgtgaaatttttgggatcagcctgtccgaccaaacacattggatcaaacggtctgacccaatagtttcaannnnnnnnnnnnnnnnnnnnnnnnnnnnnnnnnnnnnnnnnnnnnnnnnnnnnnnnnnnnnnnnnnnnnnnnnnnnnnnnnnnnnnnnnnnnnnnnnnnnnnnnnnnnnnnnnnnnnnnnnnnnnnnnnnnnnnnnnnnnnnnnnnnnnnnnnnnnnnnnnnnnnnnnnnnnnnnnnnnnnnnnnnnnnnnnnnnnnnnnnnnnnnnnnnnnnnnnnnnnnnnnnnnnnnnnnnnnnnnnnnnnnnnnnnnnnnnnnnnnnnnnnnnnnnnnnnnnnnnnnnnnnnnnnnnnnnnnnnnnnnnnnnnnnnnnnnnnnnnnnnnnnnnnnnnnnnnnnnnnnnnnnnnngatataaatagagatggaggacaagggtcttggttttgtcatgttgtcaaagagttgaacaatggttttttcgtattgttaaaaaattaaaaaaccagaggccttcaatctcttgatagatatagatagaaaaggaggacaaggccgttcttggttttgttatattgtcaaagagttgaacaatgattttttcgtgttgtcaaaaaattaaacaatgaaaaaagatggcgggtgcttgatctaatagatcggaccatggattgaaggtcttttaacttattttatatatatattgaacttatctgaagattatttaactctttgaaattgtattaacttccgaactttatgaacttttttaattcttcaaaacttatctacattttatttgaaaaaatattgaagacaaaaaaaccctcagttggtttaaagctgcggtaagatagagtgtaaatgttatttttttttattaaatcaagaaataaaaagaaatattaaataaaaagaattaaaaatggaaatgatgacagaaacttatggcttggaggagcaatacttttaagatagacctaaaccttaaataagttaaaatggaagtaatttttcagtagaatcttattccaatctatactccgtgtttactccatgtaatgcacatataataaaaaaattagaaattacatagtataaggtttgatcctgtgactgtaagtttatatactaacttcttaaccactagagcaagtgatatttagtgttatcattttaaagtataattttaacaaatgaaatttttttcttacccggaacatagctcggacctaataactagttgaacaattataatctgtaacttaaaatgatcctaattactgtactttcattacctataataatagaatcttactatcattggttcagaaaaaaaaaatcttattaaatgttaaccatttatttgtaattgaaacatacatgcacataaatgtaacttttagtttatcttaacttaaaaactgagaaaatgttagttggaaacttttgtatatatgtttggataaacgacgctcaaaagtaggggctaaaattttagtagataatataagattatactccatctgttctagatagacttctcatttttaattttggcagtattcataaataaaggaaatctttcaaaaaaatttccaatatataagaaaaaaaataatcatgtgcggttttgtttgattcgtctcattgtgtacattaggaaaattaaacttatataatttttactactatgtaattaaagatattaacgatacaaaatgtgtattgacaaacttatattggagtaataggaagtctattaagggaccgaagaaatattacgtaaataaatctaatacaaactaatataaattctactccagacaataaagattctgtcttatattgccaagatatagtagctatttattttatcttaacaaacataaatgtttctaatgcttaaacatggacatgtattattttgtaaaatattatgtattatccaaagttacatatttaaaggaagttctattgcttgctctcttttagcactgcccaaaaaggttaaagtaattttttttctctgtttaaaaaaaaaatgcattatatacagataatttttgctagtcaataaagctatccttatgacttatgagtgctacttgactagggatgtgttgtactcaattggaggtatacatacaccaagattatagagcttttattttgcctataaaaaatggaagccggataggataccaaaaaagctttgacttaaatttgtaatgcataaaaatgatgatacctaacttattagccatacttatctaagcgtacgtcaatttaaatattgtgttattgattaataatgatccttatatatccatattttgacaattaaacggtaaattagagagaaaagtttgagaaaataattatagcttacgtaatgctataatccaaagtgtctccgcacaagcgtgggacaaaatagtactttcggagaagttacaatcaacagctagggagtcttcattgttcttgaatagaaggatggaaacaaagttcaccttcttttattaaagtattaaggtttgttattagctcaatatccaatactttctctgctttttattacttcgtctgtttcaaattaaatgattttttttttattttacactatttttaaatttcacttttaccatcatttatgatttatatgtgaatgaaaacatagttacgtgtgatcttgttttttttttttttttttgtnnnnnnnnnnnnnnnnnnnnnnnnnnnnnnnnnnnnnnnnnnnnnnnnnnnnnnnnnnnnnnnnnnnnnnnnnnnnnnnnnnnnnnnnnnnnnnnnnnnnnnnnnnnnnnnnnnnnnnnnnnnnnnnnnnnnnnnnnnnnnnnnnnnnnnnnnnnnnnnnnnnnnnnnnnnnnnnnnnnnnnnnnnnnnnnnnnnnnnnnnnnnnnnnnnnnnnnnnnnnnnnnnnnnnnnnnnnnnnnnnnnnnnnnnnnnnnnnnnnnnnnnnnnnnnnnnnnnnnnnnnnnnnnnnnnnnnnnnnnnnnnnnnnnnnnnnnnnnnnnnnnnnnnnnnnnnnnnnnnnnnnnnnnnnnnnnnnnnnnnnnnnnnnnnnnnnnnnnnnnnnnnnnnnnnnnnnnnnnnnnnnnnnnnnnnnnnnnnnnnnnnnnnnnnnnnnnnnnnnnnnnnnnnnnnnnnnnnnnnnnnnnnnnnnnnnnnnnnnnnnnnnnnnnnnnnnnnnnnnnnnnnnnnnnnnnnnnnnnnnnnnnnnnnnnnnnnnnnnnnnnnnnnnnnnnnnnnnnnnnnnnnnnnnnnnnnnnnnnnnnnnnnnnnnnnnnnnnnnnnnnnnnnnnnnnnnnnnnnnnnnnnnnnnnnnnnnnnnnnnnnnnnnnnnnnnnnnnnnnnnnnnnnnnnnnnnnnnnnnnnnnnnnnnnnnnnnnnnnnnnnnnnnnnnnnnnnnnnnnnnnnnnnnnnnnnnnnnnnnnnnnnnnnnnnnnnnnnnnnnnnnnnnnnnnnnnnnnnnnnnnnnnnnnnnnnnnnnnnngtacatcaaggaaatttgcattaatgaaaaacgggagtacaacctaatggtaatacaaccaaactaaacagaaagaagaaacaacagacagtaagaaaacctctataacgcgtaaaaacaatttaacataaacactaactagaaaaagtccaggccgaataacatttgtcttgtgcgatggggagggaagatgaaggagagtgaaaatctgttgaaagacacaactctgacgatcttcatagagagattgtcgtacaactgctagtagatcctgtccactaggcacgaaatcccaaggtccttgatgagcctcctgggattctcctgattcgttgaacaaagaagtcactttcgagagtaacttcggaccctgctgcgagggtcttcgaaaatcagtcacattagactgaaacccgaaaaacaaggtggaggtcttgacgtgccccaaaacaagttgggggcgtcccacaagatgcgttttttaggtgtgatgacacatgatgtcatcacgagaaattggggcgagttagtttgatgaactacgccccactgacggatcctaagatccaaagtgacaatctcgaaaccagaagaccgacaaacaacagatctgaaacatacaaacatgaaaataatgaaagcataaactgccacccgacatatagagctccggcaaacaacaccatcaagaacttgcaccaaagacttccttggcatactaaagacactgattccaactaacactagcgggggacggggaagggacactcgactacacctaaacctaaccaggggacggggaaggggaacttagactaaaccttcgtaaaaagggggggatcggggaggggaaaaccttgaccaaggaagctggttttaaaaaccacttagccgagccaaaaaccgtgggtgggaagaagaaacagaccacaaacagggggaaccgggggatgggaactcaccgaacaggggagggggagaaatcgcacagactcggggaacgcctaaggactgggggacgaccaacgaacgaaaggttggggtggtgcgaaaacaagggagggggacgcaccgacgaacaaaaaaaccgacgaagaggccgaaaaagcgaaaggccgacggagataagattgaaaggcgacgaaaaaagaaaaaggaacaaaacgaaagaaaaacgaactcgtcggagacccgccggagacctacgcggcgccggatctccggcgagttctagggttagagggtttgttgtgtttgtttagggagaaggcagaggttttttttttttacgtgtgatcttgttagatttgtcttaacatgtattctttaatatacttttttttttataatttttgcaaatgcaaaattagagatatatgtcctctaaattttacattcacatacgtgataaataagagtgctacaactaatttgaaacggataaagtatttgaattgtttttcatttaaaaaagttcgctatcatttataatgttatatatttgccaatatgttatctctttctctctcttaccagagtttagatccagtagagttagtaaataattctaccacgtagagttgaacaaatcatagccattgattttcaaatcattggtttatatattctttcccaaaactcccccctattttccccaaaaatcctccccctccttatctctttccataaaatctgagtcgttgattttaaaatataaggtttggattcaactccactatgtagagttttcatcaaactccaccgaatccgagcccctcctaccatagtacttcttgatttccccatatttctttcctcatcttggtcctcaagcacattttaatattatgggtattaaacaatagagaaagtatttacttatagagaaagtattttcaatgattccctaaatttttttttgaaagaaagaaaagggatttcattaatatttcgccaaacggcacttacaagtcatttctgaaaaacataaaattctaaaagaaatacatatcaccctagaaatgtaaacatcgcagatttgacttaattttgccttaataaaaatcttcatctgaagcaatgcaatctgtgagttcgctctggttcggcatacgatctgcagatgcggaaattttgggatgaacgtactccaatagtcttccataattttacagaagttgtgaaaccctaattcttcatgttgaatctcgaacttcaaccaatgagaataatttctcatacctaaaaacaaaagaaccatactcacaactcccataggggagaaggagatttccaaaacagaaactaaaaaccccataaaagggtttgagaaaatctcataaagagatactaatttattgaacaaaacaagaaaatgaactaaaaactgaaaataaaagggaaaaaggggcttaccatggatgaaaacatccatggcagccccctaattgatgaagaaggggtaagggaggctagggttttagagagagaaaaggagaggggaggctaggttttaaaaaaaaatataatgattccctaaatttacttatatatatttaccaagatgacgtgatgttttacaaggcccatgatttttacgcgatcatgaaaaacacagccaatttgaatggagcaaatatctacgcgtcattttagatatttttgtatgggaaagttttttttgaccaatgtaattattaagaagcatcggccaccgggtagataagatgtcactatacatccttttccaaacttaagtatgcctgttgaacttttgttgcgtttgcagattcatttgaaattatatttcctcagatcctctacttgtaaaagaatgttccattattttcttagtttacatgatatttacaatagtatttgtctacattttgttcatattacttagtgatcagtgtatacgtcatatattagtttgaactttgaagacatttattttctatatacttcctttgtctgctaaattactttggaaagctttgttttttttattaatataagaccctttggagtttggaaatcactatctaatgaaatatataattcatcattagaacaaaaatacaaatatcgtactatcacctatcatgttccttttggatttcgcttcacaaaaatacattttaaaaaaaaataaaataacaaatggtagctaacaacttattacttttaaaagtttgtgtgcaccctaataagtactcaaagtagtatgtaacagagagagtataatgctaaaatacaaactaaataaacaagaaagtgtttctcaacaataatttgctgcaggaattaggaaacaaagtaaataaattgcatgtttatcatcaatacaatttactggtagttaattacaaacttcactcatgataattgaaagaggccactcaatttcagctaggagttgtttatttatttatttttctttcagttaaattttgactacccacaaaatcttcatctggacctaatctgcaatttgtggattttggatgaaatttctaacctatttaagtagtcttattgtttaaataacccatgcaattaaattaggttatatgggggtgattcatttaccaggcccaagattttatctcattctcaattattatcgcaacacccatgaacctaagccaacatgacttatttaccaggccagctagagaagaacaaggttgctgattttcttgtccgtgattgtagaagaaatgttagaaatctaaatgttgttagggatttacccctcccccctactgagtgtatgaacttattattgacggattgttgtaggcttccaagccaaaactctgattaagttttcttttatgccattttaaccaaaaaaaaaaaaaaagctaggaagctagctcagcgcgctctaattatttcacatgtgacatgttttacacttattcatacttctatatgcaggagagggcaatgtaggagcacaataacatcctgtctaagaaggtacttgcacttgaccagtttgtgtaatattgtaatttaatttcttagattttggttgcatgctttgatgacgaatgacgattgacgaatacatttttatgcagatcaaggagagaggaaaaaatctagagtaagtgtaatagatgtagtggtagaactagcactagcactagcactagtagtagccgccaccgccgccataaaatcattaagttcctcctgatgcatcaaatttcatgctcccacctccaattccttctttgaacacggggtagttacttcttcaacttaatttcctctattcaatattaagttaagaaacagatcacgtgattagttcgttaatattgctaattaataatcatattgttatatatcatgcattagtgggtactaaggataatttggtggagaagtaaggaggaatgatcttgacctgacgctagaaccgatatactcatgtcacatgggatgctttacaacatga

SEQ ID NO: 38 - DNA, 29237 bp, Artificial Sequence
  BvFUL genomic DNA showing sites for mutagenesis
  mutation (1)..(1): any nucleotide except a
  mutation (2)..(2): any nucleotide except t
  mutation (3)..(3): any nucleotide except g
  mutation (19)..(19): c to t
  mutation (52)..(52): c to t
  misc_feature (1029)..(1924): n is a, c, g, or t
  mutation (19373)..(19373): c to t
  mutation (19552)..(19552): c to t
  mutation (19561)..(19561): c to t
  mutation (19689)..(19689): c to t
  mutation (19704)..(19704): c to t
  misc_feature (20703)..(20722): n is a, c, g, or t
  mutation (28161)..(28161): c to t
  mutation (28185)..(28185): c to t
  mutation (28191)..(28191): c to t
  mutation (28194)..(28194): c to t
  mutation (28447)..(28447): c to t
  mutation (28450)..(28450): c to t
  mutation (28465)..(28465): c to t
  mutation (28468)..(28468): c to t
  mutation (28507)..(28507): c to t
  mutation (29166)..(29166): c to t
  mutation (29196)..(29196): c to t
  mutation (29217)..(29217): c to t
  mutation (29226)..(29226): c to t
bvhgggagaggtagggtttagctcaaaagaattgaaaacaagatcaaccgttaagtgaccttctccaaacgtcggattggattgttgaagaaagcgcacgagatctccattctctgcgatgccgatgtagctctcatcatcttctccactaaaggcaagctcttcgagtatgcttctgatacctggtatgtctaattttataacttcttcttttgtacatcaataattttatcatcgactcaactaaaagcttaagcagatggttagggttctattattattgaattacctcaaatttgtcatcgactcaactaaaagtagagtatatttcatgtagatcaggtgctttttttgaatatattgtcagttttagaactacaaaatgttgaacacaagtatttatacgcacgctgacatgtgaattttttaattgacaactttctaaattaatactctaaattactaatatgaagaacgtaatttattatttatcactttcagacaaaggcatgtttgttttttctattatttttcccatgaaaattctcaccaatatccgattctgtatgttaattttagtaatttctaattttgatgacttaataaattgtaaaaaagtataaaataaacaaatatccaaaacatctttgttttcaagagaaatatcttaaaaacttttgttttttaagagaaatatcttaaaacactttttatcatactactatgatgatgtataaatctattcaaaaaaaaaaaaaaatgatgatgtataaataatttaaagagttaagtttattagaaattatagatatttatagagctgagtaataaaataatactctacagattatatgtagctgatgtagtgtgtctgctcctgtaagatttcctttttatctccaaaaaaattgcattgatattcgagccttgccgacccccttttcctcttcaaccatttgataagatcctatgcactgagtaatctagtattatatgttagatgttatatattaataagctaaaattgtnnnnnnnnnnnnnnnnnnnnnnnnnnnnnnnnnnnnnnnnnnnnnnnnnnnnnnnnnnnnnnnnnnnnnnnnnnnnnnnnnnnnnnnnnnnnnnnnnnnnnnnnnnnnnnnnnnnnnnnnnnnnnnnnnnnnnnnnnnnnnnnnnnnnnnnnnnnnnnnnnnnnnnnnnnnnnnnnnnnnnnnnnnnnnnnnnnnnnnnnnnnnnnnnnnnnnnnnnnnnnnnnnnnnnnnnnnnnnnnnnnnnnnnnnnnnnnnnnnnnnnnnnnnnnnnnnnnnnnnnnnnnnnnnnnnnnnnnnnnnnnnnnnnnnnnnnnnnnnnnnnnnnnnnnnnnnnnnnnnnnnnnnnnnnnnnnnnnnnnnnnnnnnnnnnnnnnnnnnnnnnnnnnnnnnnnnnnnnnnnnnnnnnnnnnnnnnnnnnnnnnnnnnnnnnnnnnnnnnnnnnnnnnnnnnnnnnnnnnnnnnnnnnnnnnnnnnnnnnnnnnnnnnnnnnnnnnnnnnnnnnnnnnnnnnnnnnnnnnnnnnnnnnnnnnnnnnnnnnnnnnnnnnnnnnnnnnnnnnnnnnnnnnnnnnnnnnnnnnnnnnnnnnnnnnnnnnnnnnnnnnnnnnnnnnnnnnnnnnnnnnnnnnnnnnnnnnnnnnnnnnnnnnnnnnnnnnnnnnnnnnnnnnnnnnnnnnnnnnnnnnnnnnnnnnnnnnnnnnnnnnnnnnnnnnnnnnnnnnnnnnnnnnnnnnnnnnnnnnnnnnnnnnnnnnnnnnnnnnnnnnnnnnnnnnnnnnnnnnnnnnnnnnnnnnnnnnnnnnnnnnnnnnnnnnnnnnnnnnnnnnnnnnnnnnnnnnnnnnnnnnnnnnnnnnnnnnnnnnnnnnnnnnnnnnnnnnnnnnnnnnnnnnnnnnnnnnnngatgatattatgtatcattattatcagtcatttattattgatagataatgttattatttccatagatcatatataatcttaccatatttactccctatgattatatatttctatctattaacatagtaatagtgatatactaacaacgagtatctttcaagtaaataaatcatatatatagggttagaaggtaaaaaagacaatattttatgagactttatttacacccttcgtctcataaactcctttctattttttgtgttcactcgttttctaaagttttttctacttcttttactttttattggataaatactttttccgtctgtatgtgatctacttatattagtatttatagatagattatactcttaaagtattacattcacaaaatcatgtgaattattaattaaagtaaaattatgagtatggtattataacttaaacgaagtagttgtattgtttaaaccaataagtataataacttataaaacttaaaagttgattctacacttatcatgcacttgtgttttgatgggttaaaaattagctagtacataagtaacataacataaacttatctctgtatagtatgttgaattattactttatatttgaaaagaacaaagacacaataagtccaaaagatccgatcttttgattatcaactatgtaagtgtctttcctaaatgatcaatcaccttaattagtatactaaacaggacaattatgacatataacacttttctatttgtacaagttaattaacccattgacattcattcagttagcctacatttttcaataggtagtcatcatcattctttttttaaccaatttttttacaataaccattacctaccaacaacattttcaaataatgaactgaatgatggattccgtcaaggaaattgttcgtggacagtttgtttacctcccaaatttcctttaatctcatgctttctccatcatccaaacaatctaataccaatcgttttctctaattgcataaaccctaattgttgaatcctttaatcttgccttttcacattgcccaattcctttagtatgatattttttattcgataatccctgataagtaaattcactaatctaatttcagatggattgttgtagagattggggaattgaagattttttgccttctttgttcttgtttacaatgaaggatgaagtttcatggaatattgaagagaaatttgagaaaagaaagaaagtgtgggctttactgacgacaaaaactgtcattttggtggtttttttcactaaggcatgtttggcactagcgtttaaggtagcggttagcgatttgacaagatcaaaacgctacttaagaaaatgatgagtgtttggtaagatagtggttgttgtagcaggtagcaattagagtagattatgagtagcggttgtggaatgttactacaagtaacgtttgagatttagaggtagcagtccagcaaagaaacattgtataatagcataaggtagaattaattaaccaatgtttttttatttctttttccttttattgtttattaataattttattttatgccaattcaatgtttattttacaatagcaaaaatgtaatttaaatatttattttaaacataataaattttataagtattttagtaaaattggtaatataaatttttcgagggttgaatattttcttagatgtatacatttctttgaatagttaaaaaatcatatctcctttttgtgtaacttctttgaaaaataaatcttgaatttaactattgaacgaacatatgaaattattgtagttcatttcatattataataaatgttaggtattgtcttttacaatttcaactacttttggcaaacaattctgattaaacagctattttaatcgctgatcgttgacagcaaccgctaacagctactagaaccgctacttttgccaaacatgcctaaaccaagtaatatcggggattctttattatataaaaagttaataatgtgattatttgaaaaaaaggttgactttatatgttgtttaaagaaaaaaaaacatttattaatagaaaatatactatataggtctctatatacccagggcgaaatgaatgtgtatcttttcaaatgagtatgcgtacatgttctgtaaatgcatatttcatatgagcataatgtttttactattattatgcacatttgtgttttaatttttcaaatgagtatgtaaggaaaacatgtattcttggcatgtcagtgttagtgatttttgttgttatataaatgttttcgtgatttgtgaatgtggtacaaacattcatgtgccatggcgtttagcaaaacttttctagctcacatgatgcttcaagctaattgcaatgaactaatataagggagaggacattttacgaattagttttacattgatagtagtttgaagaagatagtttaggagatagtttgttggaatagaagctatgtgttagaattagttatagtcatcaatttttgaataagactcattattatttcaatccttctaccttttaattactagtccaactctcactctttggtattaaattacaccattcctacggactatctaacaactctaaccacggcccatactttttcttcttaacataaaataatattacgcttactaactactaactcctatgacatctaccttttcaataaaataacaattgataactatataacaacttataatctaaaagtaagtgtcttgataagtgtagagtattgtgggacgaagggagtaattcatagcaaatactatcatagcaatacaatactaggagactaagatgtgagttttgaacttcaaaaaaaaatatacgcgacatagttcaccggaagaactgcagcacaacaaatgcaaatggggattaaatgaggagttcacctacatcacacacaagagcgattgaggattttcagatctggaagaagagcgaaaaatcaggcgagagcttcaactttcggagtttaatggaagagctaatgatgattgaattattcagttggatttatcttttgtaagatgaggggatgaagttgaagattgccataataacccttgagggcgacacaatggtggtgggaatggaaatatggaccacgaccgatttatgagtggaaagaattgaagtctctgatacaatgacgttttggtatatcatcggtgctttcatggctgtcagatctaccgaaaggaaaagtagtggtgaaaacaaatgtcgttcaaaccaaccacctttgactttcaatattgaagtgacaaggaaaactggcaccttagctagtgacttggtggagtctttgcgtaaaccggtggaaaagaagcttatctttgagttttagtgtggtcttggtgcttgtttaagtggcttgactatttaggaggaaaaaaatcaattgtgaacaattggtgagtaacctaaaaatcaattgtgaacaattggtgagtaacctaaaaatcaattgtgaacaattggtgagtaacctttaaaccagactcaagagtgggaaagaggcggttagacaagtagatttagaggaagaggaggtagaaaatagattagaattttttttgggagttttcaaatgtagtggtatcggctcataacaaggtggtcaaatggatggagagcttggtcgtttgagtagtctcatggtggtgattataactacgttggcgataaacaagttcgctttaccaagaagttgattggtggaagagagattttcataaagaggggctcgtatagcaacagctttgtgtggtctcagtttcattgtcggcaaagccgtgggtggtaaatatggtgattttggagattgttatgatggagggagttatggtggtttcatgagacatggatgctatggtggtgctgtgatcggtggagaagaggagctcgtgaaaggtcactctgatggagcgggtgtaatggtggtctaggttttttcggcatcggaggttgcgtatctcgtgaaggttcacatttgtacaccggtgaatactatggtggtgaactaggatgacagtcaaggtgaccatagtagaaaaaaaaaacataaaccatgtagcttagatgatttgaaaaaaaatcatgtttttggagaagaatcttaaatattatgacagaggcaaacttgtcattgaccaaatagatgacatagcaattgcacgtgtctcgttaaaatttgaaaccataaaaaattcaaattgcacttcatatgcctttcttttggttgaaaacttcatataccctaatgcgtcaatatggttctttttccaaaaaaaaaagtaaattatttcggcgttagtaaaagcaggtccacctccataatccattttattaagccaactcctctaccctacttttgcaacctatcatttcttattttctaaaatcatatcaaaaaaacaagtgtgaacccaaaactaactatattatacctaagtctaatttcttcatccaatgtgttcaaccccatttttcaacccttccactcataaacccatcttctttcactcctaaaactttcagctcacgctcgtatcacctctttactcacatatcagcccaaacgatttcttattgaatccactaaattatgtatatcgattttttcaccaagtactccgagttttcaaaaaatttacctggtacccccaagttttcaaactacacgggatacccctaagtttcaaactaatacactcagatacccttaatgactaacgacattaatcgccgttagtcattaaccttaattttctagatttcaacctaattaaccactaaccctaaccccaaccctaaccctaataataaccctaaacctaaccctaaccacccctccccaaccctcccaccacccctgccccccatcctccactcctgcgcagccagcaggccccccacccatttgattttaaggaagaaacacgtatcagggaagggggagaacttagctctgacagcggcaacggaccaccgacgagtctggactgtaggacggcagcgtcaaggcgcgagccggttgggctactgcagttcaaagcaaacaggggaggggaatcgagccgagaagagagctaaggaaagaggggtgatgggcgttgcggagatggtgcgcatagtggtggtggtgtgggggagctgtggtgggggagaaatcgaatgggtgggggagagagggtggggggctgcggtggggttggggctggagggggtagggtgggtgggtggaggggtggtggttgggtggtagtgggacaactctcaaacatgattctttctcaaacatgattctttctcatatccttttttggatttccttaaaaaaatccatatccaaataacgttgaccggtgagggacaactctttaacactattctttctcaaatcttatgaaatcttcacatttaactcgatctccctttcaatgaacctaaagatatatattaatagagttgcaaattcctaaactctagaaaattcaaatacaacataagagtcctagattcttccacaagatgtattatatctttcaaagtttcccagataaaattagtaattaggaaactccttaacaaggatacttaaagttttatctaaatcttgcataaattgaaatccaaccataattatgaataaataatcataaagaatcctaacataaataactagaaaataagataataaagaagcaacaaaagaatctcataaccaccatttgaatcccgcatgagaacccaaatagttgttgttccttataaaaacccaccacctttcttcgggtattatgacggtattggactatagtatgagacgagatctcttaatcaccaatcaactattgtaaacttgtgagcctgaataatttatttgagatacaattctaaggttgtttatgaacgtgtttggtaaaattgttattgataactcgttcgtggaaaataaatgcaaaagtcaacatgccaaaaaaagtgctaaaatcaactttcggctttgcttgaaatgttaagttttaagctatccaagagccattagtcaaaatctattgaaagcgtactcaaaaaccatttatcaaacacccctacaaatccctttagaaaacaataggagttgtacaatataagtattgagttataaagttgatcaagtgatttaggaggttgttccaaatcaatctacaagagtttgtatacttataccccttcgtttttttaattgttacacttaggccttgtttgacaaatagagtttagcggttagagtttagattttgctgttagagttttaactttttgttaaatagatttgactgctgatttgacaacttcttcttataaatgtgtttggtaattattaacagattgctaaaagcttattaccctttatttatgtgaaatgacatgtatagacattttaatccacatgggtattattattattattattcgaggcatacaagtcattgaatatatttttacctaatcctctaaagaaaaagctcctattaggagctttttcatttcgagagtttttattccagaactctcttcaaaactcttttttaccaaagaataggagctttttcatttcaagagtttttactccagaactctctttaaaactcttttttaccaaacaccccttttagagtttttgactagtcaaaactctaaaagtggtccaaatttctcttttaactccaaaactctaattgccaaacacccccttacacttttcacgcataccaatgcaacactttgacgattaacatctccagttttttatttgtaaaaattataaagagtgcatattaataagtagggctgttcaaagtgcggtctggaccgcaccaaaccgcaacccaaaccgttgtttcgcggtttggtttggtttgcggttttaaaattgcggtttgggttatgatttcaagcaaaccgcggtttgcggtttgggttgggtttttatttttgtaaaccaaaaccgcaccgcaaaccgcaatgttacattttttttaaaaaaataaattaaatacatttatgaaggtgacatacaattataaaattgaaaaaagaagtttgaggtaaaaaactttaacacttatgataaatcattatatatgtttaattatgaattcagcttcatatctatttggactcttattaacaattttcttttaatcttaggaaacaaaagtaatgtcgcggaggaaataatggttaaaccgcaacccaaaccgcaccaaaccgttttgcgcggtttgggttgggttggtttgggaaaaagtgcggtgcggtttgggttggaaaattttcaaaccgtatatttgcggtttgggttgggttacatcccaaaccgcacaaacccaaaccgcgaacacccctattaataagatacatattaattcgaatttgacaagatccacatgactatgtttttattcgcgtataaaccacaaaagaaggttcaagtaaaatttgtgtatggtgtaacatgtcaatcaaagaacggaggtaatatttgtcaagacactttagtcacttctaaattcctataaacaaagaaatatggaagaaaactggtgatgaaaattgaaaaggtgggtataataagagagacacaattctaaaataagaaaatattaataataaaataataagttacgataggcctcatgtttgaaaacggaaaaaataaggagatagttcgtgtaaaaaggagggagtaaagggtaatgcatactttgtattgcaagcttagttttaaaaggcataagacgcaaagcgcatcgaggcacaagacgaaggcgcatgcatctcgtagttgaggcgtgtaatgattttacttcacaaccacctgagcaacccaatacagaacgaccacaagaaaaatagaaagaaaggaaatgattttgattgatcagcagaaaatacagagcattcgagaggctcagtctctcccaaggactacaagatactactaaatttcacacccccttcagtccccttacacccttatttatactacttctgctctcctattttaacggctactgacattctctgagctggcctgctattcctctttttgtgctgacatttctgaatattctgtggtagtggctccattctcacatttggacaggtttacccctccatttctttcgtgcatacgtcagccacggtttggggattgaattcattacattaccctgcccccaaagactcaccttgtcctcaaggtggaaggaagggaaacgttcttgcaccaaatctgcatcttcccacgtggcttcaaaaggtgctaagtccttccatttcagtagcacttcagtctgcgtatgcctccctctctgtgtctgacgtacgtccaataattcttcaggttccacaactagttccaagtctgctgctagttgagttggtacagtggttgctgcctgggcatctccaattgctcgtttgagctgggatacgtgaaatataggatgtattttactggtgcctggtaactggagtttataggcgaccttgcccaccttttgcagaacagggaatgggccatagaagcgggctgccagcttctcaaatggtcgcttggccaaggattgttgacggtatggctggagctttaagtaaaccagatcccccacttcaaaggactcatcgcgccttcttgtgtcagcataggctttcatcttttgctgggagcgtagtagatgaaagcgtaaatcatcgaggatggcatcccgttcttgcaacacttcctctaagttatctactggcgtttgccctctgcctactcgccacaagtgtgtgggtcacgcccgtacaacaccctgaatggagtcagcttagtagacatgtggggagaggtgttgtgtgagtattcagcccaagggagccactttgcccaagtcttcgggtgccccgccacgaaacatctcagatatgtctcaagtcctttgttcacaatctcagtttgtccatcggtttgcgggtgataggcggtgcttctccttagtgttgtcccttggagtcgaaacaactctttccaaaaagtactcagaaaaattcgatccctatccgaaacgattgatgccggaaacccatgaagttttacaacctccctgatgaaagcttcagccacttgtgagagcactaaaaggatgacgaagcccaatgaaatgcgcatatttcgataaacggtccaccactactaagatcgtgtccacccccttggacaagggcaatccttctatgaaatcaagagtgatatcctcccaaacctgagctggaatggctaagggctgcagtaggcctgctggcttttgttgagagctcttatgctgttgacaaatgctacatcgctgcacgtacaatgccacgtgcttcctcatacctatccaataccactcagccgccaacctaaggtacgtttttacttcacctgcatgtcctccttctggggaatcatggtaagctatcatcaacttaggaatgatgacggaagtgttgggaattaccattcgccccttataccgcagcttgccatcctccaccgtgaaccccacaagtggtttatctccctgcgccacttcttccctgagccttttaaggaaccaatcctcctctacctctttttggagctctgcccagtccactccttgggttgtgattatggtccctagctccatttcacctacagtttttctagaaagcgcatccgcaaccttgttggttgcccccggtttgtagtgtatttcaaagtcaaacccaattaatttgcttacccatttctgaaaatcagcccccacttcccgttgttgtgtgatgaaacgcaaactttgttgatccgtatggatcacaaatcttctccccaaaaggtaatgtttccatttctggaccgcaaggcatatggcaattaattccttctcataaacggacttgtgttgtgctctcggtccaaggagcttgctgtagaatgcaatgggcctgccctcttgcattaggactgcccccaccccatacccagacgcatccgtctcaactacgaaaggcttatggaaatcgggcatagcaagaaccggtggctgggtcatagcttcctttaagtgagagaaagctgaagtagctttttcggaccagccaaaggagtccttacgcaattgctcggtaaggggctgggcaatttgcgcgtattgcctgataaacttgcgataatacccggtcagccctaaaaatcctcgaagctccctcaaattcttgggaacttcccactccaccatggcccttatcttctccatgtctactgccaccccatgctgcgaaatttacatgccccaagtaggccactgtcttcctccccaagtcacatttcttctggttagcgaacagtttgtgcaatgctaacagctgcaacaccaatcccatgtgtcgtgcgtggtcctctttggtcttactgtagaccagaatgtcgtcgaagaagaccagcacaaacttcctcagatatggacggaaaacgttattcatgagtgactgaaaagttgctggggcattggtgagcccaaagggcattacgagaaattcgtaatgtccttcatgggtgcgaaaagcagtcttatgggtatcctccgggcgaactaaaatttgatggtatccggccttaaggtcgagtttagagaagatggtagcgccatgtaactcgtctagtagctcatcaatgaccggtatcggatacttatccggaaccgtctccttgttcaaagcccgataatcgacacaaaacctccaagaaccatcttttttcttcaccaataatacggggcttgaaaatggactagttgagggcttgatgatgcctgcctccagcatctctcggatgagtctctcgatttcgtctttttgaaattgagggtaacggtatggcctaacccccaccggattactgccttccttcaacgtgattgcatgctcatgccccctctttggtggcaggcccaccggagtatcaaaaacttccgcaaactgactaattaccttctgtaaaaattcgggtacttcttgtgcctccttcaactccgcttctccccttttcccatcatcctcaatctggttgagctccaagagaaaaccccctttttcttttcggattgcctttatcatggctctaagtgagattttagatcttgctaaggaagggtcccctctcaatgtcaccactctgccctccacttcaaactgcataacctgagttttccagttggtaatcactgaccccaatttctcgagccactgcactcctaatattaaatctgagttacccaggccgagaggtaaaaaatcctctgttacttcgatttcccccagctttaaagtcaccccttgacacaccccagtaccatggacagcttcaccattccctaaagacactccaaatccccctgcatctgagatgaccaactcaagttcctcaacagttaacaaggaaataaaattgtgagtggcacccgggtcaatcatgaccaccacctctcttcctttaatttttctagtgattttcatcgttttaggactcatcaaaccaatcacagagttgagagatacctcagtaggaagttccggtggtggttcggacggtggtgcacgagctgcgtcgctcacctcttcggtttcttcctcctcgtcatgcatcagaatcacgctgatctcttttctccggcagatgtggccggcggtccacttatcgtcacatttatagcacaacccttttgctctcttctcttgatattctttctcggaaagtcgcttgaactctacagatttttttccttgccccccagcaattggatacgtgttcaaggtgttggaatttccccctgggttttgggcccacattttgctggcaggtgggttgaggctggtcgttggattgaaggaagcccctacactccttgtcattccccctctgttataaatcgagtaaggcccattcttagttggcccacttcttttataacccacaatcctattcctttcctcaattcggcctgctagttccattgcttgctctaggtccataggattgagtaacctgacctccactttgatatcctcttccagcccattaatgaactgacccatgagtatttcttctggtactctactcaacggtgccgccttctcaataaaagtgcgtcgatactcatccaccgtggtggtttgctttgtggccaaccaccgttcccacaatgaaccatagtgggttggtcgaaactgacggaggaggtactccttcagatctgcccaccaccttatcggccgccttttattctcccactggtaccacctgagggcatccccctctatagacacaaccgccgcctccagggcttcactgctactcaggccataaaacgaaaaatatcgctcggctctaaggatccacccatccggatcggacccatggaaaatgggcatctctaactttcgatatttccagttccccccggaagtcgaacctcctggccctccacctgagccgccatccccatacgatcggcccccgagctggaaacctccatattcgtccccttctcggccccccagatttatcaggtcaggagccctccgttccggcggtcgggggtgtccagtgacggtttcgggtgtctcccgcgagggttgtggcaaggttgctcggatttcaacctgaaatttcctctgttcagcacgcaacccttgaatcgtcccatcctgtgtctcccttgaccggttaatccggtcctccagcctaacggccaagacctccatctcctcgcgactcttcctcgccgcctcattctggccttccaagatttgagcggtcaacgattcccccatggcattaatggcagattccaccgccctggacaccatggtggccactgacccttcgagggctgccattctttcttctaatgaatccaccctctgcacttcgtttcttggtgccatggatcgatgctctgataccaagtgtaatgattttacttacttcacaaccacctgagcaacccaatacagaacgaccacaagaaaaatagaaagaaaggaaatgattttgattgatcagcagaaaatacagagcattcgagaggctcagtctctcccaaggactacaagatactactaaatttcacacccccttcagtccccttacacccttatttatactacttctgctctcctattttaacggctactgacattctctgagctggcctgctattcctctttttgtgctgacatttctgaatattctgtggtagtggctccattctcacatttggacaggtttacccctccatttctttcgtgcatacgtcagccacggtttggggattgaattcattacaaggcgcacctttggtaccaagagacttagacatcaaataaagaagcattgtaatacttagaataaacattgtttttatattctaaaacacatattttctctaagacacctagtaatctcatagtggatgtcatctagtttaggtggtaaggttttattgagttggtactcaagacctcagacttagaggtggcaaacggatcatacgggtcgggtgaaaatgagtcgggtcataatcgggtcacctttgtgtccaggttacggtcaggtcgagttcgttcgggtacgagttcatattgagtccatgaggtttcatgtcatatcgggtcgggttagattggatttacaatttcgcaaataaataaaacgcatataatactaaagagagtaaattaaataattaacggacactagctaaatcatatattagtattttatgatgtattttccttaaatttatttaaaaaataactaatatgacaatttttcgggccgggttcgggttgtggtcatcattatcgggtcaatttagtatcgggtaggctcgggttcatgtcatattcgggtctattttaattcgagtcgggttatttcggatttaagctctatttcgggtcagtattttcgatgaagaacgggtttcggatcgggtcaccggatacggatctattttgccgagtcagactgcttttcaaacctaataatctcagtttttccacctattcagatttgcctatgatctctatttagataaatgagtacaatattgtgtctatccatgaaaatgaatatctcacaatgtaaaaggatatctctaaatttcactaatcactctatctgttttgaataataatattctattttattgcatgtagtaaagatcgagtatttagtgagatttggagaaaagaggaggctagagagaaactaggatttagagaggagaagggggctctgtaacacatacaagatagatactcttttacactaacttttcaagatactcaacatataaaatcagcatcatcttccaaacaacaactttaagccacccatgaatcttaattagataataaaacataatcgtgaatcatctatcctttgtttggggggatcctaaagcaattgaggaaaagctttgatgcaaatatcaattgtgtaaaaaagcaagtattcgttcgtgatgttgctatactaggttattttttggatccaaaagtcattcctactagaatcatttaggaaaattgtcagtatgaattttaaattcaggttataaccaaagataattgaaaattgtcaaacttttcaaataattccgaaataaacatgtttgtaacatggataaacttttcattgcttttcaaataattccaaaataaacatgttataacatagataaccttttcagataattccaaaataaacatgttgtatcatggataaacttttcattgtttctagtcacttaaaattctaaaaaaatctttcctccctactgttactctctctagcaccaaatctatcacatgagaaggcagaggttttcaaaataaaccgttacttaatttggtacttatttcttgatcggtgttcatatcatatgagttcctactctatatctctctactcttctaaatccttgtgtcacttcctgtgtttcataaataaaaaggaggaagtattagttttgaaacgaaaggagtatggtgcatacattgatagaaaaaagaagttatttgtccttatttcactcatataacaacaccaaattctgtattgttatcacaaaataaaacttggattatctttgtttcatagcccaaatttagaattagtttgtcagatttccaatcatctaattacaatattagagctagacctaggacaaaaggtgggtttggctacttggtaatagctatgtctagtgctaggatatgtcattgtcgtagaaccatgttatggacatcttaagaaacaaggttaacctaattggttggagatcctactttcacttttataataaagtttcgattcttgcctatttgtaaagtagaattcctaaatttcccttcactgatatttatcttaacataaaaaaatgttataaacattgggattgtatataagtcaaaataaattgacaatcttggtaacaactaagttaacattaattttataagtaaatgattaatcccaatataatctcttatttagtaaatgagacaaacttgtacaccttcgtgttagactcgttaatgttcgctaacaattcattcagtagtcaacagcattttaaatttgaaataagtgttcttgtggtttttgagagatcaagcaagaaaacatgtctctcccctttgaccaactaattgggattaagaatactagttttaagattttaagaatgagttatagtctttcttagaccgctacaatccccttgttgatatgaaccagatatattttgtgttcaaatagtagatcaatgcattgttgataatcctttgttaatgtacttgttgatcttattttgtacttttggtagatgcgctatactttctttcgattgctcattttgaactcttaactacatatgttagtttaagtagatgatttagaattgctatttcaatcttcaataagcaatttaagttgtcaaaccttgtttcacatcattagggtgaaagttatttggataaagacctatatctaattcaatccaaagcaaattagtaatgcggattggactcaaactatgtttagattggattcgaattgagtttcttttctttttcttaaaaaaattggattttccgatcgaattgagggtgattagatccaaaataaccgaatagtagataggatttgtgttgtatattagaattgggcttaaggatttccattttaacaaaaaaaccaaatggtccgactatcaaaaactataatttgatagtcatgcctatcgaaaactttattttcattctcgcacctaattatgggcttgtataaattagttctactatcgaaaactaattttgatgctcgtgcctaatttaaattttcgaaaaaatgaagttaagaaaattggatatttcggattggatccaatatatcttgtgaattattaatttggattagtttggactcaaattcttattggattggattcaaattaaaagattaaaattcaaattttgttcgaatcaaattggagtaggcttaagtttaaatcatacaccgaactttcaccactacccatcatgcttaagcttctaatgtaagagagtgtttgggagttgagctcgaacaactaaatttctaaaagaaccaagttcaaacaagaaatctaaaagctcgattaaacttgagtcaagctcaaacacctatattccttattggagcttgactgaagattgaacacttattccttattaagctttacgctaaaacattgctcgactcaactcttctacatccctatagttcaaaagaaatagttgtgggctgtggtgctcttgtagaccaacgcactagtttaacaaagctaagtgcctgactgcaattccatacacattacgatcaccatgacctagtttcagctcacactttggaagtctaatttgaacttgttctctacctccaattcattgtggggtaggaggcgatagttaagggatcaaaatcttatgatataacttgcataggctatgccactatataatgcgtcttgtgtcccatattagtttaatcaaattgaaatgttttaccatttatatcttcaattatgtatggatactaatatttgatttgacgtttgatatgatattaaatgtggactgttattcttgatgtgcttgagaagcttttttggggccagttagaaactatattccttttatggtcctaactaggttgttgttggtgtgttcccaaataacagcatggaaaggatactcgagcgctatgaaagacactcatatgcagagagataactgactgctccagatcctggatcccatgtaatccagctaggcaactatcttttctaagcatttaaatcgttgagatttcaattttaaatgtgttttaactgataattcatgcattatatgcttaggtaagtttgactctggaacacgcaaaacttaaggctaggctggacattctttagaaaaattaaaggtaataagatccagaccaaatataatttgtataataaccaccttatgaggaaaatttaagatccttgataatttcaggcattacatgggagaagaacttgataccttgagtctcaaggagctttagaatttagagcattaaattgacagtgctcttaaacacatcaggtcaaagaaggtagtttcacagttgcattagatcatcttatggatcaattggatcacttgtttgtattttagcgttgctcaacacggtcgtctaatatagtgtgcaaaacgacctacagggcaacaccttttatagggctcgaaaatacgaaaaattaaatgtttgttttagtcatattgttcaaacccaagctttatcttgtcaaaaatattttataatgattattttttagaatacattatttacatttttgcaatttatgcataatacttctaaggtccaactttataattgaaatagaagtccttaaattttaaagacgaccttgaggaaacctaatttcttctcatatataattaaatcaattattctacaagttagtagaacaaatactacaataacaacaatattgaagccctaatctcagtaggattggattgattgtatgaagtcttattagtggccgttaaatgtttcttgtaggtcaagatgacatggctcatatagtaaggttacttgactaaaagacgaggatttgtttcgacttagattttaacaagtttccctcatttgttaacacctaagcgtactaaatcaaattctaggttttactcactcaaatttccgatttaggaagggcttgaggatagttgtattatcgtaactgactaatcaaaggagcctctcttagatcaggtttcacttgccaattctaacaacttgtttggtaaaaggaatttggaatgaaaagaaaggaattgaaaagaaacattctacttttcaatgtttcattcaaaaataacattttaagtgataggaaatggaaagaagtgaaacgaaagcctctttacaaaattatcatttttctacccccccccccccccaaaaaaaaaaaaaaaaataagtagtaagtagtagaagaagaaataaataactaacaagagtagtaagtttttacgttttctttctnnnnnnnnnnnnnnnnnnnnattcaaatcagaactgaatagtcataaccggaagattagtttctctctagcgtgactagggtttgagtaaaaagagaaaacttaaatcaaacatgggatattaaggttttttttcctttcttcagttcttttctcttcccaatcctttcctaaaaatgaaccaaacaggctgcaaggttttcacttgcttaacacaagatttatttttaaaaataattacactccaaacttttaagcttaaaaccaattttaattcaaatcagaactgaatagtcataactggaagattagtttctctctagcgtgactagggtttgagtgaaaaagtctagggtttcatgtcattcttcttgcttcgagtcccttcttgggattgttgttagccattatggctaccgaaatcgttattaaatgtctaaatcttagaattactgctgaagaaaacaacttggtgtttctcgaagatgttgatgataactcgcagcaccatacgctcgcactggcgattgttggaaaggttctttcgtcaagaccatacaatttcgaggcacttaaatgaaccttaaactagatatgggtgatatccaaaggagccctacttcaccctattgaaaacggactttttgtggtacaatttgcgacaattaaggaccgatctaaggttctagtcagcagaccatggaccttcgatataaaccttgttctcttagatgctattgaagggggtactcaatcttgacccattgcccgttttggactcgcttgtataaccttcctatggactgccgatatgagaagttcatcaaaaactattgttggtgtattgggggaggtattggaagttgattttgacaggattgtttgggataaatctgcaagagtaaaggtgaagattgacattacaaaatcgttttgtcgtgtgcagatgatcaagactaacaggggtgaggctgtgatgatcaatgttaagtatgaaagacttcctacaatttgttatgtgtggaattctggccatattgaaagagattgtgtgaagacccaggaagaagagaaacaagtggagagacaatagggggtcttggaggcctctccgcgtaggggacgattaaagatggtgaaagagtcgaaagccttccttcagtgtgctcgtacactccactttaataacaaggaagaagtaaggggtgaggaaccacgggattatgtggagccgaggggttattgtcggctatcttagggggtaaaactttggtggtccaggagatagtggacggctctaaggatgccatcgaggaagttcgtgctgaaggtgcaccactctagcccccttgtaccctttgggtaatgccatgctaccttttacttttgctgttgggagtgctaatcctactccctcccaccgaaaagttaaaattaaaaacaaggcaagggttcagggtgttttgaaccaagttaatgttgtgggtgttggggggttggctaataatgggggttgtgagaaaaggatattccccaacccgatggtgttagaaaaagaaaaggggttcaatgaagagggtttaagatagcaaaacgagaggattgtatgtaacctatcagtagggaggtaactattgaggtggaggtgggcgagacccaaccccgcccgacattatgaatatcctatgttgcaactgttggggattgggcaacccccgggaagttcggatgcttcgtaggtggagcaatagtgctacactgagttcggtttttatttctaaaactatgattagtggtcgtgatgtggaaagggtgcaaagcgggtagggttttgattgggcaattggggtggatagcgttggaacttcaagagtttggtgcatttattggaaagctggggaagtggactttactctagtctctctatcaagtcatcatatttgtgggaatgtgaagcttgttgatgggaaggtatgatgcttagtgagtatttatggttgggcggatacaattcaaaagtataaaacatgggagcttatgcaatcctttcactcatatcatgggccgatattgtttggttgggacttcaatgagattttgacaatcggagaaattgaaggagggtccgaaactcaatgaagtaacatgcataattttctagaaactttagatgacatgaagcttagggaccttggctattcgggaacttggtatacataagagagaggctttaagccacggaagagaatgagggagaaacttgatcattttgttgcatcttcatcatggtgtgacttctttccgaaagctacagttgagcacttgatgcgctacaaatcggaccacactcctattttggttcgccttgtaggccatcagtgaagacataagaagaaaaagacgtagttttgttttgagactgcttgggtgcttgaggaaggttgtgaggcccaatgggtgagtcatgggccgggtttactcgcgaggtatttatcgagcgctttaaagccgtggaaggtgggttcaaagcaaggagtgatgggtctcttagtaatctgggcccgcgtgtgagggagattgaggaggccattatagatgggaggcagcgaagcagataaggactatgaggctctatgagactcctctcccacgaaagttagacgaggtgttggacaagcaggagacgttttggtttttgaggtctcgtgtgagttagataaaggatggtgatcgtaatacacaatatttccaccacaaagcttcccaacacaaacgtcgcaactacatagcggggatgtatgataataaaggggtgtggcaagataacgaagaggatattgaagggaatatttcagagtattaccaaacctcgttcggttcgtgctccccctctaggaagaacgtcgcggttgtccttgaggttgtgagcccggtgataactgatgatatgaatatggcggttatgaaatcttacactaaagatgaggtgtgggaagcactaaaccacatgaagcctaacggaatgcatgccatcctttatagaggttctggaataccttggagatgatattacatctgtcattttaggtattattcatggcacccgaccccagatgtttttaacaagactaatattgtgctcattcctaaagtcaaatccccaaatcttgtttctgagtttcgcccgattagcctctgtgatgttatctataaacttgcctcaaaagtacttgctaacagattaaaacaggtttgcctgacattgtttatgataaccagagtgcatttgtgtccggaagctatattacgaacaatgctttgatttctcttgaattatttgactctatgaaaaaatgatacagagctaggaaaggttttgtgtcgatgaaattggatatgagtaaagcctataaaagagttgagtggtgttttttcagtagtgtgttggagaagttggattttgctgaatcatgagtgaatgttgttatgagatgtgtgtcttttgtgcagtactcttttgtggttaatgataatatatgtggagctctgacaccctcaagggggctttgacagggagaccctatatccccgtatttgtttatacttgttgcagataccgttttagctcttcttagcaaggcattcaacaatgcgtggctatacttgatattctcaacaaatatgaggcagcatcaggctagaaaataaatattgacaagtcaggaatctctttcaataaaagatttgacgtattttatggccatgaaacaagttgagaagcatcagaaagacttggtatcccaactttggctaggagttcgaaaaaagtcatatttgctgacattcaagagcgaatttggaagaagctgcacggatggagagaaaaacttctcgcgggcttgaaaagaaactctcttaaaagttgtggttcaagcaattctaacctatttggtgggcgtttacagattcctaaccagtattatccaggccattcatttggccatggtaaagttttggtgggggtcgaaaagggcccacaattcgatgcatctggggggatatgtgctcaccaaaatgtttaaggagccttagctttaaagacttaggggtgttcaatgaacctaaactaaggaggaatgcgtggcatttgattcctgctggtgagtccctttcgggtcgagtgttctcggccaagtactattcgaagtcaacctttttggactcatttctaggtccggtaggtagcttctcttggaagagtatttggggggccaaggcattagttaagggtgttttatggtgcgtaggcaatggcagacaaatcaacatatggcgtgactcgcgggtgttgaatggtgatagtaggttcatccccggagagcgcgtttcaggccttgaggatgtttgtgatctaatagattttgcacaatggagtgcgatgtggaccttgtcacgattgcttcaatgaagatgatgctcaagccattttagtcatacctctaagtaagcgccttctgaaggacatggtctcttgggctttcactaaggatgaattttttttgtaaaaacaacctatatggccggttggtcgaggaatttgaatttgtttcacaaagcatggctgcaaatctggggccttaacgtgtctccgaaggtctgccacttcctttggcgtttatgctcggtacccttcctgttcgagctcttttaaaacgacgccacataactgatgatgattcatgtcctttgtctaaaggagcccggaaagcatatcacacgcgttgttctattgcccatatgtagccgaagcatgggagagtgcgggcctcacaaattgtttgcctttgtttgatggggctggtatgcttgatgcgtggggggagtgggaaacaatcgatgactagtcccttgtaagacttagcttcttggcttatcacttgtggtttaggcgaaataaatgtgtttttgaaggggtggtgagagcgaatgagagtgttgtggaatatgccactaaagctactgttgatcatggtttgtatagtgcccgcatttatggtgggtcgaaggctaccgcatccaaaagctcgaaggtatgggttccccctccagcttgtcgtacgatctaaaggttgatgcatcagtggggaatggtggatgggtggggctaggagtaatcgcctgaaactagaaaggggaggtgctcgtggctgcaactaggagggtcagagcttgtggcccgtggaaatggctgaagggaaggctctttgtcttgctcttaggcttgcctcgctcatacaacttgcaagaagtgatcgtggagtttgactgtcaatcttggtgaaccatctctccaagggtgctatttactttgcatttttaagtcaaagcttgaaccttgataaaaaaatcccgttcgacatgaaaagtgccttgattttgcgggtttgggagtgccttattgattctggggtttgatttgtaacacctttagtaaaaacatgtaagctaactgtaaaacgaacattaatcaaactaggatatgtaaaattcctaaatcaagaagaatttccacttgtgctgaatttgtccaccttgcatgacacccaataaaagcccatgtctcctagaaccccttatgccgccttattcatcttttctcaagttgagttggagtcctctatggtccactcgacttctttagcacactctcggtaaaaacttttaatattattttattttagactccaccatcttgacatttattccttcttaaacttgcttcacacaaacatctaacactagaattctatatagaatagcttgaatctctcttaggataaccttatagtaaatgcaactacgcctatccttaaacctttctaagaggagctttatcgtatttacattcgcttcactttgaaacgtcgctaagtgtatgttgcactttccaaaccatgtgttagctaagaccaagttatatgactgcataacctaaatagtcttcctcgagaaaattcactagttggatcggaagagtttgtgtaaatctatggcggcgcgggactgggccttcacgatttcaagtgttttaatgcagctcttctaggtaaacaagtttcctaatagcgtggtgactcaaatattgaggacttgttgttatactaatgctattcctggcggcacttaaggggtgaaataggtggtacaaaggagtgcttgatggcgtgtgggtagtagttgaatatatcagtatgatcaagtccatggatccctcgtacttattcgtgcaagattatttttccacgaggcaaagcgagcgagaatcttaaggtttatgatcatattcatcttgtacgtgctaagggtaatgtccctttcaataatgagctatttctccttttgagcaagagcgtatcttaagcattcctcgtagttctcgtctccccaacgatgttttatgttggaatctgaatttggagaaagacggagacttttcgttcggtctatcgagccattcttttgagttggatggcgagagcgtgatttcatcgtcaatacgctctaatttatggagtataatatggcaggatagtacctttcaacgtgttaagcttttatctgcattgtcgacacaaaggggattgagtaagcctgtgccgagtatggaaccattgtgtaatctttatgcgttggaggatcaatggagctacacttcttacgagactttgttattggaagggcttatatgggatccaactagggtagtcaaaacattggtcggggctgcgctgcaattttggggacttggcaccggcgtttttggagtagctccctcatgtggaacataggcttttgatgacgatatactaggctagatggaatataagagagaggtgtttgtttgaggaggaggtttgtgatccctatcaaaccacatgcataatctcatggcgtagcttcatgtggaacactgacatattgcatgtgtagggttaggtgcttgcctaggacaccacatgggaagagctccgttaagcttaatgtggatggagggtgtgtggaagggttgggtgcgtccactggagtggtgattagggggatggatgaaaaagcgttgtagttgcaacatagaaaggtggaggactgcgaggaaccgttaaaaaggctatattttatggtgttcatttggttgtggaagtcgatttttgaaatatggttgttggaagtgactatcttcacctcgttgaagcaacttcttcaaaagtggaaggcaaaaatagcttccatgttattgttgatgacattgttcatggtagtggtatgttaaatacttcgtcttgtagttttgttcgtagggatgggaatagggtttctcacgaactcccccatggaaatatcataatggctcatgctcataggtaaatgaataagctaacaaaattgttcatctttgcagaactaactcatgcatgaatcgatttcttagctttagtgaaaggtagacagctctagagagagcatctagtctcaaaaataccatgagattctgtagtgtcctgacatgttttatatgacaggacaaagcgttaaaggagcacaacaacttgctatccaagaaggtataagttcagcaagattgtttagtaacattgttaatcttgctgattgctttgaaacatgtcttgctatggttaacaatgttgactgaaccaaaataggtgaaggagagggagaaggtgctggcttagtaggcagaattggattagtaaaatcatgacaataactcatctggctttgtgatgtcttaagctttgccctcactgaatacagggtcagtcctcaataacctctaatcatttttccaagatccaaagtaaacatggtttcataatttaattaagatttttttgaaccatgtctccatacaaccttactaggactaatactactaatttaagaccccaacgataaacaacaataattagccatatctggctagcaccttttggacaacacaccacatgagactcttggccaacttctttgatttccttcagtctgatagatatgaatatcttctgaagagctctttggttcataattattgatttagaaaagaattcagcaaggtgagtcatttggtaaccttaaggtcattatgggggtactaaatcaaagtgaagatatatttaggtggcatcagaagagatgatatagataggttgtatcctgtcgataggttatttggatatgtatcaaaagtttcttttataatatatctatactgattggttgatgtatcaaatatccctacagattgtgaaaaaatcccctacagattgtgaaaatatccctagaacctgtgatgatataagatgtgctccgcatgctttattgaacataatgtattcaattcttgaaatgcagaggaacaagcagcagtgcagtggaagatgaagcaacataaccaccaaatctaaacagcaactctgcataaataccgtcctggatgctttaacacatctaagagcagtaa

SEQ ID NO: 39 - DNA, 21668 bp, Artificial Sequence
  BvAP1 genomic DNA showing  mutagenesis site at position 6999
  mutation (6999)..(6999): c to t
  misc_feature (9833)..(11385): n is a, c, g, or t
  misc_feature (12467)..(12605): n is a, c, g, or t
  misc_feature (13741)..(14088): n is a, c, g, or t
  misc_feature (16396)..(17194): n is a, c, g, or t
atggggagaggaagagtgcagctgaagaggatagagaataagatcaacagacaagtaactttttcaaagagaagaagtggacttgtgaagaaagctcatgaaatttctgttctttgtgatgctgaggttgctctgatcattttttctcaccgaggaaaactctttgagtattcttctgattcttcgtaagtatatatatatatatattaatagtaactacttgttttctgctttctatttttaggtctgatgcatatttaatttaggtaatattaattccttatatctgatccttaatttttttttcttttaccatttcatttttgtttgttttgaataaaagaaaatttccccttcacgtgtgtcgaataggtcaaaatttttacttgaaggatgttctctttgattactaaaataggatccaacaatcacctgaaataaaggaagaagatggtgcaaagtttttactgtcatacttagtatttgataaatattctatgatgaacttgtataaattaggaaatagacctaactttcatgcacgaaaacattattccttcattcaatttttttattacttaaggatttacttttttattgatcatatgaagtagtagtacttgtaatcattcaatttttttgttggttaaataggactacattttaaaacaacccaattttaaaattttttgtgtgaatttcttccctttttaaaaataaagtctattatcatagcttagagtagctgtggcaaagctagacgaaataatacagaaatctggaaaggaaattgtactacttacatgaacacacttatttattacttgcatgatatctgcgaaaaagtttatagcaaatttggttaatatatagcgtagtactttggatattaatattactagtgtacaaatacttgatccaatgggtaatgaaacttatggaagatttgaccatacatgatgatgctaaatattaattgttattgtccagctttgttttccctccatccattggcatcttcatctttacattgctactccactcacttgtcaattgtttcgtcctttatgttctttattcacatgtgcaccatacttcaatactttccccttctttatcctcagtttttttttcttgtcattttagggttaatatccaatgaaatctagtttgctcgttttagatctaattttaattcgatcacaaccatccatatttttgtttcttagcttgacatctattctatggatctgggatcttcggtgtatagatgttctcggttttcagatcaagatcctattcatagacccatttattgtaaacacttaaatgtgttcttaaaaagttagtggctcgccaagtcaactcaataacataacccccacgacttcattacattacacaatgaaagattagatgtatgagtttgtgaagcttataattctatttcaagtaggactaggatgttttgtgcaatcagcagctagtagtctttttaatttaagtcagtcttcattgtgcatcatatatttttagaaatatatgcaagtttgaaaccatttagaacctcatgacccgcctgactcactataaaccggcaagagcttaatttttcacagctttgtatctttatgagtagcgctagctaggggtatgggcatagaaaaaaagggtttgggttagggtcttacaagatcttatccgctatttttatttcataatctttcaaaatacatgtttaataattcaaaatacatgtttaatactatctccatttcacaacatatgcaccaattgcctagctatggtccaacctagttggtttgtagcttgcattggatggttaggatgtattggagttgtttatgtgcaatcaaattttaattacgtatcaaaaaaaaaaaaaaaaaaacatatgcaccaatttccatttggacacacttattgaccaatttttgacaatatttttctcaccattttgtaagaaaaatcaaaatcaagtggaattttgttaagtttatctcagtcaaaagattccatacatcgacattttataatttttaatcatacgcaattagaaatatcaatgtctaaagaagcgtgttggaatacgtgaaaaagcaaatgatacatgaaacagatgtagtatatagaaaacttaattttgtgtcactcggatgtatgtgggcggagccttcctagaaggcgtacccaccttagtggctctgaatctttgacgacccgttcggttggtggtgataatagatggtaatagtaatgtaatttagtctaaatttataaataaatattaatatcattacccatggtaatacaagttcttcacaaaacatgtttcatttaaaaattatcattactaccttttcaagtggtattggatgataataaaattttaggcagggaaatgggtattgggatgaacattaccatgggtaatgacatgcaatttttgttacaagaatacagtataatacattactattgccaccatgtataaccattaatcaaatggaccgtgaggatatgatgttgaagaagaagtcttaacctctacgctattatttactagggtctgtaaattttccttttttaattataattcttgtgaaatcttcttcactgatggtactagcttattaggatgggtttctttagtatattgaaggctcttgttgacagagtataaaaatatttttggggtcgcaaccatcaatttaaacttttgtttgattataaaattattttttgaacatcaacaatctacttaaatttttggttgagttagttctttgacatggtatcacaaccatcatgacataaaggtctcatattcaaatctcattcacctctcatttccaagtagaatatttacctcaggtatgggtatgagggaggcttgtgttgcatgagtcaataacggatcttgaccaataatttaacaggggcgagttgataaattaagttttaatgtaaaattttaaatgatggataaaaacactaatacacaccaaaatataaatatacttttattaatggttacaaagagcttgtagctaatgtaataaatcaaaatcccaaaggtgcaatttttaagaaattatttccatttatttatttgaccattatgaaatcttcaagaaattgagtaagtttttaagaaatttaaggtatagttcattaactaaataaactactccagtaaaaaaaaattaccaaactgctttcttaagtaaaaaaataaataaatttatattttatgattgttaggaatgagtgtgaggaaataaaaagtactattatagttaaataaaaatgaaagttcttcagagaagaagaatagaagatagtacaatcaatgttaaatatttttctaaattagacaaattgatataaaccaaaaataaaggggaagaagaaagaaataagtaaaaaaagaaagaaggaaaagaaaaaaagaaaaaagagaagcaagtgaagaaaaacaaagaagtccaaatgtgtgttgatgcaaggttcgagcttgcaacattaagggctcaaactttcttttacactttggttcactgccaccgtgcccacagcttgttatgtgacatgaagtgtagtttgcttaatttatcttatacagttatgggggaccaagcctccacccgccccttctataatctgtcagtggttgcatccacactttaagtccaatagactcttgtctgagaggaggtgatagagtatataaatatttttggggcctcaaccattagctcaatcttttgattaagttggttctgtgacacttgtactatatactagttatatatatactgtaaaactagtaccacgagaacagtccttaatacaaacaacatgcccttaatagaattttcttagtatacacttaatataggttgactagctttttgcccttcagtatgcacacaccttttataatctgtatcgttgtctggtagatgataataaacctcagtattggcaatatatgaaatgacataatggccatgtttggtgattagagtttagagtttagaggttacagttcagagtttgtggttagatgattacttttttgttcagaggatttgactgctgatttaaataattgttgtgtaaaggtgtttggtaacacttagcttattgtttagagttttgtactttttagagcatgtaaaatgacatttatggacatatgtatttttttaaaacaaattttagtagtaattatatggacaaaatagtcatttgttttttctctctccaaaactctcatgaaaaagctcctctacccagctttttcaaaagagagttttgatcagagttttcggtacaaaactctctttagtcctctctctcaccaaacacccaaattagagtttttattggtcaaaactctaaactctctccaaacctctaaactctctctaaaactctctcccccaaacacccccaatttcttagaaaaatttgttgctcctttttattgcactatatttctatctccaaacataaagtttcttttacaaattttcatttctactccataccacctttatatggcaatataatttctatgaattaaaatgttcacaagttttgaggtggatttcaagagcatggacaatatgatcatgagactctccatacaaaaattacccttaaattttataatcatacaccaagcggtcgttaaagtattggaagtgcttgagtagtttgtgaaaattaacatataataaagtgcagatctcccctctagtaagtagtaagaagtagtaagacgatgtccctcatttgagaaagagaaaaacccttatcagtttctcttgtttctttgactgaacgcaagtcaaatagaagtatgtaactaggaaatccttggagaaatagattttctttaaaactataaaagtatacctatatatatggtaacccacaaaaatgtatataatctgatcaatatctaaacaaagtattcttatgttttctttcatcttgcttatttcctccctttccttttcttactttaatttgtttactctctttaacttatttctttgcgtatctcatttcactttacaaggatatatagttgattatgacagcttaataaatatattttggaactaggatttattggttgtcgttgttattttaatttctacactgatcggctagagtttctagaacatagggctttattgaaaccattagttaacaaaattgaatgacaatgattcaatatgatagaatatgtatgtattagttaatgtttgattattgtttgtatgtatataatcaaagattatttagtaatacttctatatacatattctattagaatcacttagaaagacccattgaacaataataaggataggcagacaagcaaacaaaagaaaaataaacctgttactccttccatttcttaatgttctactcggaattatagatacacactttgacacaaattagaaagagagtgtaaaaagtggatccatattaatatttttatttttttaaatgaggagagaagtgtgggtttattatgtttcaagggagatagagagcattgaatagtgagagaatatgtgccaaagataattaaatcattgtaaatcttttgccaaataaagaataaagcatgtgagtaaaactttaaaaaatgggcgaaaaaggaaagttgagtagaactttaagagacggaaggaatatagaagaggacgtgacagatgggaggaagatcagacatcttagaaggggaatagttaaatttgagatagtcttttaattaaggttctcactaaagaagatataacagtaggggaaagctaaaggttattcaaaactttccttcccatcttcatcacttcatgtctttactttagagctcttaacacttagcctatgaaattctgaactctttgtaagattagtgatagataaaagaatcttatcaatttaatttataaatacaacaggattcaataaaaagatatagagatctataaataaagagccatactgttgtgaacttttatatctatcaaaacctttgcacattagacgtggtataactaaatcaggcttatcgaaattttttaaaattgttttcattatagcccctttatatttagaagttctaagatgattgcatagatagttgatgcaccgttctggtcgacttttttaaacacttctttttgataaatttttttttttgtattcgaatcattattttaggtgtataaagagctgcaaatgatctagatgagattgatctcggtttcatttatatgctaatagtgtgttagatacacactattaaaaaagtcatatgacttagagattattatggaaaagggatagtgcaccgatattaatataatggaaaatgacacacgagttgtccataataacatgtgaaaagtgaactatttaaaaggtttttctgacctagtacatacaaggtgcgtaggtttagctattttagttttttagttttattttttaaagtgaagttagttattgatctgaaatcatataacatgtacgtaccgtagatataaaaaactaccaagtatatatcaatttgaaataaacattattttaatatggcaaaatcacaattgttgactagacctaacactgaagaaaactatgtcatgtttatcaattatgttgcatacagttaaaaacaaatatgttagagaaatcgttatttgaaatagaaaagttgcgcaaaatagtgattaacatcaaaatatgttcagaaagtttttataaatatgtgatcttgcattgtctgttgactgtcgaggtttatgataatttcccctttttccaatgcaaaacttgttgtgctattttctaatgatatattttttcaaagtatggagaagatcctagaaaggtatgagaggtattcttacgcagaaagacggctagcttcaaatgatccagactcataggtagtgcatttatgtaaatatagatatactcttcatgcccaagaagcctgaattttttatcccactacgtactgcaaagccaagtttaattgaataattgtcctgtttaaattatttagttttcagtacaataatgtaatcattagtttgcatgtttaaaaaagaaaagcacaagttctgatcaagtgaaatataaattgtaacgaaagagccaagctagacaattacctagctaggagttatttgttatcgtttttgtttttaatttctagtttttttttttaaactagaaaatatagtttcaatcttttgttatcagttttcaaaatgacatatttaacataaatatgattgattttaaattcatttattatatcatatttcatttcaaaataagtgaaacacttgtctcaaaaagctcactctcacataaatgataaaagtgtttcacttattttaaaacggaagaattatgacttttacttttcataaaacgaaaaactgaaatatgacaataatctcaaatagcttggagaaaccagatttctatatatttccgtgatgaaatcacttttcattatacgtaggtaaactggacctttgacttcgcaaaactgaaggcgaagcttgaacttctacaaaggaatcataggtatgatggcaatatgtcataatttttctattattatttttgcttccaaaaccagaccatatgtttgtatatttatatagtgatatactccatccgtttcattttaatctatacatttacacttatcaggtatgtcaatgcaaaattttgaggatatatatctttagttttgtatttataaaaattataaaaagtacatattaataaaatacatattatgatgaatctaacaagatcccacatgacgatatttccgtccgcgtatgaataacaaataatggccaaagtgaaatttgtgaatagtgtaaaatatcaaagtgtaacaattaaaataaaacggagggagtagtacttgtttgtcacatacttacttatttttgttctctccacaatgaaactgttctttctaataattaaaaaaagtgcatatgttgatgatttctctgtcactttaagtggatattgaatagtgataatggattactttgtgtataattgcatttcacatttgggtctaattttatacccttttcgcatatcatgctttgtgaatagtacatatgatgttcaagaatgtgagaagacatatcatacttttgatatacctcaaacatgggtgtatactgtatagtgaacgaaagtgttagtgtaattttatttaggaggtttagtggtttgtcctatatataatgctagtagttatacaccatagttgttgatgagcatcaactggctttcctaacatttttttctccataactttacccttaccttacattagattactctaggattacattctacctaaaatattattactcccatcattttaggtaaatatttttactttgatttttcgattattttcaagagtttaaaataatgattaaaatttaccatgatcaggcactacttaggacaagagcttgactcacttaacatgaaggaacttcagagtttagagcaacaacttgatactgctctcaaaaatgttcgatctaggaaggtaagaaattttacttgtctaccgtagtttcataataaattagtatttgggctcgggctttgccccagattggtattgtcttttcaaatttgatatgcatttttttccatttccactaaaatatattaagaaaattcaacatttaaaggatacaaatataataatgtggatacttaaagtatgattaaaatttggttgagatggtaattgtgtcatgtataatagcaagaagtcacaagttcaaagctcgttgcaagctaaatttatttttgttgattgacatgacttatcaacacactggacaattctaatcatctagtggagtagcatatactagcaatttatgcacgtgatgtgtgccttacttttttagaatataatttataacttttttgagcataaacaaaggtaaaatttgaacattagacatatttttttgggctagctaaatttgttgtttaaacctatatcacttaaccaaactcctcttttattatttattgatttatattttatttaaaatttttaaaattaaaatgatgagcaataaaagaatgttaagtagatttattaagtatttcttatatttttatcaacaaagtattttgtgttaattaaattatttcactttgttaattgattgtattttcctttttaatttattacttgattgtgtattgattgatcaaacataatttttttgttaatttttttatgctatatttgaatttatttttctttcatctgtttttggtagagtagttgatttactaaagggtaattaaataaatttattgggggacaccatagctcccccctcccttatataatagagatttgtatagatttattgtcttcctcaattattgattaactagtcttctatgcacgcgatgcgtgtgttgattgtttgggtctattcttaatataaatttcatcaaaatataattatagtagtgtgatttacaattattgctatacaaactactgtaatttataaagttgttagaaattgagataaaaatttagatgtgaaattttgtggtcaaattatatttgtaattttttaaactgagtaaccgtttttctcatcatgtcaagttactttgttaatgcttatttaatttattattggaatttttgacccatctttaaattagaaaaggatataatnnnnnnnnnnnnnnnnnnnnnnnnnnnnnnnnnnnnnnnnnnnnnnnnnnnnnnnnnnnnnnnnnnnnnnnnnnnnnnnnnnnnnnnnnnnnnnnnnnnnnnnnnnnnnnnnnnnnnnnnnnnnnnnnnnnnnnnnnnnnnnnnnnnnnnnnnnnnnnnnnnnnnnnnnnnnnnnnnnnnnnnnnnnnnnnnnnnnnnnnnnnnnnnnnnnnnnnnnnnnnnnnnnnnnnnnnnnnnnnnnnnnnnnnnnnnnnnnnnnnnnnnnnnnnnnnnnnnnnnnnnnnnnnnnnnnnnnnnnnnnnnnnnnnnnnnnnnnnnnnnnnnnnnnnnnnnnnnnnnnnnnnnnnnnnnnnnnnnnnnnnnnnnnnnnnnnnnnnnnnnnnnnnnnnnnnnnnnnnnnnnnnnnnnnnnnnnnnnnnnnnnnnnnnnnnnnnnnnnnnnnnnnnnnnnnnnnnnnnnnnnnnnnnnnnnnnnnnnnnnnnnnnnnnnnnnnnnnnnnnnnnnnnnnnnnnnnnnnnnnnnnnnnnnnnnnnnnnnnnnnnnnnnnnnnnnnnnnnnnnnnnnnnnnnnnnnnnnnnnnnnnnnnnnnnnnnnnnnnnnnnnnnnnnnnnnnnnnnnnnnnnnnnnnnnnnnnnnnnnnnnnnnnnnnnnnnnnnnnnnnnnnnnnnnnnnnnnnnnnnnnnnnnnnnnnnnnnnnnnnnnnnnnnnnnnnnnnnnnnnnnnnnnnnnnnnnnnnnnnnnnnnnnnnnnnnnnnnnnnnnnnnnnnnnnnnnnnnnnnnnnnnnnnnnnnnnnnnnnnnnnnnnnnnnnnnnnnnnnnnnnnnnnnnnnnnnnnnnnnnnnnnnnnnnnnnnnnnnnnnnnnnnnnnnnnnnnnnnnnnnnnnnnnnnnnnnnnnnnnnnnnnnnnnnnnnnnnnnnnnnnnnnnnnnnnnnnnnnnnnnnnnnnnnnnnnnnnnnnnnnnnnnnnnnnnnnnnnnnnnnnnnnnnnnnnnnnnnnnnnnnnnnnnnnnnnnnnnnnnnnnnnnnnnnnnnnnnnnnnnnnnnnnnnnnnnnnnnnnnnnnnnnnnnnnnnnnnnnnnnnnnnnnnnnnnnnnnnnnnnnnnnnnnnnnnnnnnnnnnnnnnnnnnnnnnnnnnnnnnnnnnnnnnnnnnnnnnnnnnnnnnnnnnnnnnnnnnnnnnnnnnnnnnnnnnnnnnnnnnnnnnnnnnnnnnnnnnnnnnnnnnnnnnnnnnnnnnnnnnnnnnnnnnnnnnnnnnnnnnnnnnnnnnnnnnnnnnnnnnnnnnnnnnnnnnnnnnnnnnnnnnnnnnnnnnnnnnnnnnnnnnnnnnnnnnnnnnnnnnnnnnnnnnnnnnnnnnnnnnnnnnnnnnnnnnnnnnnnnnnnnnnnnnnnnnnnnnnnnnnnnnnnnnnnnnnnnnnnnnnnnnnnnnnnnnnnnnnnnnnnnnnnnnnnnnnnnnnnnnnnnnnnnnnnnnnnnnnnnnnnnnnnnnnnnnnnnnnnnnnnnnnnnnnnnnnnnnnnnnnnnnnnnnnnnnnnnnnnnnnnnnnnnnnnnnnntatatatatatttagctaagaaaaaaaagacatttcattgggggataccataactcccccttagcttatataatagagatactatacttcttttctgatagtgtcaaatttaattataaatctttaacattggccaattaataattggacaagaaaaaaatgagacaataataaataaggcgatcttcacagacgtattaacatgatggtaattaaaaatgttaatcatagatctttgtgttatcttaataatataaatttactaattagaatgtatcacataaagtaagtattaatagcagcataggataattcttataatggagattttatatttttttatataattatatgatttattgttgaaaatattagttgattttaactggttgtttattcaatgacagaaccaactgatgcacgagtccatttctgaactccagaagaaggtaataactccattttttactctcaaaggtttattgtttttaacttatttcttctaaccttttatatatgagaaggtattgggttagacgcgtctgaccataatattaggtcggatgactttcagttggtttcaattttatttcagttggtttcaatttttgtccagttggtttcaatttttgttcagttggtttcaattttttttagctggtttcaatttttgttcagttggtttcaatattttttagttgatcttttttatttcagttggatgtcttttaagttcagttacttatcttattgtttcatttacgtgttttattgtaactgaaaacaaaacttaagtaaatgaaataaaataagttctaaataaaagcaacttagggcctgttctccccagcttattttcagttcagttcaattcagttcagttcaattcaattcatttcagttcagttcagatcagatcagttcagttcagatcagatcagttcttgacaatacttttactctcacatatcactattcatttcagttcagttcaattcaattcagttcagttcaattcagtttagttcagttcagttcagttcaattcagttgttttatgccgaagagaacaggcccttagnnnnnnnnnnnnnnnnnnnnnnnnnnnnnnnnnnnnnnnnnnnnnnnnnnnnnnnnnnnnnnnnnnnnnnnnnnnnnnnnnnnnnnnnnnnnnnnnnnnnnnnnnnnnnnnnnnnnnnnnnnnnnnnnnnnnnnnnnnnattcatttcagttcagttcaattcaattcagttcagttcaattcagtttagttcagttcagttcagttcaattcagttgttttatgccgaagagaacaggcccttagttttcagttacttatattatcgtttcagttagttttcttattctttcatttaacaactaactaaaataaaaaaaaaaaaactaactgaaagcaaaacttaattaaatgcaaaaaattaagttctaaatgaaaccacatacgatcgaaatttcaatcatttcaaacattatggtgttttcgattctttcaaagaaggcaagctgctcccgctattctaccctctttagatcacaataaagctcaggcctcacattcaaagtttcctcaaagatggacgttccaagtatcacatagacacatagtcctcttctccaaacgctctccttcctatcttgatgtcattagcaaacttcttgatccagacggcgccaacaaccgcaccatgatctccctctaaagtactgacggcccgtttggttgttggtcataaatgatggtaatgggaatgaagttgtgtgtaaatttgtgaaaaatatcattgtccattcccatggtaatgctaatttatcttaatgtgtccactttccttctagaattttcattctcatccaataccaccttgtaaggtggtaatgagtggtaatgaaaattgcttccccttggagacaaaaatacaagtttaggagtgagattgattgctcatggagaaaaaaagtctccccatggagatattaagggtgattccctaataaaattacacttaaaatttattcccattaccgcaatttattaacatctaccaaacgggccgtgaaagtcttgaaacacatagtcgagtgagtagctttgaggaaccatctgtaaaagaacctgagggagccaatgtgtgcgtaagtaccaacggcgtgttgtcagtggaaaaggtggtgccgtggtggcactcagtagtgatggagccgccgtggtgtttgagtgttgccaaatacaaaggcggaatttcgtaatctctaatttcttctgtgaaatttttgggatcagcctgtccgaccaaacacattggatcaaacggtctgacccaatagtttcaannnnnnnnnnnnnnnnnnnnnnnnnnnnnnnnnnnnnnnnnnnnnnnnnnnnnnnnnnnnnnnnnnnnnnnnnnnnnnnnnnnnnnnnnnnnnnnnnnnnnnnnnnnnnnnnnnnnnnnnnnnnnnnnnnnnnnnnnnnnnnnnnnnnnnnnnnnnnnnnnnnnnnnnnnnnnnnnnnnnnnnnnnnnnnnnnnnnnnnnnnnnnnnnnnnnnnnnnnnnnnnnnnnnnnnnnnnnnnnnnnnnnnnnnnnnnnnnnnnnnnnnnnnnnnnnnnnnnnnnnnnnnnnnnnnnnnnnnnnnnnnnnnnnnnnnnnnnnnnnnnnnnnnnnnnnnnnnnnnnnnnnnnnngatataaatagagatggaggacaagggtcttggttttgtcatgttgtcaaagagttgaacaatggttttttcgtattgttaaaaaattaaaaaaccagaggccttcaatctcttgatagatatagatagaaaaggaggacaaggccgttcttggttttgttatattgtcaaagagttgaacaatgattttttcgtgttgtcaaaaaattaaacaatgaaaaaagatggcgggtgcttgatctaatagatcggaccatggattgaaggtcttttaacttattttatatatatattgaacttatctgaagattatttaactctttgaaattgtattaacttccgaactttatgaacttttttaattcttcaaaacttatctacattttatttgaaaaaatattgaagacaaaaaaaccctcagttggtttaaagctgcggtaagatagagtgtaaatgttatttttttttattaaatcaagaaataaaaagaaatattaaataaaaagaattaaaaatggaaatgatgacagaaacttatggcttggaggagcaatacttttaagatagacctaaaccttaaataagttaaaatggaagtaatttttcagtagaatcttattccaatctatactccgtgtttactccatgtaatgcacatataataaaaaaattagaaattacatagtataaggtttgatcctgtgactgtaagtttatatactaacttcttaaccactagagcaagtgatatttagtgttatcattttaaagtataattttaacaaatgaaatttttttcttacccggaacatagctcggacctaataactagttgaacaattataatctgtaacttaaaatgatcctaattactgtactttcattacctataataatagaatcttactatcattggttcagaaaaaaaaaatcttattaaatgttaaccatttatttgtaattgaaacatacatgcacataaatgtaacttttagtttatcttaacttaaaaactgagaaaatgttagttggaaacttttgtatatatgtttggataaacgacgctcaaaagtaggggctaaaattttagtagataatataagattatactccatctgttctagatagacttctcatttttaattttggcagtattcataaataaaggaaatctttcaaaaaaatttccaatatataagaaaaaaaataatcatgtgcggttttgtttgattcgtctcattgtgtacattaggaaaattaaacttatataatttttactactatgtaattaaagatattaacgatacaaaatgtgtattgacaaacttatattggagtaataggaagtctattaagggaccgaagaaatattacgtaaataaatctaatacaaactaatataaattctactccagacaataaagattctgtcttatattgccaagatatagtagctatttattttatcttaacaaacataaatgtttctaatgcttaaacatggacatgtattattttgtaaaatattatgtattatccaaagttacatatttaaaggaagttctattgcttgctctcttttagcactgcccaaaaaggttaaagtaattttttttctctgtttaaaaaaaaaatgcattatatacagataatttttgctagtcaataaagctatccttatgacttatgagtgctacttgactagggatgtgttgtactcaattggaggtatacatacaccaagattatagagcttttattttgcctataaaaaatggaagccggataggataccaaaaaagctttgacttaaatttgtaatgcataaaaatgatgatacctaacttattagccatacttatctaagcgtacgtcaatttaaatattgtgttattgattaataatgatccttatatatccatattttgacaattaaacggtaaattagagagaaaagtttgagaaaataattatagcttacgtaatgctataatccaaagtgtctccgcacaagcgtgggacaaaatagtactttcggagaagttacaatcaacagctagggagtcttcattgttcttgaatagaaggatggaaacaaagttcaccttcttttattaaagtattaaggtttgttattagctcaatatccaatactttctctgctttttattacttcgtctgtttcaaattaaatgattttttttttattttacactatttttaaatttcacttttaccatcatttatgatttatatgtgaatgaaaacatagttacgtgtgatcttgttttttttttttttttttgtnnnnnnnnnnnnnnnnnnnnnnnnnnnnnnnnnnnnnnnnnnnnnnnnnnnnnnnnnnnnnnnnnnnnnnnnnnnnnnnnnnnnnnnnnnnnnnnnnnnnnnnnnnnnnnnnnnnnnnnnnnnnnnnnnnnnnnnnnnnnnnnnnnnnnnnnnnnnnnnnnnnnnnnnnnnnnnnnnnnnnnnnnnnnnnnnnnnnnnnnnnnnnnnnnnnnnnnnnnnnnnnnnnnnnnnnnnnnnnnnnnnnnnnnnnnnnnnnnnnnnnnnnnnnnnnnnnnnnnnnnnnnnnnnnnnnnnnnnnnnnnnnnnnnnnnnnnnnnnnnnnnnnnnnnnnnnnnnnnnnnnnnnnnnnnnnnnnnnnnnnnnnnnnnnnnnnnnnnnnnnnnnnnnnnnnnnnnnnnnnnnnnnnnnnnnnnnnnnnnnnnnnnnnnnnnnnnnnnnnnnnnnnnnnnnnnnnnnnnnnnnnnnnnnnnnnnnnnnnnnnnnnnnnnnnnnnnnnnnnnnnnnnnnnnnnnnnnnnnnnnnnnnnnnnnnnnnnnnnnnnnnnnnnnnnnnnnnnnnnnnnnnnnnnnnnnnnnnnnnnnnnnnnnnnnnnnnnnnnnnnnnnnnnnnnnnnnnnnnnnnnnnnnnnnnnnnnnnnnnnnnnnnnnnnnnnnnnnnnnnnnnnnnnnnnnnnnnnnnnnnnnnnnnnnnnnnnnnnnnnnnnnnnnnnnnnnnnnnnnnnnnnnnnnnnnnnnnnnnnnnnnnnnnnnnnnnnnnnnnnnnnnnnnnnnnnnnnnnnnnnnnnnnnnnnnnnnnnnnngtacatcaaggaaatttgcattaatgaaaaacgggagtacaacctaatggtaatacaaccaaactaaacagaaagaagaaacaacagacagtaagaaaacctctataacgcgtaaaaacaatttaacataaacactaactagaaaaagtccaggccgaataacatttgtcttgtgcgatggggagggaagatgaaggagagtgaaaatctgttgaaagacacaactctgacgatcttcatagagagattgtcgtacaactgctagtagatcctgtccactaggcacgaaatcccaaggtccttgatgagcctcctgggattctcctgattcgttgaacaaagaagtcactttcgagagtaacttcggaccctgctgcgagggtcttcgaaaatcagtcacattagactgaaacccgaaaaacaaggtggaggtcttgacgtgccccaaaacaagttgggggcgtcccacaagatgcgttttttaggtgtgatgacacatgatgtcatcacgagaaattggggcgagttagtttgatgaactacgccccactgacggatcctaagatccaaagtgacaatctcgaaaccagaagaccgacaaacaacagatctgaaacatacaaacatgaaaataatgaaagcataaactgccacccgacatatagagctccggcaaacaacaccatcaagaacttgcaccaaagacttccttggcatactaaagacactgattccaactaacactagcgggggacggggaagggacactcgactacacctaaacctaaccaggggacggggaaggggaacttagactaaaccttcgtaaaaagggggggatcggggaggggaaaaccttgaccaaggaagctggttttaaaaaccacttagccgagccaaaaaccgtgggtgggaagaagaaacagaccacaaacagggggaaccgggggatgggaactcaccgaacaggggagggggagaaatcgcacagactcggggaacgcctaaggactgggggacgaccaacgaacgaaaggttggggtggtgcgaaaacaagggagggggacgcaccgacgaacaaaaaaaccgacgaagaggccgaaaaagcgaaaggccgacggagataagattgaaaggcgacgaaaaaagaaaaaggaacaaaacgaaagaaaaacgaactcgtcggagacccgccggagacctacgcggcgccggatctccggcgagttctagggttagagggtttgttgtgtttgtttagggagaaggcagaggttttttttttttacgtgtgatcttgttagatttgtcttaacatgtattctttaatatacttttttttttataatttttgcaaatgcaaaattagagatatatgtcctctaaattttacattcacatacgtgataaataagagtgctacaactaatttgaaacggataaagtatttgaattgtttttcatttaaaaaagttcgctatcatttataatgttatatatttgccaatatgttatctctttctctctcttaccagagtttagatccagtagagttagtaaataattctaccacgtagagttgaacaaatcatagccattgattttcaaatcattggtttatatattctttcccaaaactcccccctattttccccaaaaatcctccccctccttatctctttccataaaatctgagtcgttgattttaaaatataaggtttggattcaactccactatgtagagttttcatcaaactccaccgaatccgagcccctcctaccatagtacttcttgatttccccatatttctttcctcatcttggtcctcaagcacattttaatattatgggtattaaacaatagagaaagtatttacttatagagaaagtattttcaatgattccctaaatttttttttgaaagaaagaaaagggatttcattaatatttcgccaaacggcacttacaagtcatttctgaaaaacataaaattctaaaagaaatacatatcaccctagaaatgtaaacatcgcagatttgacttaattttgccttaataaaaatcttcatctgaagcaatgcaatctgtgagttcgctctggttcggcatacgatctgcagatgcggaaattttgggatgaacgtactccaatagtcttccataattttacagaagttgtgaaaccctaattcttcatgttgaatctcgaacttcaaccaatgagaataatttctcatacctaaaaacaaaagaaccatactcacaactcccataggggagaaggagatttccaaaacagaaactaaaaaccccataaaagggtttgagaaaatctcataaagagatactaatttattgaacaaaacaagaaaatgaactaaaaactgaaaataaaagggaaaaaggggcttaccatggatgaaaacatccatggcagccccctaattgatgaagaaggggtaagggaggctagggttttagagagagaaaaggagaggggaggctaggttttaaaaaaaaatataatgattccctaaatttacttatatatatttaccaagatgacgtgatgttttacaaggcccatgatttttacgcgatcatgaaaaacacagccaatttgaatggagcaaatatctacgcgtcattttagatatttttgtatgggaaagttttttttgaccaatgtaattattaagaagcatcggccaccgggtagataagatgtcactatacatccttttccaaacttaagtatgcctgttgaacttttgttgcgtttgcagattcatttgaaattatatttcctcagatcctctacttgtaaaagaatgttccattattttcttagtttacatgatatttacaatagtatttgtctacattttgttcatattacttagtgatcagtgtatacgtcatatattagtttgaactttgaagacatttattttctatatacttcctttgtctgctaaattactttggaaagctttgttttttttattaatataagaccctttggagtttggaaatcactatctaatgaaatatataattcatcattagaacaaaaatacaaatatcgtactatcacctatcatgttccttttggatttcgcttcacaaaaatacattttaaaaaaaaataaaataacaaatggtagctaacaacttattacttttaaaagtttgtgtgcaccctaataagtactcaaagtagtatgtaacagagagagtataatgctaaaatacaaactaaataaacaagaaagtgtttctcaacaataatttgctgcaggaattaggaaacaaagtaaataaattgcatgtttatcatcaatacaatttactggtagttaattacaaacttcactcatgataattgaaagaggccactcaatttcagctaggagttgtttatttatttatttttctttcagttaaattttgactacccacaaaatcttcatctggacctaatctgcaatttgtggattttggatgaaatttctaacctatttaagtagtcttattgtttaaataacccatgcaattaaattaggttatatgggggtgattcatttaccaggcccaagattttatctcattctcaattattatcgcaacacccatgaacctaagccaacatgacttatttaccaggccagctagagaagaacaaggttgctgattttcttgtccgtgattgtagaagaaatgttagaaatctaaatgttgttagggatttacccctcccccctactgagtgtatgaacttattattgacggattgttgtaggcttccaagccaaaactctgattaagttttcttttatgccattttaaccaaaaaaaaaaaaaaagctaggaagctagctcagcgcgctctaattatttcacatgtgacatgttttacacttattcatacttctatatgcaggagagggcaatgcaggagcacaataacatcctgtctaagaaggtacttgcacttgaccagtttgtgtaatattgtaatttaatttcttagattttggttgcatgctttgatgacgaatgacgattgacgaatacatttttatgcagatcaaggagagaggaaaaaatctagagcaagtgcaacagatgcagtggcagaaccagcaccagcaccagcaccagcagcagccgccaccgccgccacaaaatcatcaagttcctcctgatgcatcaaatttcatgctcccacctccaattccttctttgaacacggggtagttacttcttcaacttaatttcctctattcaatattaagttaagaaacagatcacgtgattagttcgttaatattgctaattaataatcatattgttatatatcatgcattagtgggtaccaaggacaatttggtggagaagtaaggaggaatgatcttgacctgacgctagaaccgatatactcatgtcacatgggatgctttacaacatga

SEQ ID NO: 40 - DNA, 29237 bp, Artificial Sequence
  BvFUL genomic DNA showing  mutagenesis site at position 19552
  misc_feature (1029)..(1924): n is a, c, g, or t
  mutation (19552)..(19552): c to t
  misc_feature (20703)..(20722): n is a, c, g, or t
atggggagaggtagggttcagctcaaaagaattgaaaacaagatcaaccgtcaagtgaccttctccaaacgtcggattggattgttgaagaaagcgcacgagatctccattctctgcgatgccgatgtagctctcatcatcttctccactaaaggcaagctcttcgagtatgcttctgatacctggtatgtctaattttataacttcttcttttgtacatcaataattttatcatcgactcaactaaaagcttaagcagatggttagggttctattattattgaattacctcaaatttgtcatcgactcaactaaaagtagagtatatttcatgtagatcaggtgctttttttgaatatattgtcagttttagaactacaaaatgttgaacacaagtatttatacgcacgctgacatgtgaattttttaattgacaactttctaaattaatactctaaattactaatatgaagaacgtaatttattatttatcactttcagacaaaggcatgtttgttttttctattatttttcccatgaaaattctcaccaatatccgattctgtatgttaattttagtaatttctaattttgatgacttaataaattgtaaaaaagtataaaataaacaaatatccaaaacatctttgttttcaagagaaatatcttaaaaacttttgttttttaagagaaatatcttaaaacactttttatcatactactatgatgatgtataaatctattcaaaaaaaaaaaaaaatgatgatgtataaataatttaaagagttaagtttattagaaattatagatatttatagagctgagtaataaaataatactctacagattatatgtagctgatgtagtgtgtctgctcctgtaagatttcctttttatctccaaaaaaattgcattgatattcgagccttgccgacccccttttcctcttcaaccatttgataagatcctatgcactgagtaatctagtattatatgttagatgttatatattaataagctaaaattgtnnnnnnnnnnnnnnnnnnnnnnnnnnnnnnnnnnnnnnnnnnnnnnnnnnnnnnnnnnnnnnnnnnnnnnnnnnnnnnnnnnnnnnnnnnnnnnnnnnnnnnnnnnnnnnnnnnnnnnnnnnnnnnnnnnnnnnnnnnnnnnnnnnnnnnnnnnnnnnnnnnnnnnnnnnnnnnnnnnnnnnnnnnnnnnnnnnnnnnnnnnnnnnnnnnnnnnnnnnnnnnnnnnnnnnnnnnnnnnnnnnnnnnnnnnnnnnnnnnnnnnnnnnnnnnnnnnnnnnnnnnnnnnnnnnnnnnnnnnnnnnnnnnnnnnnnnnnnnnnnnnnnnnnnnnnnnnnnnnnnnnnnnnnnnnnnnnnnnnnnnnnnnnnnnnnnnnnnnnnnnnnnnnnnnnnnnnnnnnnnnnnnnnnnnnnnnnnnnnnnnnnnnnnnnnnnnnnnnnnnnnnnnnnnnnnnnnnnnnnnnnnnnnnnnnnnnnnnnnnnnnnnnnnnnnnnnnnnnnnnnnnnnnnnnnnnnnnnnnnnnnnnnnnnnnnnnnnnnnnnnnnnnnnnnnnnnnnnnnnnnnnnnnnnnnnnnnnnnnnnnnnnnnnnnnnnnnnnnnnnnnnnnnnnnnnnnnnnnnnnnnnnnnnnnnnnnnnnnnnnnnnnnnnnnnnnnnnnnnnnnnnnnnnnnnnnnnnnnnnnnnnnnnnnnnnnnnnnnnnnnnnnnnnnnnnnnnnnnnnnnnnnnnnnnnnnnnnnnnnnnnnnnnnnnnnnnnnnnnnnnnnnnnnnnnnnnnnnnnnnnnnnnnnnnnnnnnnnnnnnnnnnnnnnnnnnnnnnnnnnnnnnnnnnnnnnnnnnnnnnnnnnnnnnnnnnnnnnnnnnnnnnnnnnnnnnnnnnnnnnnnnnnnnnnnnnnnnngatgatattatgtatcattattatcagtcatttattattgatagataatgttattatttccatagatcatatataatcttaccatatttactccctatgattatatatttctatctattaacatagtaatagtgatatactaacaacgagtatctttcaagtaaataaatcatatatatagggttagaaggtaaaaaagacaatattttatgagactttatttacacccttcgtctcataaactcctttctattttttgtgttcactcgttttctaaagttttttctacttcttttactttttattggataaatactttttccgtctgtatgtgatctacttatattagtatttatagatagattatactcttaaagtattacattcacaaaatcatgtgaattattaattaaagtaaaattatgagtatggtattataacttaaacgaagtagttgtattgtttaaaccaataagtataataacttataaaacttaaaagttgattctacacttatcatgcacttgtgttttgatgggttaaaaattagctagtacataagtaacataacataaacttatctctgtatagtatgttgaattattactttatatttgaaaagaacaaagacacaataagtccaaaagatccgatcttttgattatcaactatgtaagtgtctttcctaaatgatcaatcaccttaattagtatactaaacaggacaattatgacatataacacttttctatttgtacaagttaattaacccattgacattcattcagttagcctacatttttcaataggtagtcatcatcattctttttttaaccaatttttttacaataaccattacctaccaacaacattttcaaataatgaactgaatgatggattccgtcaaggaaattgttcgtggacagtttgtttacctcccaaatttcctttaatctcatgctttctccatcatccaaacaatctaataccaatcgttttctctaattgcataaaccctaattgttgaatcctttaatcttgccttttcacattgcccaattcctttagtatgatattttttattcgataatccctgataagtaaattcactaatctaatttcagatggattgttgtagagattggggaattgaagattttttgccttctttgttcttgtttacaatgaaggatgaagtttcatggaatattgaagagaaatttgagaaaagaaagaaagtgtgggctttactgacgacaaaaactgtcattttggtggtttttttcactaaggcatgtttggcactagcgtttaaggtagcggttagcgatttgacaagatcaaaacgctacttaagaaaatgatgagtgtttggtaagatagtggttgttgtagcaggtagcaattagagtagattatgagtagcggttgtggaatgttactacaagtaacgtttgagatttagaggtagcagtccagcaaagaaacattgtataatagcataaggtagaattaattaaccaatgtttttttatttctttttccttttattgtttattaataattttattttatgccaattcaatgtttattttacaatagcaaaaatgtaatttaaatatttattttaaacataataaattttataagtattttagtaaaattggtaatataaatttttcgagggttgaatattttcttagatgtatacatttctttgaatagttaaaaaatcatatctcctttttgtgtaacttctttgaaaaataaatcttgaatttaactattgaacgaacatatgaaattattgtagttcatttcatattataataaatgttaggtattgtcttttacaatttcaactacttttggcaaacaattctgattaaacagctattttaatcgctgatcgttgacagcaaccgctaacagctactagaaccgctacttttgccaaacatgcctaaaccaagtaatatcggggattctttattatataaaaagttaataatgtgattatttgaaaaaaaggttgactttatatgttgtttaaagaaaaaaaaacatttattaatagaaaatatactatataggtctctatatacccagggcgaaatgaatgtgtatcttttcaaatgagtatgcgtacatgttctgtaaatgcatatttcatatgagcataatgtttttactattattatgcacatttgtgttttaatttttcaaatgagtatgtaaggaaaacatgtattcttggcatgtcagtgttagtgatttttgttgttatataaatgttttcgtgatttgtgaatgtggtacaaacattcatgtgccatggcgtttagcaaaacttttctagctcacatgatgcttcaagctaattgcaatgaactaatataagggagaggacattttacgaattagttttacattgatagtagtttgaagaagatagtttaggagatagtttgttggaatagaagctatgtgttagaattagttatagtcatcaatttttgaataagactcattattatttcaatccttctaccttttaattactagtccaactctcactctttggtattaaattacaccattcctacggactatctaacaactctaaccacggcccatactttttcttcttaacataaaataatattacgcttactaactactaactcctatgacatctaccttttcaataaaataacaattgataactatataacaacttataatctaaaagtaagtgtcttgataagtgtagagtattgtgggacgaagggagtaattcatagcaaatactatcatagcaatacaatactaggagactaagatgtgagttttgaacttcaaaaaaaaatatacgcgacatagttcaccggaagaactgcagcacaacaaatgcaaatggggattaaatgaggagttcacctacatcacacacaagagcgattgaggattttcagatctggaagaagagcgaaaaatcaggcgagagcttcaactttcggagtttaatggaagagctaatgatgattgaattattcagttggatttatcttttgtaagatgaggggatgaagttgaagattgccataataacccttgagggcgacacaatggtggtgggaatggaaatatggaccacgaccgatttatgagtggaaagaattgaagtctctgatacaatgacgttttggtatatcatcggtgctttcatggctgtcagatctaccgaaaggaaaagtagtggtgaaaacaaatgtcgttcaaaccaaccacctttgactttcaatattgaagtgacaaggaaaactggcaccttagctagtgacttggtggagtctttgcgtaaaccggtggaaaagaagcttatctttgagttttagtgtggtcttggtgcttgtttaagtggcttgactatttaggaggaaaaaaatcaattgtgaacaattggtgagtaacctaaaaatcaattgtgaacaattggtgagtaacctaaaaatcaattgtgaacaattggtgagtaacctttaaaccagactcaagagtgggaaagaggcggttagacaagtagatttagaggaagaggaggtagaaaatagattagaattttttttgggagttttcaaatgtagtggtatcggctcataacaaggtggtcaaatggatggagagcttggtcgtttgagtagtctcatggtggtgattataactacgttggcgataaacaagttcgctttaccaagaagttgattggtggaagagagattttcataaagaggggctcgtatagcaacagctttgtgtggtctcagtttcattgtcggcaaagccgtgggtggtaaatatggtgattttggagattgttatgatggagggagttatggtggtttcatgagacatggatgctatggtggtgctgtgatcggtggagaagaggagctcgtgaaaggtcactctgatggagcgggtgtaatggtggtctaggttttttcggcatcggaggttgcgtatctcgtgaaggttcacatttgtacaccggtgaatactatggtggtgaactaggatgacagtcaaggtgaccatagtagaaaaaaaaaacataaaccatgtagcttagatgatttgaaaaaaaatcatgtttttggagaagaatcttaaatattatgacagaggcaaacttgtcattgaccaaatagatgacatagcaattgcacgtgtctcgttaaaatttgaaaccataaaaaattcaaattgcacttcatatgcctttcttttggttgaaaacttcatataccctaatgcgtcaatatggttctttttccaaaaaaaaaagtaaattatttcggcgttagtaaaagcaggtccacctccataatccattttattaagccaactcctctaccctacttttgcaacctatcatttcttattttctaaaatcatatcaaaaaaacaagtgtgaacccaaaactaactatattatacctaagtctaatttcttcatccaatgtgttcaaccccatttttcaacccttccactcataaacccatcttctttcactcctaaaactttcagctcacgctcgtatcacctctttactcacatatcagcccaaacgatttcttattgaatccactaaattatgtatatcgattttttcaccaagtactccgagttttcaaaaaatttacctggtacccccaagttttcaaactacacgggatacccctaagtttcaaactaatacactcagatacccttaatgactaacgacattaatcgccgttagtcattaaccttaattttctagatttcaacctaattaaccactaaccctaaccccaaccctaaccctaataataaccctaaacctaaccctaaccacccctccccaaccctcccaccacccctgccccccatcctccactcctgcgcagccagcaggccccccacccatttgattttaaggaagaaacacgtatcagggaagggggagaacttagctctgacagcggcaacggaccaccgacgagtctggactgtaggacggcagcgtcaaggcgcgagccggttgggctactgcagttcaaagcaaacaggggaggggaatcgagccgagaagagagctaaggaaagaggggtgatgggcgttgcggagatggtgcgcatagtggtggtggtgtgggggagctgtggtgggggagaaatcgaatgggtgggggagagagggtggggggctgcggtggggttggggctggagggggtagggtgggtgggtggaggggtggtggttgggtggtagtgggacaactctcaaacatgattctttctcaaacatgattctttctcatatccttttttggatttccttaaaaaaatccatatccaaataacgttgaccggtgagggacaactctttaacactattctttctcaaatcttatgaaatcttcacatttaactcgatctccctttcaatgaacctaaagatatatattaatagagttgcaaattcctaaactctagaaaattcaaatacaacataagagtcctagattcttccacaagatgtattatatctttcaaagtttcccagataaaattagtaattaggaaactccttaacaaggatacttaaagttttatctaaatcttgcataaattgaaatccaaccataattatgaataaataatcataaagaatcctaacataaataactagaaaataagataataaagaagcaacaaaagaatctcataaccaccatttgaatcccgcatgagaacccaaatagttgttgttccttataaaaacccaccacctttcttcgggtattatgacggtattggactatagtatgagacgagatctcttaatcaccaatcaactattgtaaacttgtgagcctgaataatttatttgagatacaattctaaggttgtttatgaacgtgtttggtaaaattgttattgataactcgttcgtggaaaataaatgcaaaagtcaacatgccaaaaaaagtgctaaaatcaactttcggctttgcttgaaatgttaagttttaagctatccaagagccattagtcaaaatctattgaaagcgtactcaaaaaccatttatcaaacacccctacaaatccctttagaaaacaataggagttgtacaatataagtattgagttataaagttgatcaagtgatttaggaggttgttccaaatcaatctacaagagtttgtatacttataccccttcgtttttttaattgttacacttaggccttgtttgacaaatagagtttagcggttagagtttagattttgctgttagagttttaactttttgttaaatagatttgactgctgatttgacaacttcttcttataaatgtgtttggtaattattaacagattgctaaaagcttattaccctttatttatgtgaaatgacatgtatagacattttaatccacatgggtattattattattattattcgaggcatacaagtcattgaatatatttttacctaatcctctaaagaaaaagctcctattaggagctttttcatttcgagagtttttattccagaactctcttcaaaactcttttttaccaaagaataggagctttttcatttcaagagtttttactccagaactctctttaaaactcttttttaccaaacaccccttttagagtttttgactagtcaaaactctaaaagtggtccaaatttctcttttaactccaaaactctaattgccaaacacccccttacacttttcacgcataccaatgcaacactttgacgattaacatctccagttttttatttgtaaaaattataaagagtgcatattaataagtagggctgttcaaagtgcggtctggaccgcaccaaaccgcaacccaaaccgttgtttcgcggtttggtttggtttgcggttttaaaattgcggtttgggttatgatttcaagcaaaccgcggtttgcggtttgggttgggtttttatttttgtaaaccaaaaccgcaccgcaaaccgcaatgttacattttttttaaaaaaataaattaaatacatttatgaaggtgacatacaattataaaattgaaaaaagaagtttgaggtaaaaaactttaacacttatgataaatcattatatatgtttaattatgaattcagcttcatatctatttggactcttattaacaattttcttttaatcttaggaaacaaaagtaatgtcgcggaggaaataatggttaaaccgcaacccaaaccgcaccaaaccgttttgcgcggtttgggttgggttggtttgggaaaaagtgcggtgcggtttgggttggaaaattttcaaaccgtatatttgcggtttgggttgggttacatcccaaaccgcacaaacccaaaccgcgaacacccctattaataagatacatattaattcgaatttgacaagatccacatgactatgtttttattcgcgtataaaccacaaaagaaggttcaagtaaaatttgtgtatggtgtaacatgtcaatcaaagaacggaggtaatatttgtcaagacactttagtcacttctaaattcctataaacaaagaaatatggaagaaaactggtgatgaaaattgaaaaggtgggtataataagagagacacaattctaaaataagaaaatattaataataaaataataagttacgataggcctcatgtttgaaaacggaaaaaataaggagatagttcgtgtaaaaaggagggagtaaagggtaatgcatactttgtattgcaagcttagttttaaaaggcataagacgcaaagcgcatcgaggcacaagacgaaggcgcatgcatctcgtagttgaggcgtgtaatgattttacttcacaaccacctgagcaacccaatacagaacgaccacaagaaaaatagaaagaaaggaaatgattttgattgatcagcagaaaatacagagcattcgagaggctcagtctctcccaaggactacaagatactactaaatttcacacccccttcagtccccttacacccttatttatactacttctgctctcctattttaacggctactgacattctctgagctggcctgctattcctctttttgtgctgacatttctgaatattctgtggtagtggctccattctcacatttggacaggtttacccctccatttctttcgtgcatacgtcagccacggtttggggattgaattcattacattaccctgcccccaaagactcaccttgtcctcaaggtggaaggaagggaaacgttcttgcaccaaatctgcatcttcccacgtggcttcaaaaggtgctaagtccttccatttcagtagcacttcagtctgcgtatgcctccctctctgtgtctgacgtacgtccaataattcttcaggttccacaactagttccaagtctgctgctagttgagttggtacagtggttgctgcctgggcatctccaattgctcgtttgagctgggatacgtgaaatataggatgtattttactggtgcctggtaactggagtttataggcgaccttgcccaccttttgcagaacagggaatgggccatagaagcgggctgccagcttctcaaatggtcgcttggccaaggattgttgacggtatggctggagctttaagtaaaccagatcccccacttcaaaggactcatcgcgccttcttgtgtcagcataggctttcatcttttgctgggagcgtagtagatgaaagcgtaaatcatcgaggatggcatcccgttcttgcaacacttcctctaagttatctactggcgtttgccctctgcctactcgccacaagtgtgtgggtcacgcccgtacaacaccctgaatggagtcagcttagtagacatgtggggagaggtgttgtgtgagtattcagcccaagggagccactttgcccaagtcttcgggtgccccgccacgaaacatctcagatatgtctcaagtcctttgttcacaatctcagtttgtccatcggtttgcgggtgataggcggtgcttctccttagtgttgtcccttggagtcgaaacaactctttccaaaaagtactcagaaaaattcgatccctatccgaaacgattgatgccggaaacccatgaagttttacaacctccctgatgaaagcttcagccacttgtgagagcactaaaaggatgacgaagcccaatgaaatgcgcatatttcgataaacggtccaccactactaagatcgtgtccacccccttggacaagggcaatccttctatgaaatcaagagtgatatcctcccaaacctgagctggaatggctaagggctgcagtaggcctgctggcttttgttgagagctcttatgctgttgacaaatgctacatcgctgcacgtacaatgccacgtgcttcctcatacctatccaataccactcagccgccaacctaaggtacgtttttacttcacctgcatgtcctccttctggggaatcatggtaagctatcatcaacttaggaatgatgacggaagtgttgggaattaccattcgccccttataccgcagcttgccatcctccaccgtgaaccccacaagtggtttatctccctgcgccacttcttccctgagccttttaaggaaccaatcctcctctacctctttttggagctctgcccagtccactccttgggttgtgattatggtccctagctccatttcacctacagtttttctagaaagcgcatccgcaaccttgttggttgcccccggtttgtagtgtatttcaaagtcaaacccaattaatttgcttacccatttctgaaaatcagcccccacttcccgttgttgtgtgatgaaacgcaaactttgttgatccgtatggatcacaaatcttctccccaaaaggtaatgtttccatttctggaccgcaaggcatatggcaattaattccttctcataaacggacttgtgttgtgctctcggtccaaggagcttgctgtagaatgcaatgggcctgccctcttgcattaggactgcccccaccccatacccagacgcatccgtctcaactacgaaaggcttatggaaatcgggcatagcaagaaccggtggctgggtcatagcttcctttaagtgagagaaagctgaagtagctttttcggaccagccaaaggagtccttacgcaattgctcggtaaggggctgggcaatttgcgcgtattgcctgataaacttgcgataatacccggtcagccctaaaaatcctcgaagctccctcaaattcttgggaacttcccactccaccatggcccttatcttctccatgtctactgccaccccatgctgcgaaatttacatgccccaagtaggccactgtcttcctccccaagtcacatttcttctggttagcgaacagtttgtgcaatgctaacagctgcaacaccaatcccatgtgtcgtgcgtggtcctctttggtcttactgtagaccagaatgtcgtcgaagaagaccagcacaaacttcctcagatatggacggaaaacgttattcatgagtgactgaaaagttgctggggcattggtgagcccaaagggcattacgagaaattcgtaatgtccttcatgggtgcgaaaagcagtcttatgggtatcctccgggcgaactaaaatttgatggtatccggccttaaggtcgagtttagagaagatggtagcgccatgtaactcgtctagtagctcatcaatgaccggtatcggatacttatccggaaccgtctccttgttcaaagcccgataatcgacacaaaacctccaagaaccatcttttttcttcaccaataatacggggcttgaaaatggactagttgagggcttgatgatgcctgcctccagcatctctcggatgagtctctcgatttcgtctttttgaaattgagggtaacggtatggcctaacccccaccggattactgccttccttcaacgtgattgcatgctcatgccccctctttggtggcaggcccaccggagtatcaaaaacttccgcaaactgactaattaccttctgtaaaaattcgggtacttcttgtgcctccttcaactccgcttctccccttttcccatcatcctcaatctggttgagctccaagagaaaaccccctttttcttttcggattgcctttatcatggctctaagtgagattttagatcttgctaaggaagggtcccctctcaatgtcaccactctgccctccacttcaaactgcataacctgagttttccagttggtaatcactgaccccaatttctcgagccactgcactcctaatattaaatctgagttacccaggccgagaggtaaaaaatcctctgttacttcgatttcccccagctttaaagtcaccccttgacacaccccagtaccatggacagcttcaccattccctaaagacactccaaatccccctgcatctgagatgaccaactcaagttcctcaacagttaacaaggaaataaaattgtgagtggcacccgggtcaatcatgaccaccacctctcttcctttaatttttctagtgattttcatcgttttaggactcatcaaaccaatcacagagttgagagatacctcagtaggaagttccggtggtggttcggacggtggtgcacgagctgcgtcgctcacctcttcggtttcttcctcctcgtcatgcatcagaatcacgctgatctcttttctccggcagatgtggccggcggtccacttatcgtcacatttatagcacaacccttttgctctcttctcttgatattctttctcggaaagtcgcttgaactctacagatttttttccttgccccccagcaattggatacgtgttcaaggtgttggaatttccccctgggttttgggcccacattttgctggcaggtgggttgaggctggtcgttggattgaaggaagcccctacactccttgtcattccccctctgttataaatcgagtaaggcccattcttagttggcccacttcttttataacccacaatcctattcctttcctcaattcggcctgctagttccattgcttgctctaggtccataggattgagtaacctgacctccactttgatatcctcttccagcccattaatgaactgacccatgagtatttcttctggtactctactcaacggtgccgccttctcaataaaagtgcgtcgatactcatccaccgtggtggtttgctttgtggccaaccaccgttcccacaatgaaccatagtgggttggtcgaaactgacggaggaggtactccttcagatctgcccaccaccttatcggccgccttttattctcccactggtaccacctgagggcatccccctctatagacacaaccgccgcctccagggcttcactgctactcaggccataaaacgaaaaatatcgctcggctctaaggatccacccatccggatcggacccatggaaaatgggcatctctaactttcgatatttccagttccccccggaagtcgaacctcctggccctccacctgagccgccatccccatacgatcggcccccgagctggaaacctccatattcgtccccttctcggccccccagatttatcaggtcaggagccctccgttccggcggtcgggggtgtccagtgacggtttcgggtgtctcccgcgagggttgtggcaaggttgctcggatttcaacctgaaatttcctctgttcagcacgcaacccttgaatcgtcccatcctgtgtctcccttgaccggttaatccggtcctccagcctaacggccaagacctccatctcctcgcgactcttcctcgccgcctcattctggccttccaagatttgagcggtcaacgattcccccatggcattaatggcagattccaccgccctggacaccatggtggccactgacccttcgagggctgccattctttcttctaatgaatccaccctctgcacttcgtttcttggtgccatggatcgatgctctgataccaagtgtaatgattttacttacttcacaaccacctgagcaacccaatacagaacgaccacaagaaaaatagaaagaaaggaaatgattttgattgatcagcagaaaatacagagcattcgagaggctcagtctctcccaaggactacaagatactactaaatttcacacccccttcagtccccttacacccttatttatactacttctgctctcctattttaacggctactgacattctctgagctggcctgctattcctctttttgtgctgacatttctgaatattctgtggtagtggctccattctcacatttggacaggtttacccctccatttctttcgtgcatacgtcagccacggtttggggattgaattcattacaaggcgcacctttggtaccaagagacttagacatcaaataaagaagcattgtaatacttagaataaacattgtttttatattctaaaacacatattttctctaagacacctagtaatctcatagtggatgtcatctagtttaggtggtaaggttttattgagttggtactcaagacctcagacttagaggtggcaaacggatcatacgggtcgggtgaaaatgagtcgggtcataatcgggtcacctttgtgtccaggttacggtcaggtcgagttcgttcgggtacgagttcatattgagtccatgaggtttcatgtcatatcgggtcgggttagattggatttacaatttcgcaaataaataaaacgcatataatactaaagagagtaaattaaataattaacggacactagctaaatcatatattagtattttatgatgtattttccttaaatttatttaaaaaataactaatatgacaatttttcgggccgggttcgggttgtggtcatcattatcgggtcaatttagtatcgggtaggctcgggttcatgtcatattcgggtctattttaattcgagtcgggttatttcggatttaagctctatttcgggtcagtattttcgatgaagaacgggtttcggatcgggtcaccggatacggatctattttgccgagtcagactgcttttcaaacctaataatctcagtttttccacctattcagatttgcctatgatctctatttagataaatgagtacaatattgtgtctatccatgaaaatgaatatctcacaatgtaaaaggatatctctaaatttcactaatcactctatctgttttgaataataatattctattttattgcatgtagtaaagatcgagtatttagtgagatttggagaaaagaggaggctagagagaaactaggatttagagaggagaagggggctctgtaacacatacaagatagatactcttttacactaacttttcaagatactcaacatataaaatcagcatcatcttccaaacaacaactttaagccacccatgaatcttaattagataataaaacataatcgtgaatcatctatcctttgtttggggggatcctaaagcaattgaggaaaagctttgatgcaaatatcaattgtgtaaaaaagcaagtattcgttcgtgatgttgctatactaggttattttttggatccaaaagtcattcctactagaatcatttaggaaaattgtcagtatgaattttaaattcaggttataaccaaagataattgaaaattgtcaaacttttcaaataattccgaaataaacatgtttgtaacatggataaacttttcattgcttttcaaataattccaaaataaacatgttataacatagataaccttttcagataattccaaaataaacatgttgtatcatggataaacttttcattgtttctagtcacttaaaattctaaaaaaatctttcctccctactgttactctctctagcaccaaatctatcacatgagaaggcagaggttttcaaaataaaccgttacttaatttggtacttatttcttgatcggtgttcatatcatatgagttcctactctatatctctctactcttctaaatccttgtgtcacttcctgtgtttcataaataaaaaggaggaagtattagttttgaaacgaaaggagtatggtgcatacattgatagaaaaaagaagttatttgtccttatttcactcatataacaacaccaaattctgtattgttatcacaaaataaaacttggattatctttgtttcatagcccaaatttagaattagtttgtcagatttccaatcatctaattacaatattagagctagacctaggacaaaaggtgggtttggctacttggtaatagctatgtctagtgctaggatatgtcattgtcgtagaaccatgttatggacatcttaagaaacaaggttaacctaattggttggagatcctactttcacttttataataaagtttcgattcttgcctatttgtaaagtagaattcctaaatttcccttcactgatatttatcttaacataaaaaaatgttataaacattgggattgtatataagtcaaaataaattgacaatcttggtaacaactaagttaacattaattttataagtaaatgattaatcccaatataatctcttatttagtaaatgagacaaacttgtacaccttcgtgttagactcgttaatgttcgctaacaattcattcagtagtcaacagcattttaaatttgaaataagtgttcttgtggtttttgagagatcaagcaagaaaacatgtctctcccctttgaccaactaattgggattaagaatactagttttaagattttaagaatgagttatagtctttcttagaccgctacaatccccttgttgatatgaaccagatatattttgtgttcaaatagtagatcaatgcattgttgataatcctttgttaatgtacttgttgatcttattttgtacttttggtagatgcgctatactttctttcgattgctcattttgaactcttaactacatatgttagtttaagtagatgatttagaattgctatttcaatcttcaataagcaatttaagttgtcaaaccttgtttcacatcattagggtgaaagttatttggataaagacctatatctaattcaatccaaagcaaattagtaatgcggattggactcaaactatgtttagattggattcgaattgagtttcttttctttttcttaaaaaaattggattttccgatcgaattgagggtgattagatccaaaataaccgaatagtagataggatttgtgttgtatattagaattgggcttaaggatttccattttaacaaaaaaaccaaatggtccgactatcaaaaactataatttgatagtcatgcctatcgaaaactttattttcattctcgcacctaattatgggcttgtataaattagttctactatcgaaaactaattttgatgctcgtgcctaatttaaattttcgaaaaaatgaagttaagaaaattggatatttcggattggatccaatatatcttgtgaattattaatttggattagtttggactcaaattcttattggattggattcaaattaaaagattaaaattcaaattttgttcgaatcaaattggagtaggcttaagtttaaatcatacaccgaactttcaccactacccatcatgcttaagcttctaatgtaagagagtgtttgggagttgagctcgaacaactaaatttctaaaagaaccaagttcaaacaagaaatctaaaagctcgattaaacttgagtcaagctcaaacacctatattccttattggagcttgactgaagattgaacacttattccttattaagctttacgctaaaacattgctcgactcaactcttctacatccctatagttcaaaagaaatagttgtgggctgtggtgctcttgtagaccaacgcactagtttaacaaagctaagtgcctgactgcaattccatacacattacgatcaccatgacctagtttcagctcacactttggaagtctaatttgaacttgttctctacctccaattcattgtggggtaggaggcgatagttaagggatcaaaatcttatgatataacttgcataggctatgccactatataatgcgtcttgtgtcccatattagtttaatcaaattgaaatgttttaccatttatatcttcaattatgtatggatactaatatttgatttgacgtttgatatgatattaaatgtggactgttattcttgatgtgcttgagaagcttttttggggccagttagaaactatattccttttatggtcctaactaggttgttgttggtgtgttcccaaataacagcatggaaaggatactcgagcgctatgaaagacactcatatgcagagagacaactgactgctccagatcctggatcccatgtaatccagctaggcaactatcttttctaagcatttaaatcgttgagatttcaattttaaatgtgttttaactgataattcatgcattatatgcttaggtaagtttgactctggaacacgcaaaacttaaggctaggctggacattctttagaaaaatcaaaggtaataagatccagaccaaatataatttgtataataaccaccttatgaggaaaatttaagatccttgataatttcaggcattacatgggagaagaacttgataccttgagtctcaaggagcttcagaatttagagcatcaaattgacagtgctcttaaacacatcaggtcaaagaaggtagtttcacagttgcattagatcatcttatggatcaattggatcacttgtttgtattttagcgttgctcaacacggtcgtctaatatagtgtgcaaaacgacctacagggcaacaccttttatagggctcgaaaatacgaaaaattaaatgtttgttttagtcatattgttcaaacccaagctttatcttgtcaaaaatattttataatgattattttttagaatacattatttacatttttgcaatttatgcataatacttctaaggtccaactttataattgaaatagaagtccttaaattttaaagacgaccttgaggaaacctaatttcttctcatatataattaaatcaattattctacaagttagtagaacaaatactacaataacaacaatattgaagccctaatctcagtaggattggattgattgtatgaagtcttattagtggccgttaaatgtttcttgtaggtcaagatgacatggctcatatagtaaggttacttgactaaaagacgaggatttgtttcgacttagattttaacaagtttccctcatttgttaacacctaagcgtactaaatcaaattctaggttttactcactcaaatttccgatttaggaagggcttgaggatagttgtattatcgtaactgactaatcaaaggagcctctcttagatcaggtttcacttgccaattctaacaacttgtttggtaaaaggaatttggaatgaaaagaaaggaattgaaaagaaacattctacttttcaatgtttcattcaaaaataacattttaagtgataggaaatggaaagaagtgaaacgaaagcctctttacaaaattatcatttttctacccccccccccccccaaaaaaaaaaaaaaaaataagtagtaagtagtagaagaagaaataaataactaacaagagtagtaagtttttacgttttctttctnnnnnnnnnnnnnnnnnnnnattcaaatcagaactgaatagtcataaccggaagattagtttctctctagcgtgactagggtttgagtaaaaagagaaaacttaaatcaaacatgggatattaaggttttttttcctttcttcagttcttttctcttcccaatcctttcctaaaaatgaaccaaacaggctgcaaggttttcacttgcttaacacaagatttatttttaaaaataattacactccaaacttttaagcttaaaaccaattttaattcaaatcagaactgaatagtcataactggaagattagtttctctctagcgtgactagggtttgagtgaaaaagtctagggtttcatgtcattcttcttgcttcgagtcccttcttgggattgttgttagccattatggctaccgaaatcgttattaaatgtctaaatcttagaattactgctgaagaaaacaacttggtgtttctcgaagatgttgatgataactcgcagcaccatacgctcgcactggcgattgttggaaaggttctttcgtcaagaccatacaatttcgaggcacttaaatgaaccttaaactagatatgggtgatatccaaaggagccctacttcaccctattgaaaacggactttttgtggtacaatttgcgacaattaaggaccgatctaaggttctagtcagcagaccatggaccttcgatataaaccttgttctcttagatgctattgaagggggtactcaatcttgacccattgcccgttttggactcgcttgtataaccttcctatggactgccgatatgagaagttcatcaaaaactattgttggtgtattgggggaggtattggaagttgattttgacaggattgtttgggataaatctgcaagagtaaaggtgaagattgacattacaaaatcgttttgtcgtgtgcagatgatcaagactaacaggggtgaggctgtgatgatcaatgttaagtatgaaagacttcctacaatttgttatgtgtggaattctggccatattgaaagagattgtgtgaagacccaggaagaagagaaacaagtggagagacaatagggggtcttggaggcctctccgcgtaggggacgattaaagatggtgaaagagtcgaaagccttccttcagtgtgctcgtacactccactttaataacaaggaagaagtaaggggtgaggaaccacgggattatgtggagccgaggggttattgtcggctatcttagggggtaaaactttggtggtccaggagatagtggacggctctaaggatgccatcgaggaagttcgtgctgaaggtgcaccactctagcccccttgtaccctttgggtaatgccatgctaccttttacttttgctgttgggagtgctaatcctactccctcccaccgaaaagttaaaattaaaaacaaggcaagggttcagggtgttttgaaccaagttaatgttgtgggtgttggggggttggctaataatgggggttgtgagaaaaggatattccccaacccgatggtgttagaaaaagaaaaggggttcaatgaagagggtttaagatagcaaaacgagaggattgtatgtaacctatcagtagggaggtaactattgaggtggaggtgggcgagacccaaccccgcccgacattatgaatatcctatgttgcaactgttggggattgggcaacccccgggaagttcggatgcttcgtaggtggagcaatagtgctacactgagttcggtttttatttctaaaactatgattagtggtcgtgatgtggaaagggtgcaaagcgggtagggttttgattgggcaattggggtggatagcgttggaacttcaagagtttggtgcatttattggaaagctggggaagtggactttactctagtctctctatcaagtcatcatatttgtgggaatgtgaagcttgttgatgggaaggtatgatgcttagtgagtatttatggttgggcggatacaattcaaaagtataaaacatgggagcttatgcaatcctttcactcatatcatgggccgatattgtttggttgggacttcaatgagattttgacaatcggagaaattgaaggagggtccgaaactcaatgaagtaacatgcataattttctagaaactttagatgacatgaagcttagggaccttggctattcgggaacttggtatacataagagagaggctttaagccacggaagagaatgagggagaaacttgatcattttgttgcatcttcatcatggtgtgacttctttccgaaagctacagttgagcacttgatgcgctacaaatcggaccacactcctattttggttcgccttgtaggccatcagtgaagacataagaagaaaaagacgtagttttgttttgagactgcttgggtgcttgaggaaggttgtgaggcccaatgggtgagtcatgggccgggtttactcgcgaggtatttatcgagcgctttaaagccgtggaaggtgggttcaaagcaaggagtgatgggtctcttagtaatctgggcccgcgtgtgagggagattgaggaggccattatagatgggaggcagcgaagcagataaggactatgaggctctatgagactcctctcccacgaaagttagacgaggtgttggacaagcaggagacgttttggtttttgaggtctcgtgtgagttagataaaggatggtgatcgtaatacacaatatttccaccacaaagcttcccaacacaaacgtcgcaactacatagcggggatgtatgataataaaggggtgtggcaagataacgaagaggatattgaagggaatatttcagagtattaccaaacctcgttcggttcgtgctccccctctaggaagaacgtcgcggttgtccttgaggttgtgagcccggtgataactgatgatatgaatatggcggttatgaaatcttacactaaagatgaggtgtgggaagcactaaaccacatgaagcctaacggaatgcatgccatcctttatagaggttctggaataccttggagatgatattacatctgtcattttaggtattattcatggcacccgaccccagatgtttttaacaagactaatattgtgctcattcctaaagtcaaatccccaaatcttgtttctgagtttcgcccgattagcctctgtgatgttatctataaacttgcctcaaaagtacttgctaacagattaaaacaggtttgcctgacattgtttatgataaccagagtgcatttgtgtccggaagctatattacgaacaatgctttgatttctcttgaattatttgactctatgaaaaaatgatacagagctaggaaaggttttgtgtcgatgaaattggatatgagtaaagcctataaaagagttgagtggtgttttttcagtagtgtgttggagaagttggattttgctgaatcatgagtgaatgttgttatgagatgtgtgtcttttgtgcagtactcttttgtggttaatgataatatatgtggagctctgacaccctcaagggggctttgacagggagaccctatatccccgtatttgtttatacttgttgcagataccgttttagctcttcttagcaaggcattcaacaatgcgtggctatacttgatattctcaacaaatatgaggcagcatcaggctagaaaataaatattgacaagtcaggaatctctttcaataaaagatttgacgtattttatggccatgaaacaagttgagaagcatcagaaagacttggtatcccaactttggctaggagttcgaaaaaagtcatatttgctgacattcaagagcgaatttggaagaagctgcacggatggagagaaaaacttctcgcgggcttgaaaagaaactctcttaaaagttgtggttcaagcaattctaacctatttggtgggcgtttacagattcctaaccagtattatccaggccattcatttggccatggtaaagttttggtgggggtcgaaaagggcccacaattcgatgcatctggggggatatgtgctcaccaaaatgtttaaggagccttagctttaaagacttaggggtgttcaatgaacctaaactaaggaggaatgcgtggcatttgattcctgctggtgagtccctttcgggtcgagtgttctcggccaagtactattcgaagtcaacctttttggactcatttctaggtccggtaggtagcttctcttggaagagtatttggggggccaaggcattagttaagggtgttttatggtgcgtaggcaatggcagacaaatcaacatatggcgtgactcgcgggtgttgaatggtgatagtaggttcatccccggagagcgcgtttcaggccttgaggatgtttgtgatctaatagattttgcacaatggagtgcgatgtggaccttgtcacgattgcttcaatgaagatgatgctcaagccattttagtcatacctctaagtaagcgccttctgaaggacatggtctcttgggctttcactaaggatgaattttttttgtaaaaacaacctatatggccggttggtcgaggaatttgaatttgtttcacaaagcatggctgcaaatctggggccttaacgtgtctccgaaggtctgccacttcctttggcgtttatgctcggtacccttcctgttcgagctcttttaaaacgacgccacataactgatgatgattcatgtcctttgtctaaaggagcccggaaagcatatcacacgcgttgttctattgcccatatgtagccgaagcatgggagagtgcgggcctcacaaattgtttgcctttgtttgatggggctggtatgcttgatgcgtggggggagtgggaaacaatcgatgactagtcccttgtaagacttagcttcttggcttatcacttgtggtttaggcgaaataaatgtgtttttgaaggggtggtgagagcgaatgagagtgttgtggaatatgccactaaagctactgttgatcatggtttgtatagtgcccgcatttatggtgggtcgaaggctaccgcatccaaaagctcgaaggtatgggttccccctccagcttgtcgtacgatctaaaggttgatgcatcagtggggaatggtggatgggtggggctaggagtaatcgcctgaaactagaaaggggaggtgctcgtggctgcaactaggagggtcagagcttgtggcccgtggaaatggctgaagggaaggctctttgtcttgctcttaggcttgcctcgctcatacaacttgcaagaagtgatcgtggagtttgactgtcaatcttggtgaaccatctctccaagggtgctatttactttgcatttttaagtcaaagcttgaaccttgataaaaaaatcccgttcgacatgaaaagtgccttgattttgcgggtttgggagtgccttattgattctggggtttgatttgtaacacctttagtaaaaacatgtaagctaactgtaaaacgaacattaatcaaactaggatatgtaaaattcctaaatcaagaagaatttccacttgtgctgaatttgtccaccttgcatgacacccaataaaagcccatgtctcctagaaccccttatgccgccttattcatcttttctcaagttgagttggagtcctctatggtccactcgacttctttagcacactctcggtaaaaacttttaatattattttattttagactccaccatcttgacatttattccttcttaaacttgcttcacacaaacatctaacactagaattctatatagaatagcttgaatctctcttaggataaccttatagtaaatgcaactacgcctatccttaaacctttctaagaggagctttatcgtatttacattcgcttcactttgaaacgtcgctaagtgtatgttgcactttccaaaccatgtgttagctaagaccaagttatatgactgcataacctaaatagtcttcctcgagaaaattcactagttggatcggaagagtttgtgtaaatctatggcggcgcgggactgggccttcacgatttcaagtgttttaatgcagctcttctaggtaaacaagtttcctaatagcgtggtgactcaaatattgaggacttgttgttatactaatgctattcctggcggcacttaaggggtgaaataggtggtacaaaggagtgcttgatggcgtgtgggtagtagttgaatatatcagtatgatcaagtccatggatccctcgtacttattcgtgcaagattatttttccacgaggcaaagcgagcgagaatcttaaggtttatgatcatattcatcttgtacgtgctaagggtaatgtccctttcaataatgagctatttctccttttgagcaagagcgtatcttaagcattcctcgtagttctcgtctccccaacgatgttttatgttggaatctgaatttggagaaagacggagacttttcgttcggtctatcgagccattcttttgagttggatggcgagagcgtgatttcatcgtcaatacgctctaatttatggagtataatatggcaggatagtacctttcaacgtgttaagcttttatctgcattgtcgacacaaaggggattgagtaagcctgtgccgagtatggaaccattgtgtaatctttatgcgttggaggatcaatggagctacacttcttacgagactttgttattggaagggcttatatgggatccaactagggtagtcaaaacattggtcggggctgcgctgcaattttggggacttggcaccggcgtttttggagtagctccctcatgtggaacataggcttttgatgacgatatactaggctagatggaatataagagagaggtgtttgtttgaggaggaggtttgtgatccctatcaaaccacatgcataatctcatggcgtagcttcatgtggaacactgacatattgcatgtgtagggttaggtgcttgcctaggacaccacatgggaagagctccgttaagcttaatgtggatggagggtgtgtggaagggttgggtgcgtccactggagtggtgattagggggatggatgaaaaagcgttgtagttgcaacatagaaaggtggaggactgcgaggaaccgttaaaaaggctatattttatggtgttcatttggttgtggaagtcgatttttgaaatatggttgttggaagtgactatcttcacctcgttgaagcaacttcttcaaaagtggaaggcaaaaatagcttccatgttattgttgatgacattgttcatggtagtggtatgttaaatacttcgtcttgtagttttgttcgtagggatgggaatagggtttctcacgaactcccccatggaaatatcataatggctcatgctcataggtaaatgaataagctaacaaaattgttcatctttgcagaaccaactcatgcatgaatcgatttctcagcttcagcgaaaggtagacagctctagagagagcatctagtctcaaaaataccatgagattctgtagtgtcctgacatgttttatatgacaggacaaagcgttaaaggagcacaacaacttgctatccaagaaggtataagttcagcaagattgtttagtaacattgttaatcttgctgattgctttgaaacatgtcttgctatggttaacaatgttgactgaaccaaaataggtgaaggagagggagaaggtgctggctcagcaggcagaattggatcagcaaaatcatgacaataactcatctggctttgtgatgtctcaagctttgccctcactgaatacagggtcagtcctcaataacctctaatcatttttccaagatccaaagtaaacatggtttcataatttaattaagatttttttgaaccatgtctccatacaaccttactaggactaatactactaatttaagaccccaacgataaacaacaataattagccatatctggctagcaccttttggacaacacaccacatgagactcttggccaacttctttgatttccttcagtctgatagatatgaatatcttctgaagagctctttggttcataattattgatttagaaaagaattcagcaaggtgagtcatttggtaaccttaaggtcattatgggggtactaaatcaaagtgaagatatatttaggtggcatcagaagagatgatatagataggttgtatcctgtcgataggttatttggatatgtatcaaaagtttcttttataatatatctatactgattggttgatgtatcaaatatccctacagattgtgaaaaaatcccctacagattgtgaaaatatccctagaacctgtgatgatataagatgtgctccgcatgctttattgaacataatgtattcaattcttgaaatgcagaggaacaagcagcagtgcagtggaagatgaagcaacacaaccaccaaatctaaacagcaactctgcacaaataccgtcctggatgcttcaacacatccaagagcagtaa

SEQ ID NO: 41 - protein, 256 aa, Arabidopsis thaliana
MGRGRVQLKRIENKINRQVTFSKRRAGLLKKAHEISVLCDAEVALVVFSHKGKLFEYSTDSCMEKILERYERYSYAERQLIAPESDVNTNWSMEYNRLKAKIELLERNQRHYLGEDLQAMSPKELQNLEQQLDTALKHIRTRKNQLMYESINELQKKEKAIQEQNSMLSKQIKEREKILRAQQEQWDQQNQGHNMPPPLPPQQHQIQHPYMLSHQPSPFLNMGGLYQEDDPMAMRRNDLELTLEPVYNCNLGCFAA

SEQ ID NO: 42 - protein, 242 aa, Arabidopsis thaliana
MGRGRVQLKRIENKINRQVTFSKRRSGLLKKAHEISVLCDAEVALIVFSSKGKLFEYSTDSCMERILERYDRYLYSDKQLVGRDVSQSENWVLEHAKLKARVEVLEKNKRNFMGEDLDSLSLKELQSLEHQLDAAIKSIRSRKNQAMFESISALQKKDKALQDHNNSLLKKIKEREKKTGQQEGQLVQCSNSSSVLLPQYCVTSSRDGFVERVGGENGGASSLTEPNSLLPAWMLRPTTTNE